European Patent Application EP 4 527 856 A1, published March 26, 2025. Title: FUSION PROTEIN COMPRISING LIGHT PROTEIN AND ANTI-FAP ANTIBODY AND USE THEREOF. Applicant: Kanaph Therapeutics Inc. Application KR PCT/KR2023/006839, filed May 19, 2023. The sequence listing filed with the application follows.

SEQUENCE LISTING (298 sequences)

SEQ ID NO: 1 - protein, 454 aa, synthetic construct
  REGION 1..454: note = anti-hu FAP HC-hu IgG1 Fc Knob DANG
QVQLVQSGAEVKKPGASVKVSCKTSRYTFTEYTIHWVRQAPGQRLEWIGGINPNNGIPNYNQKFKGRVTITVDTSASTAYMELSSLRSEDTAVYYCARRRIAYGYDEGHAMDYWGQGTLVTVSSASTKGPSVFPLAPSSKSTSGGTAALGCLVKDYFPEPVTVSWNSGALTSGVHTFPAVLQSSGLYSLSSVVTVPSSSLGTQTYICNVNHKPSNTKVDKKVEPKSCDKTHTCPPCPAPELLGGPSVFLFPPKPKDTLMISRTPEVTCVVVAVSHEDPEVKFNWYVDGVEVHNAKTKPREEQYGSTYRVVSVLTVLHQDWLNGKEYKCKVSNKALPAPIEKTISKAKGQPREPQVYTLPPSRDELTKNQVSLWCLVKGFYPSDIAVEWESNGQPENNYKTTPPVLDSDGSFFLYSKLTVDKSRWQQGNVFSCSVMHEALHNHYTQKSLSLSPGK

SEQ ID NO: 2 - protein, 220 aa, synthetic construct
  REGION 1..220: note = anti-hu FAP LC
DIVMTQSPDSLAVSLGERATINCKSSQSLLYSRNQKNYLAWYQQKPGQPPKLLIFWASTRESGVPDRFSGSGFGTDFTLTISSLQAEDVAVYYCQQYFSYPLTFGQGTKVEIKRTVAAPSVFIFPPSDEQLKSGTASVVCLLNNFYPREAKVQWKVDNALQSGNSQESVTEQDSKDSTYSLSSTLTLSKADYEKHKVYACEVTHQGLSSPVTKSFNRGEC

SEQ ID NO: 3 - protein, 693 aa, synthetic construct
  REGION 1..693: note = hu scLIGHT3-hu IgG1 Fc hole DANG
EVNPAAHLTGANSSLTGSGGPLLWETQLGLAFLRGLSYHDGALVVTKAGYYYIYSKVQLGGVGCPLGLASTITHGLYKRTPRYPEELELLVSQQSPCGRATSSSRVWWDSSFLGGVVHLEAGEKVVVRVLDERLVRLRDGTRSYFGAFMVGGSGEVNPAAHLTGANSSLTGSGGPLLWETQLGLAFLRGLSYHDGALVVTKAGYYYIYSKVQLGGVGCPLGLASTITHGLYKRTPRYPEELELLVSQQSPCGRATSSSRVWWDSSFLGGVVHLEAGEKVVVRVLDERLVRLRDGTRSYFGAFMVGGSGEVNPAAHLTGANSSLTGSGGPLLWETQLGLAFLRGLSYHDGALVVTKAGYYYIYSKVQLGGVGCPLGLASTITHGLYKRTPRYPEELELLVSQQSPCGRATSSSRVWWDSSFLGGVVHLEAGEKVVVRVLDERLVRLRDGTRSYFGAFMVGGSGGGGSDKTHTCPPCPAPELLGGPSVFLFPPKPKDTLMISRTPEVTCVVVAVSHEDPEVKFNWYVDGVEVHNAKTKPREEQYGSTYRVVSVLTVLHQDWLNGKEYKCKVSNKALPAPIEKTISKAKGQPREPQVYTLPPSRDELTKNQVSLSCAVKGFYPSDIAVEWESNGQPENNYKTTPPVLDSDGSFFLVSKLTVDKSRWQQGNVFSCSVMHEALHNHYTQKSLSLSPGK

SEQ ID NO: 4 - protein, 454 aa, synthetic construct
  REGION 1..454: note = anti-hu FAP HC-hu IgG1 Fc knob
QVQLVQSGAEVKKPGASVKVSCKTSRYTFTEYTIHWVRQAPGQRLEWIGGINPNNGIPNYNQKFKGRVTITVDTSASTAYMELSSLRSEDTAVYYCARRRIAYGYDEGHAMDYWGQGTLVTVSSASTKGPSVFPLAPSSKSTSGGTAALGCLVKDYFPEPVTVSWNSGALTSGVHTFPAVLQSSGLYSLSSVVTVPSSSLGTQTYICNVNHKPSNTKVDKKVEPKSCDKTHTCPPCPAPELLGGPSVFLFPPKPKDTLMISRTPEVTCVVVDVSHEDPEVKFNWYVDGVEVHNAKTKPREEQYNSTYRVVSVLTVLHQDWLNGKEYKCKVSNKALPAPIEKTISKAKGQPREPQVYTLPPSRDELTKNQVSLWCLVKGFYPSDIAVEWESNGQPENNYKTTPPVLDSDGSFFLYSKLTVDKSRWQQGNVFSCSVMHEALHNHYTQKSLSLSPGK

SEQ ID NO: 5 - protein, 693 aa, synthetic construct
  REGION 1..693: note = hu scLIGHT3-hu IgG1 Fc hole
EVNPAAHLTGANSSLTGSGGPLLWETQLGLAFLRGLSYHDGALVVTKAGYYYIYSKVQLGGVGCPLGLASTITHGLYKRTPRYPEELELLVSQQSPCGRATSSSRVWWDSSFLGGVVHLEAGEKVVVRVLDERLVRLRDGTRSYFGAFMVGGSGEVNPAAHLTGANSSLTGSGGPLLWETQLGLAFLRGLSYHDGALVVTKAGYYYIYSKVQLGGVGCPLGLASTITHGLYKRTPRYPEELELLVSQQSPCGRATSSSRVWWDSSFLGGVVHLEAGEKVVVRVLDERLVRLRDGTRSYFGAFMVGGSGEVNPAAHLTGANSSLTGSGGPLLWETQLGLAFLRGLSYHDGALVVTKAGYYYIYSKVQLGGVGCPLGLASTITHGLYKRTPRYPEELELLVSQQSPCGRATSSSRVWWDSSFLGGVVHLEAGEKVVVRVLDERLVRLRDGTRSYFGAFMVGGSGGGGSDKTHTCPPCPAPELLGGPSVFLFPPKPKDTLMISRTPEVTCVVVDVSHEDPEVKFNWYVDGVEVHNAKTKPREEQYNSTYRVVSVLTVLHQDWLNGKEYKCKVSNKALPAPIEKTISKAKGQPREPQVYTLPPSRDELTKNQVSLSCAVKGFYPSDIAVEWESNGQPENNYKTTPPVLDSDGSFFLVSKLTVDKSRWQQGNVFSCSVMHEALHNHYTQKSLSLSPGK

SEQ ID NO: 6 - protein, 737 aa, synthetic construct
  REGION 1..737: note = hu scLIGHT3(GGGGS4)-hu IgG1 Fc hole DANG
EVNPAAHLTGANSSLTGSGGPLLWETQLGLAFLRGLSYHDGALVVTKAGYYYIYSKVQLGGVGCPLGLASTITHGLYKRTPRYPEELELLVSQQSPCGRATSSSRVWWDSSFLGGVVHLEAGEKVVVRVLDERLVRLRDGTRSYFGAFMVGGGGSGGGGSGGGGSGGGGSEVNPAAHLTGANSSLTGSGGPLLWETQLGLAFLRGLSYHDGALVVTKAGYYYIYSKVQLGGVGCPLGLASTITHGLYKRTPRYPEELELLVSQQSPCGRATSSSRVWWDSSFLGGVVHLEAGEKVVVRVLDERLVRLRDGTRSYFGAFMVGGGGSGGGGSGGGGSGGGGSEVNPAAHLTGANSSLTGSGGPLLWETQLGLAFLRGLSYHDGALVVTKAGYYYIYSKVQLGGVGCPLGLASTITHGLYKRTPRYPEELELLVSQQSPCGRATSSSRVWWDSSFLGGVVHLEAGEKVVVRVLDERLVRLRDGTRSYFGAFMVGGGGSGGGGSGGGGSGGGGSDKTHTCPPCPAPELLGGPSVFLFPPKPKDTLMISRTPEVTCVVVAVSHEDPEVKFNWYVDGVEVHNAKTKPREEQYGSTYRVVSVLTVLHQDWLNGKEYKCKVSNKALPAPIEKTISKAKGQPREPQVYTLPPSRDELTKNQVSLSCAVKGFYPSDIAVEWESNGQPENNYKTTPPVLDSDGSFFLVSKLTVDKSRWQQGNVFSCSVMHEALHNHYTQKSLSLSPGK

SEQ ID NO: 7 - protein, 693 aa, synthetic construct
  REGION 1..693: note = hu scLIGHT(226-231)3-hu IgG1 Fc hole DANG
EVNPAAHLTGANSSLTGSGGPLLWETQLGLAFLRGLSYHDGALVVTKAGYYYIYSKVQLGGVGCPLGLASTITHGLYKRTPRYPEELELLVSQQSPCGRATSSSRVWWDSSFLGGVVHLEAGEKVVVRVLDERLVDYTKEDRSYFGAFMVGGSGEVNPAAHLTGANSSLTGSGGPLLWETQLGLAFLRGLSYHDGALVVTKAGYYYIYSKVQLGGVGCPLGLASTITHGLYKRTPRYPEELELLVSQQSPCGRATSSSRVWWDSSFLGGVVHLEAGEKVVVRVLDERLVDYTKEDRSYFGAFMVGGSGEVNPAAHLTGANSSLTGSGGPLLWETQLGLAFLRGLSYHDGALVVTKAGYYYIYSKVQLGGVGCPLGLASTITHGLYKRTPRYPEELELLVSQQSPCGRATSSSRVWWDSSFLGGVVHLEAGEKVVVRVLDERLVDYTKEDRSYFGAFMVGGSGGGGSDKTHTCPPCPAPELLGGPSVFLFPPKPKDTLMISRTPEVTCVVVAVSHEDPEVKFNWYVDGVEVHNAKTKPREEQYGSTYRVVSVLTVLHQDWLNGKEYKCKVSNKALPAPIEKTISKAKGQPREPQVYTLPPSRDELTKNQVSLSCAVKGFYPSDIAVEWESNGQPENNYKTTPPVLDSDGSFFLVSKLTVDKSRWQQGNVFSCSVMHEALHNHYTQKSLSLSPGK

SEQ ID NO: 8 - protein, 693 aa, synthetic construct
  REGION 1..693: note = hu scLIGHT(195-198)3-hu IgG1 Fc hole DANG
EVNPAAHLTGANSSLTGSGGPLLWETQLGLAFLRGLSYHDGALVVTKAGYYYIYSKVQLGGVGCPLGLASTITHGLYKRTPRYPEELELLVSQQSPCGRATSSSSNWFDSSFLGGVVHLEAGEKVVVRVLDERLVRLRDGTRSYFGAFMVGGSGEVNPAAHLTGANSSLTGSGGPLLWETQLGLAFLRGLSYHDGALVVTKAGYYYIYSKVQLGGVGCPLGLASTITHGLYKRTPRYPEELELLVSQQSPCGRATSSSSNWFDSSFLGGVVHLEAGEKVVVRVLDERLVRLRDGTRSYFGAFMVGGSGEVNPAAHLTGANSSLTGSGGPLLWETQLGLAFLRGLSYHDGALVVTKAGYYYIYSKVQLGGVGCPLGLASTITHGLYKRTPRYPEELELLVSQQSPCGRATSSSSNWFDSSFLGGVVHLEAGEKVVVRVLDERLVRLRDGTRSYFGAFMVGGSGGGGSDKTHTCPPCPAPELLGGPSVFLFPPKPKDTLMISRTPEVTCVVVAVSHEDPEVKFNWYVDGVEVHNAKTKPREEQYGSTYRVVSVLTVLHQDWLNGKEYKCKVSNKALPAPIEKTISKAKGQPREPQVYTLPPSRDELTKNQVSLSCAVKGFYPSDIAVEWESNGQPENNYKTTPPVLDSDGSFFLVSKLTVDKSRWQQGNVFSCSVMHEALHNHYTQKSLSLSPGK

SEQ ID NO: 9 - protein, 768 aa, synthetic construct
  REGION 1..768: note = anti-hu FAP HC hu IgG1 Fc knob DANG-hu scLIGHT2
QVQLVQSGAEVKKPGASVKVSCKTSRYTFTEYTIHWVRQAPGQRLEWIGGINPNNGIPNYNQKFKGRVTITVDTSASTAYMELSSLRSEDTAVYYCARRRIAYGYDEGHAMDYWGQGTLVTVSSASTKGPSVFPLAPSSKSTSGGTAALGCLVKDYFPEPVTVSWNSGALTSGVHTFPAVLQSSGLYSLSSVVTVPSSSLGTQTYICNVNHKPSNTKVDKKVEPKSCDKTHTCPPCPAPELLGGPSVFLFPPKPKDTLMISRTPEVTCVVVAVSHEDPEVKFNWYVDGVEVHNAKTKPREEQYGSTYRVVSVLTVLHQDWLNGKEYKCKVSNKALPAPIEKTISKAKGQPREPQVYTLPPSRDELTKNQVSLWCLVKGFYPSDIAVEWESNGQPENNYKTTPPVLDSDGSFFLYSKLTVDKSRWQQGNVFSCSVMHEALHNHYTQKSLSLSPGKGGGGSGGGGSEVNPAAHLTGANSSLTGSGGPLLWETQLGLAFLRGLSYHDGALVVTKAGYYYIYSKVQLGGVGCPLGLASTITHGLYKRTPRYPEELELLVSQQSPCGRATSSSRVWWDSSFLGGVVHLEAGEKVVVRVLDERLVRLRDGTRSYFGAFMVGGSGEVNPAAHLTGANSSLTGSGGPLLWETQLGLAFLRGLSYHDGALVVTKAGYYYIYSKVQLGGVGCPLGLASTITHGLYKRTPRYPEELELLVSQQSPCGRATSSSRVWWDSSFLGGVVHLEAGEKVVVRVLDERLVRLRDGTRSYFGAFMV

SEQ ID NO: 10 - protein, 614 aa, synthetic construct
  REGION 1..614: note = anti-hu FAP HC hu IgG1 Fc hole DANG-hu LIGHT
QVQLVQSGAEVKKPGASVKVSCKTSRYTFTEYTIHWVRQAPGQRLEWIGGINPNNGIPNYNQKFKGRVTITVDTSASTAYMELSSLRSEDTAVYYCARRRIAYGYDEGHAMDYWGQGTLVTVSSASTKGPSVFPLAPSSKSTSGGTAALGCLVKDYFPEPVTVSWNSGALTSGVHTFPAVLQSSGLYSLSSVVTVPSSSLGTQTYICNVNHKPSNTKVDKKVEPKSCDKTHTCPPCPAPELLGGPSVFLFPPKPKDTLMISRTPEVTCVVVAVSHEDPEVKFNWYVDGVEVHNAKTKPREEQYGSTYRVVSVLTVLHQDWLNGKEYKCKVSNKALPAPIEKTISKAKGQPREPQVYTLPPSRDELTKNQVSLSCAVKGFYPSDIAVEWESNGQPENNYKTTPPVLDSDGSFFLVSKLTVDKSRWQQGNVFSCSVMHEALHNHYTQKSLSLSPGKGGGGSGGGGSEVNPAAHLTGANSSLTGSGGPLLWETQLGLAFLRGLSYHDGALVVTKAGYYYIYSKVQLGGVGCPLGLASTITHGLYKRTPRYPEELELLVSQQSPCGRATSSSRVWWDSSFLGGVVHLEAGEKVVVRVLDERLVRLRDGTRSYFGAFMV

SEQ ID NO: 11 - protein, 613 aa, synthetic construct
  REGION 1..613: note = anti-hu FAP HC hu IgG1 Fc DANG-hu LIGHT
QVQLVQSGAEVKKPGASVKVSCKTSRYTFTEYTIHWVRQAPGQRLEWIGGINPNNGIPNYNQKFKGRVTITVDTSASTAYMELSSLRSEDTAVYYCARRRIAYGYDEGHAMDYWGQGTLVTVSSASTKGPSVFPLAPSSKSTSGGTAALGCLVKDYFPEPVTVSWNSGALTSGVHTFPAVLQSSGLYSLSSVVTVPSSSLGTQTYICNVNHKPSNTKVDKKVEPKSCDKTHTCPPCPAPELLGGPSVFLFPPKPKDTLMISRTPEVTCVVVAVSHEDPEVKFNWYVDGVEVHNAKTKPREEQYGSTYRVVSVLTVLHQDWLNGKEYKCKVSNKALPAPIEKTISKAKGQPREPQVYTLPPSRDELTKNQVSLTCLVKGFYPSDIAVEWESNGQPENNYKTTPPVLDSDGSFFLYSKLTVDKSRWQQGNVFSCSVMHEALHNHYTQKSLSLSPGGGGGSGGGGSEVNPAAHLTGANSSLTGSGGPLLWETQLGLAFLRGLSYHDGALVVTKAGYYYIYSKVQLGGVGCPLGLASTITHGLYKRTPRYPEELELLVSQQSPCGRATSSSRVWWDSSFLGGVVHLEAGEKVVVRVLDERLVRLRDGTRSYFGAFMV

SEQ ID NO: 12 - protein, 767 aa, synthetic construct
  REGION 1..767: note = anti-hu FAP HC hu IgG1 Fc knob-hu scLIGHT2
QVQLVQSGAEVKKPGASVKVSCKTSRYTFTEYTIHWVRQAPGQRLEWIGGINPNNGIPNYNQKFKGRVTITVDTSASTAYMELSSLRSEDTAVYYCARRRIAYGYDEGHAMDYWGQGTLVTVSSASTKGPSVFPLAPSSKSTSGGTAALGCLVKDYFPEPVTVSWNSGALTSGVHTFPAVLQSSGLYSLSSVVTVPSSSLGTQTYICNVNHKPSNTKVDKKVEPKSCDKTHTCPPCPAPELLGGPSVFLFPPKPKDTLMISRTPEVTCVVVDVSHEDPEVKFNWYVDGVEVHNAKTKPREEQYNSTYRVVSVLTVLHQDWLNGKEYKCKVSNKALPAPIEKTISKAKGQPREPQVYTLPPSRDELTKNQVSLWCLVKGFYPSDIAVEWESNGQPENNYKTTPPVLDSDGSFFLYSKLTVDKSRWQQGNVFSCSVMHEALHNHYTQKSLSLSPGGGGGSGGGGSEVNPAAHLTGANSSLTGSGGPLLWETQLGLAFLRGLSYHDGALVVTKAGYYYIYSKVQLGGVGCPLGLASTITHGLYKRTPRYPEELELLVSQQSPCGRATSSSRVWWDSSFLGGVVHLEAGEKVVVRVLDERLVRLRDGTRSYFGAFMVGGSGEVNPAAHLTGANSSLTGSGGPLLWETQLGLAFLRGLSYHDGALVVTKAGYYYIYSKVQLGGVGCPLGLASTITHGLYKRTPRYPEELELLVSQQSPCGRATSSSRVWWDSSFLGGVVHLEAGEKVVVRVLDERLVRLRDGTRSYFGAFMV

SEQ ID NO: 13 - protein, 613 aa, synthetic construct
  REGION 1..613: note = anti-hu FAP HC hu IgG1 Fc hole-hu LIGHT
QVQLVQSGAEVKKPGASVKVSCKTSRYTFTEYTIHWVRQAPGQRLEWIGGINPNNGIPNYNQKFKGRVTITVDTSASTAYMELSSLRSEDTAVYYCARRRIAYGYDEGHAMDYWGQGTLVTVSSASTKGPSVFPLAPSSKSTSGGTAALGCLVKDYFPEPVTVSWNSGALTSGVHTFPAVLQSSGLYSLSSVVTVPSSSLGTQTYICNVNHKPSNTKVDKKVEPKSCDKTHTCPPCPAPELLGGPSVFLFPPKPKDTLMISRTPEVTCVVVDVSHEDPEVKFNWYVDGVEVHNAKTKPREEQYNSTYRVVSVLTVLHQDWLNGKEYKCKVSNKALPAPIEKTISKAKGQPREPQVYTLPPSRDELTKNQVSLSCAVKGFYPSDIAVEWESNGQPENNYKTTPPVLDSDGSFFLVSKLTVDKSRWQQGNVFSCSVMHEALHNHYTQKSLSLSPGGGGGSGGGGSEVNPAAHLTGANSSLTGSGGPLLWETQLGLAFLRGLSYHDGALVVTKAGYYYIYSKVQLGGVGCPLGLASTITHGLYKRTPRYPEELELLVSQQSPCGRATSSSRVWWDSSFLGGVVHLEAGEKVVVRVLDERLVRLRDGTRSYFGAFMV

SEQ ID NO: 14 - protein, 227 aa, synthetic construct
  REGION 1..227: note = hu IgG1 Fc hole DANG
DKTHTCPPCPAPELLGGPSVFLFPPKPKDTLMISRTPEVTCVVVAVSHEDPEVKFNWYVDGVEVHNAKTKPREEQYGSTYRVVSVLTVLHQDWLNGKEYKCKVSNKALPAPIEKTISKAKGQPREPQVYTLPPSRDELTKNQVSLSCAVKGFYPSDIAVEWESNGQPENNYKTTPPVLDSDGSFFLVSKLTVDKSRWQQGNVFSCSVMHEALHNHYTQKSLSLSPGK

SEQ ID NO: 15 - protein, 227 aa, synthetic construct
  REGION 1..227: note = hu IgG1 Fc knob DANG
DKTHTCPPCPAPELLGGPSVFLFPPKPKDTLMISRTPEVTCVVVAVSHEDPEVKFNWYVDGVEVHNAKTKPREEQYGSTYRVVSVLTVLHQDWLNGKEYKCKVSNKALPAPIEKTISKAKGQPREPQVYTLPPSRDELTKNQVSLWCLVKGFYPSDIAVEWESNGQPENNYKTTPPVLDSDGSFFLYSKLTVDKSRWQQGNVFSCSVMHEALHNHYTQKSLSLSPGK

SEQ ID NO: 16 - protein, 454 aa, synthetic construct
  REGION 1..454: note = anti-hu FAP HC hu IgG1 Fc DANG
QVQLVQSGAEVKKPGASVKVSCKTSRYTFTEYTIHWVRQAPGQRLEWIGGINPNNGIPNYNQKFKGRVTITVDTSASTAYMELSSLRSEDTAVYYCARRRIAYGYDEGHAMDYWGQGTLVTVSSASTKGPSVFPLAPSSKSTSGGTAALGCLVKDYFPEPVTVSWNSGALTSGVHTFPAVLQSSGLYSLSSVVTVPSSSLGTQTYICNVNHKPSNTKVDKKVEPKSCDKTHTCPPCPAPELLGGPSVFLFPPKPKDTLMISRTPEVTCVVVAVSHEDPEVKFNWYVDGVEVHNAKTKPREEQYGSTYRVVSVLTVLHQDWLNGKEYKCKVSNKALPAPIEKTISKAKGQPREPQVYTLPPSRDELTKNQVSLTCLVKGFYPSDIAVEWESNGQPENNYKTTPPVLDSDGSFFLYSKLTVDKSRWQQGNVFSCSVMHEALHNHYTQKSLSLSPGK

SEQ ID NO: 17 - protein, 718 aa, synthetic construct
  REGION 1..718: note = hu scLIGHT-LTb2-hu IgG1 Fc hole DANG
EVNPAAHLTGANSSLTGSGGPLLWETQLGLAFLRGLSYHDGALVVTKAGYYYIYSKVQLGGVGCPLGLASTITHGLYKRTPRYPEELELLVSQQSPCGRATSSSRVWWDSSFLGGVVHLEAGEKVVVRVLDERLVRLRDGTRSYFGAFMVGGGGSGGGGSGGGGSLPAAHLIGAPLKGQGLGWETTKEQAFLTSGTQFSDAEGLALPQDGLYYLYCLVGYRGRAPPGGGDPQGRSVTLRSSLYRAGGAYGPGTPELLLEGAETVTPVLDPARRQGYGPLWYTSVGFGGLVQLRRGERVYVNISHPDMVDFARGKTFFGAVMVGGSGLPAAHLIGAPLKGQGLGWETTKEQAFLTSGTQFSDAEGLALPQDGLYYLYCLVGYRGRAPPGGGDPQGRSVTLRSSLYRAGGAYGPGTPELLLEGAETVTPVLDPARRQGYGPLWYTSVGFGGLVQLRRGERVYVNISHPDMVDFARGKTFFGAVMVGGSGGGGSDKTHTCPPCPAPELLGGPSVFLFPPKPKDTLMISRTPEVTCVVVAVSHEDPEVKFNWYVDGVEVHNAKTKPREEQYGSTYRVVSVLTVLHQDWLNGKEYKCKVSNKALPAPIEKTISKAKGQPREPQVYTLPPSRDELTKNQVSLSCAVKGFYPSDIAVEWESNGQPENNYKTTPPVLDSDGSFFLVSKLTVDKSRWQQGNVFSCSVMHEALHNHYTQKSLSLSPGK

SEQ ID NO: 18 - protein, 693 aa, synthetic construct
  REGION 1..693: note = hu scLIGHT-LIGHT(L118K, G119E)2-hu IgG1 Fc hole DANG
EVNPAAHLTGANSSLTGSGGPLLWETQLGLAFLRGLSYHDGALVVTKAGYYYIYSKVQLGGVGCPLGLASTITHGLYKRTPRYPEELELLVSQQSPCGRATSSSRVWWDSSFLGGVVHLEAGEKVVVRVLDERLVRLRDGTRSYFGAFMVGGSGEVNPAAHLTGANSSLTGSGGPLLWETQKELAFLRGLSYHDGALVVTKAGYYYIYSKVQLGGVGCPLGLASTITHGLYKRTPRYPEELELLVSQQSPCGRATSSSRVWWDSSFLGGVVHLEAGEKVVVRVLDERLVRLRDGTRSYFGAFMVGGSGEVNPAAHLTGANSSLTGSGGPLLWETQKELAFLRGLSYHDGALVVTKAGYYYIYSKVQLGGVGCPLGLASTITHGLYKRTPRYPEELELLVSQQSPCGRATSSSRVWWDSSFLGGVVHLEAGEKVVVRVLDERLVRLRDGTRSYFGAFMVGGSGGGGSDKTHTCPPCPAPELLGGPSVFLFPPKPKDTLMISRTPEVTCVVVAVSHEDPEVKFNWYVDGVEVHNAKTKPREEQYGSTYRVVSVLTVLHQDWLNGKEYKCKVSNKALPAPIEKTISKAKGQPREPQVYTLPPSRDELTKNQVSLSCAVKGFYPSDIAVEWESNGQPENNYKTTPPVLDSDGSFFLVSKLTVDKSRWQQGNVFSCSVMHEALHNHYTQKSLSLSPGK

SEQ ID NO: 19 - protein, 718 aa, synthetic construct
  REGION 1..718: note = hu scLIGHT(226-231)-LTb2-hu IgG1 Fc hole DANG
EVNPAAHLTGANSSLTGSGGPLLWETQLGLAFLRGLSYHDGALVVTKAGYYYIYSKVQLGGVGCPLGLASTITHGLYKRTPRYPEELELLVSQQSPCGRATSSSRVWWDSSFLGGVVHLEAGEKVVVRVLDERLVDYTKEDRSYFGAFMVGGGGSGGGGSGGGGSLPAAHLIGAPLKGQGLGWETTKEQAFLTSGTQFSDAEGLALPQDGLYYLYCLVGYRGRAPPGGGDPQGRSVTLRSSLYRAGGAYGPGTPELLLEGAETVTPVLDPARRQGYGPLWYTSVGFGGLVQLRRGERVYVNISHPDMVDFARGKTFFGAVMVGGSGLPAAHLIGAPLKGQGLGWETTKEQAFLTSGTQFSDAEGLALPQDGLYYLYCLVGYRGRAPPGGGDPQGRSVTLRSSLYRAGGAYGPGTPELLLEGAETVTPVLDPARRQGYGPLWYTSVGFGGLVQLRRGERVYVNISHPDMVDFARGKTFFGAVMVGGSGGGGSDKTHTCPPCPAPELLGGPSVFLFPPKPKDTLMISRTPEVTCVVVAVSHEDPEVKFNWYVDGVEVHNAKTKPREEQYGSTYRVVSVLTVLHQDWLNGKEYKCKVSNKALPAPIEKTISKAKGQPREPQVYTLPPSRDELTKNQVSLSCAVKGFYPSDIAVEWESNGQPENNYKTTPPVLDSDGSFFLVSKLTVDKSRWQQGNVFSCSVMHEALHNHYTQKSLSLSPGK

SEQ ID NO: 20 - protein, 718 aa, synthetic construct
  REGION 1..718: note = hu scLIGHT(195-198)-LTb2-hu IgG1 Fc hole DANG
EVNPAAHLTGANSSLTGSGGPLLWETQLGLAFLRGLSYHDGALVVTKAGYYYIYSKVQLGGVGCPLGLASTITHGLYKRTPRYPEELELLVSQQSPCGRATSSSSNWFDSSFLGGVVHLEAGEKVVVRVLDERLVRLRDGTRSYFGAFMVGGGGSGGGGSGGGGSLPAAHLIGAPLKGQGLGWETTKEQAFLTSGTQFSDAEGLALPQDGLYYLYCLVGYRGRAPPGGGDPQGRSVTLRSSLYRAGGAYGPGTPELLLEGAETVTPVLDPARRQGYGPLWYTSVGFGGLVQLRRGERVYVNISHPDMVDFARGKTFFGAVMVGGSGLPAAHLIGAPLKGQGLGWETTKEQAFLTSGTQFSDAEGLALPQDGLYYLYCLVGYRGRAPPGGGDPQGRSVTLRSSLYRAGGAYGPGTPELLLEGAETVTPVLDPARRQGYGPLWYTSVGFGGLVQLRRGERVYVNISHPDMVDFARGKTFFGAVMVGGSGGGGSDKTHTCPPCPAPELLGGPSVFLFPPKPKDTLMISRTPEVTCVVVAVSHEDPEVKFNWYVDGVEVHNAKTKPREEQYGSTYRVVSVLTVLHQDWLNGKEYKCKVSNKALPAPIEKTISKAKGQPREPQVYTLPPSRDELTKNQVSLSCAVKGFYPSDIAVEWESNGQPENNYKTTPPVLDSDGSFFLVSKLTVDKSRWQQGNVFSCSVMHEALHNHYTQKSLSLSPGK

SEQ ID NO: 21 - protein, 707 aa, synthetic construct
  REGION 1..707: note = hu scLIGHT-LTb2(GGSG)-hu IgG1 Fc hole DANG
EVNPAAHLTGANSSLTGSGGPLLWETQLGLAFLRGLSYHDGALVVTKAGYYYIYSKVQLGGVGCPLGLASTITHGLYKRTPRYPEELELLVSQQSPCGRATSSSRVWWDSSFLGGVVHLEAGEKVVVRVLDERLVRLRDGTRSYFGAFMVGGSGLPAAHLIGAPLKGQGLGWETTKEQAFLTSGTQFSDAEGLALPQDGLYYLYCLVGYRGRAPPGGGDPQGRSVTLRSSLYRAGGAYGPGTPELLLEGAETVTPVLDPARRQGYGPLWYTSVGFGGLVQLRRGERVYVNISHPDMVDFARGKTFFGAVMVGGSGLPAAHLIGAPLKGQGLGWETTKEQAFLTSGTQFSDAEGLALPQDGLYYLYCLVGYRGRAPPGGGDPQGRSVTLRSSLYRAGGAYGPGTPELLLEGAETVTPVLDPARRQGYGPLWYTSVGFGGLVQLRRGERVYVNISHPDMVDFARGKTFFGAVMVGGSGGGGSDKTHTCPPCPAPELLGGPSVFLFPPKPKDTLMISRTPEVTCVVVAVSHEDPEVKFNWYVDGVEVHNAKTKPREEQYGSTYRVVSVLTVLHQDWLNGKEYKCKVSNKALPAPIEKTISKAKGQPREPQVYTLPPSRDELTKNQVSLSCAVKGFYPSDIAVEWESNGQPENNYKTTPPVLDSDGSFFLVSKLTVDKSRWQQGNVFSCSVMHEALHNHYTQKSLSLSPGK

SEQ ID NO: 22 - protein, 447 aa, synthetic construct
  REGION 1..447: note = anti-mu FAP HC mu IgG2a Fc knob DANG
QVQLQQSGAELARPGASVNLSCKASGYTFTNNGINWLKQRTGQGLEWIGEIYPRSTNTLYNEKFKGKATLTADRSSNTAYMELRSLTSEDSAVYFCARTLTAPFAFWGQGTLVTVSAAKTTAPSVYPLAPVCGDTTGSSVTLGCLVKGYFPEPVTLTWNSGSLSSGVHTFPAVLQSDLYTLSSSVTVTSSTWPSQSITCNVAHPASSTKVDKKIEPRGPTIKPCPPCKCPAPNLLGGPSVFIFPPKIKDVLMISLSPIVTCVVVAVSEDDPDVQISWFVNNVEVHTAQTQTHREDYGSTLRVVSALPIQHQDWMSGKEFKCKVNNKDLPAPIERTISKPKGSVRAPQVYVLPPPEEEMTKKQVTLWCMVTDFMPEDIYVEWTNNGKTELNYKNTEPVLDSDGSYFMYSKLRVEKKNWVERNSYSCSVVHEGLHNHHTTKSFSRTPGK

SEQ ID NO: 23 - protein, 213 aa, synthetic construct
  REGION 1..213: note = anti-mu FAP LC
QIVLTQSPAIMSASPGEKVTMTCSASSGVNFMHWYQQKSGTSPKRWIFDTSKLASGVPARFSGSGSGTSYSLTISSMEAEDAATYYCQQWSFNPPTFGGGTKLEIKRADAAPTVSIFPPSSEQLTSGGASVVCFLNNFYPKDINVKWKIDGSERQNGVLNSWTDQDSKDSTYSMSSTLTLTKDEYERHNSYTCEATHKTSTSPIVKSFNRNEC

SEQ ID NO: 24 - protein, 696 aa, synthetic construct
  REGION 1..696: note = mu scLIGHT3-mu IgG2a Fc hole DANG
NPAAHLTGANASLIGIGGPLLWETRLGLAFLRGLTYHDGALVTMEPGYYYVYSKVQLSGVGCPQGLANGLPITHGLYKRTSRYPKELELLVSRRSPCGRANSSRVWWDSSFLGGVVHLEAGEEVVVRVPGNRLVRPRDGTRSYFGAFMVGGSGNPAAHLTGANASLIGIGGPLLWETRLGLAFLRGLTYHDGALVTMEPGYYYVYSKVQLSGVGCPQGLANGLPITHGLYKRTSRYPKELELLVSRRSPCGRANSSRVWWDSSFLGGVVHLEAGEEVVVRVPGNRLVRPRDGTRSYFGAFMVGGSGNPAAHLTGANASLIGIGGPLLWETRLGLAFLRGLTYHDGALVTMEPGYYYVYSKVQLSGVGCPQGLANGLPITHGLYKRTSRYPKELELLVSRRSPCGRANSSRVWWDSSFLGGVVHLEAGEEVVVRVPGNRLVRPRDGTRSYFGAFMVGGSGGGGSEPRGPTIKPCPPCKCPAPNLLGGPSVFIFPPKIKDVLMISLSPIVTCVVVAVSEDDPDVQISWFVNNVEVHTAQTQTHREDYGSTLRVVSALPIQHQDWMSGKEFKCKVNNKDLPAPIERTISKPKGSVRAPQVYVLPPPEEEMTKKQVTLSCAVTDFMPEDIYVEWTNNGKTELNYKNTEPVLDSDGSYFMVSKLRVEKKNWVERNSYSCSVVHEGLHNHHTTKSFSRTPGK

SEQ ID NO: 25 - protein, 460 aa, synthetic construct
  REGION 1..460: note = anti-mu FAP HC mu IgG2a Fc knob
QVQLQQSGAELARPGASVNLSCKASGYTFTNNGINWLKQRTGQGLEWIGEIYPRSTNTLYNEKFKGKATLTADRSSNTAYMELRSLTSEDSAVYFCARTLTAPFAFWGQGTLVTVSAAKTTAPSVYPLAPAKTTAPSVYPLAPVCGDTTGSSVTLGCLVKGYFPEPVTLTWNSGSLSSGVHTFPAVLQSDLYTLSSSVTVTSSTWPSQSITCNVAHPASSTKVDKKIEPRGPTIKPCPPCKCPAPNLLGGPSVFIFPPKIKDVLMISLSPIVTCVVVDVSEDDPDVQISWFVNNVEVHTAQTQTHREDYNSTLRVVSALPIQHQDWMSGKEFKCKVNNKDLPAPIERTISKPKGSVRAPQVYVLPPPEEEMTKKQVTLWCMVTDFMPEDIYVEWTNNGKTELNYKNTEPVLDSDGSYFMYSKLRVEKKNWVERNSYSCSVVHEGLHNHHTTKSFSRTPGK

SEQ ID NO: 26 - protein, 696 aa, synthetic construct
  REGION 1..696: note = mu scLIGHT3-mu IgG2a Fc hole
NPAAHLTGANASLIGIGGPLLWETRLGLAFLRGLTYHDGALVTMEPGYYYVYSKVQLSGVGCPQGLANGLPITHGLYKRTSRYPKELELLVSRRSPCGRANSSRVWWDSSFLGGVVHLEAGEEVVVRVPGNRLVRPRDGTRSYFGAFMVGGSGNPAAHLTGANASLIGIGGPLLWETRLGLAFLRGLTYHDGALVTMEPGYYYVYSKVQLSGVGCPQGLANGLPITHGLYKRTSRYPKELELLVSRRSPCGRANSSRVWWDSSFLGGVVHLEAGEEVVVRVPGNRLVRPRDGTRSYFGAFMVGGSGNPAAHLTGANASLIGIGGPLLWETRLGLAFLRGLTYHDGALVTMEPGYYYVYSKVQLSGVGCPQGLANGLPITHGLYKRTSRYPKELELLVSRRSPCGRANSSRVWWDSSFLGGVVHLEAGEEVVVRVPGNRLVRPRDGTRSYFGAFMVGGSGGGGSEPRGPTIKPCPPCKCPAPNLLGGPSVFIFPPKIKDVLMISLSPIVTCVVVDVSEDDPDVQISWFVNNVEVHTAQTQTHREDYNSTLRVVSALPIQHQDWMSGKEFKCKVNNKDLPAPIERTISKPKGSVRAPQVYVLPPPEEEMTKKQVTLSCAVTDFMPEDIYVEWTNNGKTELNYKNTEPVLDSDGSYFMVSKLRVEKKNWVERNSYSCSVVHEGLHNHHTTKSFSRTPGK

SEQ ID NO: 27 - protein, 696 aa, synthetic construct
  REGION 1..696: note = mu scLIGHT(225-230)3-mu IgG2a Fc hole DANG
NPAAHLTGANASLIGIGGPLLWETRLGLAFLRGLTYHDGALVTMEPGYYYVYSKVQLSGVGCPQGLANGLPITHGLYKRTSRYPKELELLVSRRSPCGRANSSRVWWDSSFLGGVVHLEAGEEVVVRVPGNRLVDYTKEDRSYFGAFMVGGSGNPAAHLTGANASLIGIGGPLLWETRLGLAFLRGLTYHDGALVTMEPGYYYVYSKVQLSGVGCPQGLANGLPITHGLYKRTSRYPKELELLVSRRSPCGRANSSRVWWDSSFLGGVVHLEAGEEVVVRVPGNRLVDYTKEDRSYFGAFMVGGSGNPAAHLTGANASLIGIGGPLLWETRLGLAFLRGLTYHDGALVTMEPGYYYVYSKVQLSGVGCPQGLANGLPITHGLYKRTSRYPKELELLVSRRSPCGRANSSRVWWDSSFLGGVVHLEAGEEVVVRVPGNRLVDYTKEDRSYFGAFMVGGSGGGGSEPRGPTIKPCPPCKCPAPNLLGGPSVFIFPPKIKDVLMISLSPIVTCVVVAVSEDDPDVQISWFVNNVEVHTAQTQTHREDYGSTLRVVSALPIQHQDWMSGKEFKCKVNNKDLPAPIERTISKPKGSVRAPQVYVLPPPEEEMTKKQVTLSCAVTDFMPEDIYVEWTNNGKTELNYKNTEPVLDSDGSYFMVSKLRVEKKNWVERNSYSCSVVHEGLHNHHTTKSFSRTPGK

SEQ ID NO: 28 - protein, 696 aa, synthetic construct; identical to SEQ ID NO: 27
  REGION 1..696: note = mu scLIGHT(194-197)3-mu IgG2a Fc hole DANG

SEQ ID NO: 29 - protein, 759 aa, synthetic construct
  REGION 1..759: note = anti-mu FAP HC mu IgG2a Fc knob DANG-mu scLIGHT2
QVQLQQSGAELARPGASVNLSCKASGYTFTNNGINWLKQRTGQGLEWIGEIYPRSTNTLYNEKFKGKATLTADRSSNTAYMELRSLTSEDSAVYFCARTLTAPFAFWGQGTLVTVSAAKTTAPSVYPLAPVCGDTTGSSVTLGCLVKGYFPEPVTLTWNSGSLSSGVHTFPAVLQSDLYTLSSSVTVTSSTWPSQSITCNVAHPASSTKVDKKIEPRGPTIKPCPPCKCPAPNLLGGPSVFIFPPKIKDVLMISLSPIVTCVVVAVSEDDPDVQISWFVNNVEVHTAQTQTHREDYGSTLRVVSALPIQHQDWMSGKEFKCKVNNKDLPAPIERTISKPKGSVRAPQVYVLPPPEEEMTKKQVTLWCMVTDFMPEDIYVEWTNNGKTELNYKNTEPVLDSDGSYFMYSKLRVEKKNWVERNSYSCSVVHEGLHNHHTTKSFSRTPGKGGGGSGGGGSNPAAHLTGANASLIGIGGPLLWETRLGLAFLRGLTYHDGALVTMEPGYYYVYSKVQLSGVGCPQGLANGLPITHGLYKRTSRYPKELELLVSRRSPCGRANSSRVWWDSSFLGGVVHLEAGEEVVVRVPGNRLVRPRDGTRSYFGAFMVGGSGNPAAHLTGANASLIGIGGPLLWETRLGLAFLRGLTYHDGALVTMEPGYYYVYSKVQLSGVGCPQGLANGLPITHGLYKRTSRYPKELELLVSRRSPCGRANSSRVWWDSSFLGGVVHLEAGEEVVVRVPGNRLVRPRDGTRSYFGAFMV

SEQ ID NO: 30 - protein, 606 aa, synthetic construct
  REGION 1..606: note = anti-mu FAP HC mu IgG2a Fc hole DANG-mu LIGHT
QVQLQQSGAELARPGASVNLSCKASGYTFTNNGINWLKQRTGQGLEWIGEIYPRSTNTLYNEKFKGKATLTADRSSNTAYMELRSLTSEDSAVYFCARTLTAPFAFWGQGTLVTVSAAKTTAPSVYPLAPVCGDTTGSSVTLGCLVKGYFPEPVTLTWNSGSLSSGVHTFPAVLQSDLYTLSSSVTVTSSTWPSQSITCNVAHPASSTKVDKKIEPRGPTIKPCPPCKCPAPNLLGGPSVFIFPPKIKDVLMISLSPIVTCVVVAVSEDDPDVQISWFVNNVEVHTAQTQTHREDYGSTLRVVSALPIQHQDWMSGKEFKCKVNNKDLPAPIERTISKPKGSVRAPQVYVLPPPEEEMTKKQVTLSCAVTDFMPEDIYVEWTNNGKTELNYKNTEPVLDSDGSYFMVSKLRVEKKNWVERNSYSCSVVHEGLHNHHTTKSFSRTPGKGGGGSGGGGSNPAAHLTGANASLIGIGGPLLWETRLGLAFLRGLTYHDGALVTMEPGYYYVYSKVQLSGVGCPQGLANGLPITHGLYKRTSRYPKELELLVSRRSPCGRANSSRVWWDSSFLGGVVHLEAGEEVVVRVPGNRLVRPRDGTRSYFGAFMV

SEQ ID NO: 31 - protein, 605 aa, synthetic construct
  REGION 1..605: note = anti-mu FAP HC mu IgG2a Fc DANG-mu LIGHT
QVQLQQSGAELARPGASVNLSCKASGYTFTNNGINWLKQRTGQGLEWIGEIYPRSTNTLYNEKFKGKATLTADRSSNTAYMELRSLTSEDSAVYFCARTLTAPFAFWGQGTLVTVSAAKTTAPSVYPLAPVCGDTTGSSVTLGCLVKGYFPEPVTLTWNSGSLSSGVHTFPAVLQSDLYTLSSSVTVTSSTWPSQSITCNVAHPASSTKVDKKIEPRGPTIKPCPPCKCPAPNLLGGPSVFIFPPKIKDVLMISLSPIVTCVVVAVSEDDPDVQISWFVNNVEVHTAQTQTHREDYGSTLRVVSALPIQHQDWMSGKEFKCKVNNKDLPAPIERTISKPKGSVRAPQVYVLPPPEEEMTKKQVTLTCMVTDFMPEDIYVEWTNNGKTELNYKNTEPVLDSDGSYFMYSKLRVEKKNWVERNSYSCSVVHEGLHNHHTTKSFSRTPGGGGGSGGGGSNPAAHLTGANASLIGIGGPLLWETRLGLAFLRGLTYHDGALVTMEPGYYYVYSKVQLSGVGCPQGLANGLPITHGLYKRTSRYPKELELLVSRRSPCGRANSSRVWWDSSFLGGVVHLEAGEEVVVRVPGNRLVRPRDGTRSYFGAFMV

SEQ ID NO: 32 - protein, 233 aa, synthetic construct
  REGION 1..233: note = mu IgG2a Fc hole DANG
EPRGPTIKPCPPCKCPAPNLLGGPSVFIFPPKIKDVLMISLSPIVTCVVVAVSEDDPDVQISWFVNNVEVHTAQTQTHREDYGSTLRVVSALPIQHQDWMSGKEFKCKVNNKDLPAPIERTISKPKGSVRAPQVYVLPPPEEEMTKKQVTLSCAVTDFMPEDIYVEWTNNGKTELNYKNTEPVLDSDGSYFMVSKLRVEKKNWVERNSYSCSVVHEGLHNHHTTKSFSRTPGK

SEQ ID NO: 33 - protein, 233 aa, synthetic construct
  REGION 1..233: note = mu IgG2a Fc knob DANG
EPRGPTIKPCPPCKCPAPNLLGGPSVFIFPPKIKDVLMISLSPIVTCVVVAVSEDDPDVQISWFVNNVEVHTAQTQTHREDYGSTLRVVSALPIQHQDWMSGKEFKCKVNNKDLPAPIERTISKPKGSVRAPQVYVLPPPEEEMTKKQVTLWCMVTDFMPEDIYVEWTNNGKTELNYKNTEPVLDSDGSYFMYSKLRVEKKNWVERNSYSCSVVHEGLHNHHTTKSFSRTPGK

SEQ ID NO: 34 - protein, 233 aa, synthetic construct
  REGION 1..233: note = mu IgG2a Fc knob
EPRGPTIKPCPPCKCPAPNLLGGPSVFIFPPKIKDVLMISLSPIVTCVVVDVSEDDPDVQISWFVNNVEVHTAQTQTHREDYNSTLRVVSALPIQHQDWMSGKEFKCKVNNKDLPAPIERTISKPKGSVRAPQVYVLPPPEEEMTKKQVTLWCMVTDFMPEDIYVEWTNNGKTELNYKNTEPVLDSDGSYFMYSKLRVEKKNWVERNSYSCSVVHEGLHNHHTTKSFSRTPGK

SEQ ID NO: 35 - protein, 447 aa, synthetic construct
  REGION 1..447: note = anti-mu FAP HC mu IgG2a Fc DANG
QVQLQQSGAELARPGASVNLSCKASGYTFTNNGINWLKQRTGQGLEWIGEIYPRSTNTLYNEKFKGKATLTADRSSNTAYMELRSLTSEDSAVYFCARTLTAPFAFWGQGTLVTVSAAKTTAPSVYPLAPVCGDTTGSSVTLGCLVKGYFPEPVTLTWNSGSLSSGVHTFPAVLQSDLYTLSSSVTVTSSTWPSQSITCNVAHPASSTKVDKKIEPRGPTIKPCPPCKCPAPNLLGGPSVFIFPPKIKDVLMISLSPIVTCVVVAVSEDDPDVQISWFVNNVEVHTAQTQTHREDYGSTLRVVSALPIQHQDWMSGKEFKCKVNNKDLPAPIERTISKPKGSVRAPQVYVLPPPEEEMTKKQVTLTCMVTDFMPEDIYVEWTNNGKTELNYKNTEPVLDSDGSYFMYSKLRVEKKNWVERNSYSCSVVHEGLHNHHTTKSFSRTPGK

SEQ ID NO: 36 - protein, 715 aa, synthetic construct
  REGION 1..715: note = mu scLIGHT-LTb2-mu IgG2a Fc hole DANG
NPAAHLTGANASLIGIGGPLLWETRLGLAFLRGLTYHDGALVTMEPGYYYVYSKVQLSGVGCPQGLANGLPITHGLYKRTSRYPKELELLVSRRSPCGRANSSRVWWDSSFLGGVVHLEAGEEVVVRVPGNRLVRPRDGTRSYFGAFMVGGGGSGGGGSGGGGSLPAAHLIGAWMSGQGLSWEASQEEAFLRSGAQFSPTHGLALPQDGVYYLYCHVGYRGRTPPAGRSRARSLTLRSALYRAGGAYGRGSPELLLEGAETVTPVVDPIGYGSLWYTSVGFGGLAQLRSGERVYVNISHPDMVDYRRGKTFFGAVMVGGSGLPAAHLIGAWMSGQGLSWEASQEEAFLRSGAQFSPTHGLALPQDGVYYLYCHVGYRGRTPPAGRSRARSLTLRSALYRAGGAYGRGSPELLLEGAETVTPVVDPIGYGSLWYTSVGFGGLAQLRSGERVYVNISHPDMVDYRRGKTFFGAVMVGGSGGGGSEPRGPTIKPCPPCKCPAPNLLGGPSVFIFPPKIKDVLMISLSPIVTCVVVAVSEDDPDVQISWFVNNVEVHTAQTQTHREDYGSTLRVVSALPIQHQDWMSGKEFKCKVNNKDLPAPIERTISKPKGSVRAPQVYVLPPPEEEMTKKQVTLSCAVTDFMPEDIYVEWTNNGKTELNYKNTEPVLDSDGSYFMVSKLRVEKKNWVERNSYSCSVVHEGLHNHHTTKSFSRTPGK

SEQ ID NO: 37 - protein, 715 aa, synthetic construct
  REGION 1..715: note = mu scLIGHT-LTb2-mu IgG2a Fc hole
NPAAHLTGANASLIGIGGPLLWETRLGLAFLRGLTYHDGALVTMEPGYYYVYSKVQLSGVGCPQGLANGLPITHGLYKRTSRYPKELELLVSRRSPCGRANSSRVWWDSSFLGGVVHLEAGEEVVVRVPGNRLVRPRDGTRSYFGAFMVGGGGSGGGGSGGGGSLPAAHLIGAWMSGQGLSWEASQEEAFLRSGAQFSPTHGLALPQDGVYYLYCHVGYRGRTPPAGRSRARSLTLRSALYRAGGAYGRGSPELLLEGAETVTPVVDPIGYGSLWYTSVGFGGLAQLRSGERVYVNISHPDMVDYRRGKTFFGAVMVGGSGLPAAHLIGAWMSGQGLSWEASQEEAFLRSGAQFSPTHGLALPQDGVYYLYCHVGYRGRTPPAGRSRARSLTLRSALYRAGGAYGRGSPELLLEGAETVTPVVDPIGYGSLWYTSVGFGGLAQLRSGERVYVNISHPDMVDYRRGKTFFGAVMVGGSGGGGSEPRGPTIKPCPPCKCPAPNLLGGPSVFIFPPKIKDVLMISLSPIVTCVVVDVSEDDPDVQISWFVNNVEVHTAQTQTHREDYNSTLRVVSALPIQHQDWMSGKEFKCKVNNKDLPAPIERTISKPKGSVRAPQVYVLPPPEEEMTKKQVTLSCAVTDFMPEDIYVEWTNNGKTELNYKNTEPVLDSDGSYFMVSKLRVEKKNWVERNSYSCSVVHEGLHNHHTTKSFSRTPGK

SEQ ID NO: 38 - DNA, 1362 bp, synthetic construct
  misc_feature 1..1362: note = DNA sequence of anti-hu FAP HC hu IgG1 Fc knob DANG
  source 1..1362: mol_type = other DNA
caggtgcagctggtgcagtccggagcagaggtgaagaagccaggagcctctgtgaaggtgagctgcaagacctccagatacaccttcacagagtatacaatccactgggtgcgccaggcacctggacagcggctggagtggatcggaggcatcaaccccaacaatggcatccctaactacaatcagaagtttaagggcagagtgaccatcacagtggacacctccgcctctacagcctatatggagctgagctccctgaggagcgaggataccgccgtgtactattgcgcccggagaaggatcgcctacggctatgacgagggccacgccatggattactggggccagggcaccctggtgacagtgtctagcgcctctaccaagggaccaagcgtgttcccactggcaccatcctctaagagcacctccggaggaacagccgccctgggctgtctggtgaaggactatttcccagagcccgtgacagtgtcctggaactctggcgccctgacctccggagtgcacacatttcctgccgtgctgcagagctccggcctgtacagcctgtctagcgtggtgaccgtgccatcctctagcctgggcacccagacatatatctgcaacgtgaatcacaagcctagcaatacaaaggtggacaagaaggtggagccaaagtcctgtgataagacccacacatgccccccttgtcctgcaccagagctgctgggaggaccaagcgtgttcctgtttccacccaagcccaaggacaccctgatgatctctcgcaccccagaggtgacatgcgtggtggtggccgtgagccacgaggaccccgaggtgaagtttaactggtacgtggatggcgtggaggtgcacaatgccaagaccaagccaagagaggagcagtacggctccacctatagggtggtgtctgtgctgacagtgctgcaccaggattggctgaacggcaaggagtataagtgcaaggtgtccaataaggccctgcccgcccctatcgagaagaccatctctaaggcaaagggacagcctagggagccacaggtgtacaccctgcctccatcccgggacgagctgacaaagaaccaggtgtctctgtggtgtctggtgaagggcttctatccctctgatatcgccgtggagtgggagagcaatggccagcctgagaacaattacaagaccacaccccctgtgctggacagcgatggctccttctttctgtatagcaagctgaccgtggataagtcccggtggcagcagggcaacgtgttttcttgtagcgtgatgcacgaggccctgcacaatcactacacacagaagtccctgtctctgagccctggcaag

SEQ ID NO: 39 - DNA, 660 bp, synthetic construct
  misc_feature 1..660: note = DNA sequence of anti-hu FAP LC
  source 1..660: mol_type = other DNA
gacatcgtgatgacccagtcccctgattctctggccgtgagcctgggagagagggcaacaatcaactgcaagagctcccagagcctgctgtactcccgcaaccagaagaattacctggcctggtatcagcagaagcccggccagccccctaagctgctgatcttctgggcatctaccagggagagcggagtgcctgacagattttctggcagcggcttcggcacagacttcaccctgacaatctctagcctgcaggccgaggacgtggccgtgtactattgccagcagtacttctcctatcctctgacctttggccagggcacaaaggtggagatcaagaggaccgtggcagcaccaagcgtgttcatctttccaccctccgacgagcagctgaagtccggcaccgcctctgtggtgtgcctgctgaacaatttctacccaagggaggccaaggtgcagtggaaggtggataacgccctgcagagcggcaattcccaggagtctgtgaccgagcaggacagcaaggattccacatattctctgtcctctaccctgacactgtctaaggccgattacgagaagcacaaggtgtatgcatgcgaggtgacccaccagggactgagctccccagtgacaaagtcctttaatcggggcgagtgt

SEQ ID NO: 40 - DNA, 2079 bp, synthetic construct
  misc_feature 1..2079: note = DNA sequence of hu scLIGHT3-hu IgG1 Fc hole DANG
  source 1..2079: mol_type = other DNA
gaggtgaacccagcagcacacctgaccggagccaatagctccctgacaggctccggaggaccactgctgtgggagacccagctgggactggccttcctgaggggactgtcttatcacgacggcgccctggtggtgacaaaggcaggctactattacatctactccaaggtgcagctgggaggagtgggatgcccactgggactggcctctaccatcacacacggcctgtataagaggaccccaaggtaccctgaggagctggagctgctggtgtcccagcagtctccctgtggcagggccacatctagctcccgcgtgtggtgggattctagcttcctgggaggagtggtgcacctggaggcaggagagaaggtggtggtgcgggtgctggacgagagactggtgcggctgagagatggcacccggtcttacttcggagcctttatggtgggaggcagcggagaggtgaaccctgccgcccacctgactggcgccaattcctctctgacaggcagcggcggccctctgctgtgggaaactcagctgggcctggcctttctgagaggcctgtcctaccatgatggcgccctggtcgtgacaaaggcaggctattactatatctacagtaaagtccagctgggcggagtgggatgccctctgggactggcctccactattacccatggcctgtataagcggaccccaagataccccgaagaactggagctgctggtgagccagcagtccccatgtggaagggccacaagctcctctagagtgtggtgggatagctccttcctgggcggcgtcgtccacctggaggcaggcgagaaggtggtggtgagggtgctggacgagcgcctggtgaggctgagggatggaaccaggtcctacttcggcgcctttatggtcggcggctctggagaggtgaacccagcagcccacctgaccggcgccaattctagcctgacaggcagcggaggacctctgctgtgggaaacacagctgggactggcctttctgaggggactgtcctaccatgacggcgccctggtcgtcaccaaagccggatactattacatctactctaaagtccagctggggggcgtcggctgcccactgggactggcaagcactattacccacggactgtataagaggacccctcgctacccagaagaactggaactgctggtgtctcagcagagcccttgtggcagggccacatcctctagtcgcgtgtggtgggactcctctttcctgggcggcgtcgtgcacctggaagccggcgaaaaagtcgtggtgcgggtgctggatgagagactggtgcggttaagagatggcacccggagctatttcggcgcctttatggtgggcggcagcggaggaggaggctccgacaagacccacacatgcccaccttgtccagcaccagagctgctgggaggaccatccgtgttcctgtttccacccaagcccaaggataccctgatgatcagcagaaccccagaggtgacatgcgtggtcgtggccgtgtcccacgaggaccctgaggtgaagtttaactggtacgtggatggcgtggaggtgcacaatgccaagacaaagccccgggaggagcagtatggctctacctacagagtggtgagcgtgctgacagtgctgcaccaggactggctgaacggcaaggagtataagtgcaaggtgtctaataaggccctgcctgccccaatcgagaagaccatcagcaaggcaaagggacagccaagggagcctcaggtgtacaccctgcctccaagccgcgacgagctgacaaagaaccaggtgagcctgtcctgtgccgtgaagggcttctatcctagcgatatcgccgtggagtgggagtccaatggccagccagagaacaattacaagaccacaccccctgtgctggactccgatggctctttctttctggtgtccaagctgaccgtggataagtctcggtggcagcagggcaacgtgttttcttgtagcgtgatgcacgaggccctgcacaatcactacacacagaagtccctgtctctgagccccggcaag

SEQ ID NO: 41 - DNA, 1362 bp, synthetic construct
  misc_feature 1..1362: note = anti-hu FAP HC hu IgG1 Fc knob
  source 1..1362: mol_type = other DNA
caggtgcagctggtgcagtccggagcagaggtgaagaagccaggagcctctgtgaaggtgagctgcaagacctccagatacaccttcacagagtatacaatccactgggtgcgccaggcacctggacagcggctggagtggatcggaggcatcaaccccaacaatggcatccctaactacaatcagaagtttaagggcagagtgaccatcacagtggacacctccgcctctacagcctatatggagctgagctccctgaggagcgaggataccgccgtgtactattgcgcccggagaaggatcgcctacggctatgacgagggccacgccatggattactggggccagggcaccctggtgacagtgtctagcgcctctaccaagggaccaagcgtgttcccactggcaccatcctctaagagcacctccggaggaacagccgccctgggctgtctggtgaaggactatttcccagagcccgtgacagtgtcctggaactctggcgccctgacctccggagtgcacacatttcctgccgtgctgcagagctccggcctgtacagcctgtctagcgtggtgaccgtgccatcctctagcctgggcacccagacatatatctgcaacgtgaatcacaagcctagcaatacaaaggtggacaagaaggtggagccaaagtcctgtgataagacccacacatgccccccttgtcctgcaccagagctgctgggaggaccaagcgtgttcctgtttccacccaagcccaaggacaccctgatgatctctcgcaccccagaggtgacatgcgtggtggtggacgtgagccacgaggaccccgaggtgaagtttaactggtacgtggatggcgtggaggtgcacaatgccaagaccaagccaagagaggagcagtacaactccacctatagggtggtgtctgtgctgacagtgctgcaccaggattggctgaacggcaaggagtataagtgcaaggtgtccaataaggccctgcccgcccctatcgagaagaccatctctaaggcaaagggacagcctagggagccacaggtgtacaccctgcctccatcccgggacgagctgacaaagaaccaggtgtctctgtggtgtctggtgaagggcttctatccctctgatatcgccgtggagtgggagagcaatggccagcctgagaacaattacaagaccacaccccctgtgctggacagcgatggctccttctttctgtatagcaagctgaccgtggataagtcccggtggcagcagggcaacgtgttttcttgtagcgtgatgcacgaggccctgcacaatcactacacacagaagtccctgtctctgagccctggcaag

SEQ ID NO: 42 - DNA, 2079 bp, synthetic construct
  misc_feature 1..2079: note = DNA sequence of hu scLIGHT3-hu IgG1 Fc hole
  source 1..2079: mol_type = other DNA
gaggtgaacccagcagcacacctgaccggagccaatagctccctgacaggctccggaggaccactgctgtgggagacccagctgggactggccttcctgaggggactgtcttatcacgacggcgccctggtggtgacaaaggcaggctactattacatctactccaaggtgcagctgggaggagtgggatgcccactgggactggcctctaccatcacacacggcctgtataagaggaccccaaggtaccctgaggagctggagctgctggtgtcccagcagtctccctgtggcagggccacatctagctcccgcgtgtggtgggattctagcttcctgggaggagtggtgcacctggaggcaggagagaaggtggtggtgcgggtgctggacgagagactggtgcggctgagagatggcacccggtcttacttcggagcctttatggtgggaggcagcggagaggtgaaccctgccgcccacctgactggcgccaattcctctctgacaggcagcggcggccctctgctgtgggaaactcagctgggcctggcctttctgagaggcctgtcctaccatgatggcgccctggtcgtgacaaaggcaggctattactatatctacagtaaagtccagctgggcggagtgggatgccctctgggactggcctccactattacccatggcctgtataagcggaccccaagataccccgaagaactggagctgctggtgagccagcagtccccatgtggaagggccacaagctcctctagagtgtggtgggatagctccttcctgggcggcgtcgtccacctggaggcaggcgagaaggtggtggtgagggtgctggacgagcgcctggtgaggctgagggatggaaccaggtcctacttcggcgcctttatggtcggcggctctggagaggtgaacccagcagcccacctgaccggcgccaattctagcctgacaggcagcggaggacctctgctgtgggaaacacagctgggactggcctttctgaggggactgtcctaccatgacggcgccctggtcgtcaccaaagccggatactattacatctactctaaagtccagctggggggcgtcggctgcccactgggactggcaagcactattacccacggactgtataagaggacccctcgctacccagaagaactggaactgctggtgtctcagcagagcccttgtggcagggccacatcctctagtcgcgtgtggtgggactcctctttcctgggcggcgtcgtgcacctggaagccggcgaaaaagtcgtggtgcgggtgctggatgagagactggtgcggttaagagatggcacccggagctatttcggcgcctttatggtgggcggcagcggaggaggaggctccgacaagacccacacatgcccaccttgtccagcaccagagctgctgggaggaccatccgtgttcctgtttccacccaagcccaaggataccctgatgatcagcagaaccccagaggtgacatgcgtggtcgtggacgtgtcccacgaggaccctgaggtgaagtttaactggtacgtggatggcgtggaggtgcacaatgccaagacaaagccccgggaggagcagtataactctacctacagagtggtgagcgtgctgacagtgctgcaccaggactggctgaacggcaaggagtataagtgcaaggtgtctaataaggccctgcctgccccaatcgagaagaccatcagcaaggcaaagggacagccaagggagcctcaggtgtacaccctgcctccaagccgcgacgagctgacaaagaaccaggtgagcctgtcctgtgccgtgaagggcttctatcctagcgatatcgccgtggagtgggagtccaatggccagccagagaacaattacaagaccacaccccctgtgctggactccgatggctctttctttctggtgtccaagctgaccgtggataagtctcggtggcagcagggcaacgtgttttcttgtagcgtgatgcacgaggccctgcacaatcactacacacagaagtccctgtctctgagccccggcaag

SEQ ID NO: 43 - DNA, 2211 bp, synthetic construct
  misc_feature 1..2211: note = DNA sequence of hu scLIGHT3(GGGGS4)-hu IgG1 Fc hole DANG
  source 1..2211: mol_type = other DNA
gaggtgaacccagcagcacacctgaccggagccaatagctccctgacaggctccggaggaccactgctgtgggagacccagctgggactggccttcctgaggggactgtcttatcacgacggcgccctggtggtgacaaaggcaggctactattacatctactccaaggtgcagctgggaggagtgggatgcccactgggactggcctctaccatcacacacggcctgtataagaggaccccaaggtaccctgaggagctggagctgctggtgtcccagcagtctccctgtggcagggccacatctagctcccgcgtgtggtgggattctagcttcctgggaggagtggtgcacctggaggcaggagagaaggtggtggtgcgggtgctggacgagagactggtgcggctgagagatggcacccggtcttacttcggagcctttatggtgggcggaggcgggtctggaggtggagggagtggaggaggggggagcggtgggggaggtagcgaggtgaaccctgccgcccacctgactggcgccaattcctctctgacaggcagcggcggccctctgctgtgggaaactcagctgggcctggcctttctgagaggcctgtcctaccatgatggcgccctggtcgtgacaaaggcaggctattactatatctacagtaaagtccagctgggcggagtgggatgccctctgggactggcctccactattacccatggcctgtataagcggaccccaagataccccgaagaactggagctgctggtgagccagcagtccccatgtggaagggccacaagctcctctagagtgtggtgggatagctccttcctgggcggcgtcgtccacctggaggcaggcgagaaggtggtggtgagggtgctggacgagcgcctggtgaggctgagggatggaaccaggtcctacttcggcgcctttatggtcggtgggggaggtagcggcggaggcgggtctggaggtggagggagtggaggaggggggagcgaggtgaacccagcagcccacctgaccggcgccaattctagcctgacaggcagcggaggacctctgctgtgggaaacacagctgggactggcctttctgaggggactgtcctaccatgacggcgccctggtcgtcaccaaagccggatactattacatctactctaaagtccagctggggggcgtcggctgcccactgggactggcaagcactattacccacggactgtataagaggacccctcgctacccagaagaactggaactgctggtgtctcagcagagcccttgtggcagggccacatcctctagtcgcgtgtggtgggactcctctttcctgggcggcgtcgtgcacctggaagccggcgaaaaagtcgtggtgcgggtgctggatgagagactggtgcggttaagagatggcacccggagctatttcggcgcctttatggtgggaggaggaggaagcggcggaggcggatccggaggaggcggcagcggaggaggaggctccgacaagacccacacatgcccaccttgtccagcaccagagctgctgggaggaccatccgtgttcctgtttccacccaagcccaaggataccctgatgatcagcagaaccccagaggtgacatgcgtggtcgtggccgtgtcccacgaggaccctgaggtgaagtttaactggtacgtggatggcgtggaggtgcacaatgccaagacaaagccccgggaggagcagtatggctctacctacagagtggtgagcgtgctgacagtgctgcaccaggactggctgaacggcaaggagtataagtgcaaggtgtctaataaggccctgcctgccccaatcgagaagaccatcagcaaggcaaagggacagccaagggagcctcaggtgtacaccctgcctccaagccgcgacgagctgacaaagaaccaggtgagcctgtcctgtgccgtgaagggcttctatcctagcgatatcgccgtggagtgggagtccaatggccagccagagaacaattacaagaccacaccccctgtgctggactccgatggctctttctttctggtgtccaagctgaccgtggataagtctcggtggcagcagggcaacgtgttttcttgtagcgtgatgcacgaggccctgcacaatcactacacacagaagtccctgtctctgagccccggcaag

SEQ ID NO: 44 - DNA, 2079 bp, synthetic construct
  misc_feature 1..2079: note = DNA sequence of hu scLIGHT(226-231)3-hu IgG1 Fc hole DANG
  source 1..2079: mol_type = other DNA
gaggtcaaccccgcagcccacctgacgggagccaacagtagcctgaccgggagcggcggtcccctgctgtgggagactcagcttggcctggcatttctgcgaggtttgagctaccatgacggcgctcttgttgtgaccaaggcgggttactactacatctattcaaaggttcagctggggggtgtcggttgcccactgggtctcgcctcaaccatcacccacggcctgtataaaaggaccccgaggtacccggaggaacttgaattgcttgtgagccagcagagcccctgtggtcgggccacctcaagctcacgggtttggtgggattcctctttcctgggcggtgttgtgcatcttgaagccggtgagaaagtggtagtgagggtcctggacgagcgactcgtcgactataccaaggaggacaggtcatattttggcgcatttatggtaggaggatcaggagaggtgaacccagccgcccatctgactggggccaactcaagtcttaccggcagcggaggccccctgttgtgggaaacgcaattggggctggcgttcctgagggggctgagctatcacgacggtgccctggtggttaccaaagcgggctactattacatttatagcaaggtgcaacttggcggcgtcggctgccccttgggtctggcgagcacgattacccatggcctctacaagaggacgcccagataccccgaagagctggagttgctcgtgtcccagcagtcaccttgtggaagggcgacctccagttccagggtgtggtgggacagcagcttcttgggcggagtcgtccacctggaggcaggcgaaaaggtggtggtgagagtgcttgatgagaggctggtggactacactaaggaagatagaagctatttcggcgctttcatggtcggcggaagcggtgaggtaaatcccgctgctcatttgaccggcgccaattcctctctgaccggcagcggaggccctctgctgtgggagacccagctgggactggcttttctgaggggactctcctaccatgatggagctctggtcgtcaccaaggccggatactactacatctactccaaagtgcaactcggaggagtcggctgtcctctcggactggccagcacaattacccatggactgtacaaaaggacccctaggtaccccgaagaactggagctgctcgtgtcccaacaatccccttgcggaagagctacatccagctccagagtctggtgggacagctcctttctgggaggagtggtccacctcgaagccggcgagaaagtcgtggtcagagtgctggacgagagactcgtcgactataccaaagaggacagaagctactttggcgctttcatggtgggcggaagcggcggaggcggaagcgataagacacacacatgccctccttgccccgcccccgagctgctcggaggccctagcgtgtttctgttcccccccaagcccaaagacacactgatgatctccagaacccccgaggtgacatgcgtggtggtggctgtgtcccatgaggaccccgaagtcaagttcaactggtacgtcgacggcgtggaagtccacaacgccaagacaaagcctagagaggagcaatacggcagcacatatagggtcgtgagcgtgctgaccgtcctccaccaagactggctcaacggcaaggagtacaagtgcaaggtctccaataaagctctgcccgctcccatcgagaaaaccatcagcaaggccaaaggccagcctagggagccccaagtgtacacactgcctccctctagagacgagctgaccaagaatcaagtgtccctcagctgcgctgtcaagggcttctaccccagcgacattgccgtggaatgggagagcaacggccagcccgagaacaactataagaccaccccccccgtgctggattccgatggctccttctttctggtgagcaaactgacagtggacaagtctagatggcagcaaggcaacgtctttagctgcagcgtcatgcacgaggctctgcacaatcactacacccagaagtctctgtctctgagccccggcaaa

SEQ ID NO: 45 - DNA, 2079 bp, synthetic construct
  misc_feature 1..2079: note = DNA sequence of hu scLIGHT(195-198)3-hu IgG1 Fc hole DANG
  source 1..2079: mol_type = other DNA
gaggtcaaccccgcagcccacctgacgggagccaacagtagcctgaccgggagcggcggtcccctgctgtgggagactcagcttggcctggcatttctgcgaggtttgagctaccatgacggcgctcttgttgtgaccaaggcgggttactactacatctattcaaaggttcagctggggggtgtcggttgcccactgggtctcgcctcaaccatcacccacggcctgtataaaaggaccccgaggtacccggaggaacttgaattgcttgtgagccagcagagcccctgtggtcgggccacctcaagctcaagtaactggttcgattcctctttcctgggcggtgttgtgcatcttgaagccggtgagaaagtggtagtgagggtcctggacgagcgactcgtcagactgcgagatggcacgaggtcatattttggcgcatttatggtaggaggatcaggagaggtgaacccagccgcccatctgactggggccaactcaagtcttaccggcagcggaggccccctgttgtgggaaacgcaattggggctggcgttcctgagggggctgagctatcacgacggtgccctggtggttaccaaagcgggctactattacatttatagcaaggtgcaacttggcggcgtcggctgccccttgggtctggcgagcacgattacccatggcctctacaagaggacgcccagataccccgaagagctggagttgctcgtgtcccagcagtcaccttgtggaagggcgacctccagttccagcaactggtttgacagcagcttcttgggcggagtcgtccacctggaggcaggcgaaaaggtggtggtgagagtgcttgatgagaggctggtgaggctgagggacggcaccagaagctatttcggcgctttcatggtcggcggaagcggtgaggtaaatcccgctgctcatttgaccggcgccaattcctctctgaccggcagcggaggccctctgctgtgggagacccagctgggactggcttttctgaggggactctcctaccatgatggagctctggtcgtcaccaaggccggatactactacatctactccaaagtgcaactcggaggagtcggctgtcctctcggactggccagcacaattacccatggactgtacaaaaggacccctaggtaccccgaagaactggagctgctcgtgtcccaacaatccccttgcggaagagctacatccagctccagcaattggttcgacagctcctttctgggaggagtggtccacctcgaagccggcgagaaagtcgtggtcagagtgctggacgagagactcgtccgattgagggatggaaccagaagctactttggcgctttcatggtgggcggaagcggcggaggcggaagcgataagacacacacatgccctccttgccccgcccccgagctgctcggaggccctagcgtgtttctgttcccccccaagcccaaagacacactgatgatctccagaacccccgaggtgacatgcgtggtggtggctgtgtcccatgaggaccccgaagtcaagttcaactggtacgtcgacggcgtggaagtccacaacgccaagacaaagcctagagaggagcaatacggcagcacatatagggtcgtgagcgtgctgaccgtcctccaccaagactggctcaacggcaaggagtacaagtgcaaggtctccaataaagctctgcccgctcccatcgagaaaaccatcagcaaggccaaaggccagcctagggagccccaagtgtacacactgcctccctctagagacgagctgaccaagaatcaagtgtccctcagctgcgctgtcaagggcttctaccccagcgacattgccgtggaatgggagagcaacggccagcccgagaacaactataagaccaccccccccgtgctggattccgatggctccttctttctggtgagcaaactgacagtggacaagtctagatggcagcaaggcaacgtctttagctgcagcgtcatgcacgaggctctgcacaatcactacacccagaagtctctgtctctgagccccggcaaa

SEQ ID NO: 46 - DNA, 2304 bp, synthetic construct
  misc_feature 1..2304: note = DNA sequence of anti-hu FAP HC hu IgG1 Fc knob DANG-hu scLIGHT2
  source 1..2304: mol_type = other DNA
caggtgcagctggtgcagtccggagcagaggtgaagaagccaggagcctctgtgaaggtgagctgcaagacctccagatacaccttcacagagtatacaatccactgggtgcgccaggcacctggacagcggctggagtggatcggaggcatcaaccccaacaatggcatccctaactacaatcagaagtttaagggcagagtgaccatcacagtggacacctccgcctctacagcctatatggagctgagctccctgaggagcgaggataccgccgtgtactattgcgcccggagaaggatcgcctacggctatgacgagggccacgccatggattactggggccagggcaccctggtgacagtgtctagcgcctctaccaagggaccaagcgtgttcccactggcaccatcctctaagagcacctccggaggaacagccgccctgggctgtctggtgaaggactatttcccagagcccgtgacagtgtcctggaactctggcgccctgacctccggagtgcacacatttcctgccgtgctgcagagctccggcctgtacagcctgtctagcgtggtgaccgtgccatcctctagcctgggcacccagacatatatctgcaacgtgaatcacaagcctagcaatacaaaggtggacaagaaggtggagccaaagtcctgtgataagacccacacatgccccccttgtcctgcaccagagctgctgggaggaccaagcgtgttcctgtttccacccaagcccaaggacaccctgatgatctctcgcaccccagaggtgacatgcgtggtggtggccgtgagccacgaggaccccgaggtgaagtttaactggtacgtggatggcgtggaggtgcacaatgccaagaccaagccaagagaggagcagtacggctccacctatagggtggtgtctgtgctgacagtgctgcaccaggattggctgaacggcaaggagtataagtgcaaggtgtccaataaggccctgcccgcccctatcgagaagaccatctctaaggcaaagggacagcctagggagccacaggtgtacaccctgcctccatcccgggacgagctgacaaagaaccaggtgtctctgtggtgtctggtgaagggcttctatccctctgatatcgccgtggagtgggagagcaatggccagcctgagaacaattacaagaccacaccccctgtgctggacagcgatggctccttctttctgtatagcaagctgaccgtggataagtcccggtggcagcagggcaacgtgttttcttgtagcgtgatgcacgaggccctgcacaatcactacacacagaagtccctgtctctgagccctggcaagggtggaggtggctcaggaggaggcggttctgaagtgaaccctgccgctcatctgactggggctaactcaagtctgaccggaagtgggggacctctgctgtgggaaactcagctggggctggccttcctgaggggcctgagctatcacgacggcgccctggtggtgaccaaggcaggctactattacatctacagcaaggtgcagctgggaggagtgggatgcccactgggcctggcatccaccatcacacacggcctgtataagaggacccctcgctacccagaggagctggagctgctggtgagccagcagtccccttgtggaagggccacaagctcctctagagtgtggtgggatagctcctttctgggaggagtggtgcacctggaggcaggagagaaggtggtggtgcgggtgctggacgagagactggtgcggctgagagatggcaccagatcctatttcggcgcctttatggtgggtgggtctggcgaggtgaaccccgccgcccatctgaccggcgccaatagcagcctgacaggcagcggcggccctctgctgtgggagacacagctgggtcttgcttttctgcgcggcctgtcttatcacgacggcgctctggtcgtgaccaaggccggctactactacatctacagcaaggtgcaactgggcggcgtgggatgtcctctgggcctggcctctaccatcacacacggcctgtacaaaagaacccctcggtaccccgaggaactggaactcctggtcagccagcaatctccatgcggcagagccaccagctcttctagagtgtggtgggatagcagcttcctgggcggcgtggtgcacctggaggccggcgagaaggtggtggtcagagtgctggacgagagactggtgcggctgagagatgggaccagaagctacttcggcgcctttatggtg

SEQ ID NO: 47 - DNA, 1842 bp, synthetic construct
  misc_feature 1..1842: note = DNA sequence of anti-hu FAP HC hu IgG1 Fc hole DANG-hu LIGHT
  source 1..1842: mol_type = other DNA
caggtgcagctggtgcagtccggagcagaggtgaagaagccaggagcctctgtgaaggtgagctgcaagacctccagatacaccttcacagagtatacaatccactgggtgcgccaggcacctggacagcggctggagtggatcggaggcatcaaccccaacaatggcatccctaactacaatcagaagtttaagggcagagtgaccatcacagtggacacctccgcctctacagcctatatggagctgagctccctgaggagcgaggataccgccgtgtactattgcgcccggagaaggatcgcctacggctatgacgagggccacgccatggattactggggccagggcaccctggtgacagtgtctagcgcctctaccaagggaccaagcgtgttcccactggcaccatcctctaagagcacctccggaggaacagccgccctgggctgtctggtgaaggactatttcccagagcccgtgacagtgtcctggaactctggcgccctgacctccggagtgcacacatttcctgccgtgctgcagagctccggcctgtacagcctgtctagcgtggtgaccgtgccatcctctagcctgggcacccagacatatatctgcaacgtgaatcacaagcctagcaatacaaaggtggacaagaaggtggagccaaagtcctgtgacaagacccacacatgcccaccatgtccagcacctgagctgctgggaggaccatccgtgttcctgtttcctccaaagcccaaggatacactgatgatcagccgcacacctgaggtgacctgcgtggtggtggccgtgtcccacgaggaccccgaggtgaagtttaactggtacgtggacggcgtggaggtgcacaatgccaagaccaagcccagggaggagcagtacggctctacatatcgcgtggtgagcgtgctgaccgtgctgcaccaggactggctgaacggcaaggagtacaagtgcaaggtgtctaataaggccctgccagcccccatcgagaagaccatcagcaaggcaaagggacagccaagggagcctcaggtgtatacactgccccctagccgcgatgagctgaccaagaaccaggtgtccctgtcttgtgccgtgaagggcttctacccatccgacatcgccgtggagtgggagtctaatggccagcccgagaacaattataagaccacaccacccgtgctggactccgatggctctttctttctggtgagcaagctgacagtggacaagtccagatggcagcagggcaacgtgtttagctgctccgtgatgcacgaggccctgcacaatcactacacccagaagtctctgagcctgtcccctggcaagggtggaggtggctcaggaggaggcggttctgaagtgaaccctgccgctcatctgactggggctaactcaagtctgaccggaagtgggggacctctgctgtgggaaactcagctggggctggccttcctgaggggcctgagctatcacgacggcgccctggtggtgaccaaggcaggctactattacatctacagcaaggtgcagctgggaggagtgggatgcccactgggcctggcatccaccatcacacacggcctgtataagaggacccctcgctacccagaggagctggagctgctggtgagccagcagtccccttgtggaagggccacaagctcctctagagtgtggtgggatagctcctttctgggaggagtggtgcacctggaggcaggagagaaggtggtggtgcgggtgctggacgagagactggtgcggctgagagatggcaccagatcctatttcggcgcctttatggtg

SEQ ID NO: 48 - DNA, 1839 bp, synthetic construct
  misc_feature 1..1839: note = DNA sequence of anti-hu FAP HC hu IgG1 Fc DANG-hu LIGHT
  source 1..1839: mol_type = other DNA
caggtgcagctggtgcagtccggagcagaggtgaagaagccaggagcctctgtgaaggtgagctgcaagacctccagatacaccttcacagagtatacaatccactgggtgcgccaggcacctggacagcggctggagtggatcggaggcatcaaccccaacaatggcatccctaactacaatcagaagtttaagggcagagtgaccatcacagtggacacctccgcctctacagcctatatggagctgagctccctgaggagcgaggataccgccgtgtactattgcgcccggagaaggatcgcctacggctatgacgagggccacgccatggattactggggccagggcaccctggtgacagtgtctagcgcctctaccaagggaccaagcgtgttcccactggcaccatcctctaagagcacctccggaggaacagccgccctgggctgtctggtgaaggactatttcccagagcccgtgacagtgtcctggaactctggcgccctgacctccggagtgcacacatttcctgccgtgctgcagagctccggcctgtacagcctgtctagcgtggtgaccgtgccatcctctagcctgggcacccagacatatatctgcaacgtgaatcacaagcctagcaatacaaaggtggacaagaaggtggagccaaagtcctgtgataagacccacacatgccccccttgtcctgcaccagagctgctgggaggaccaagcgtgttcctgtttccacccaagcccaaggacaccctgatgatctctcgcaccccagaggtgacatgcgtggtggtggccgtgagccacgaggaccccgaggtgaagtttaactggtacgtggatggcgtggaggtgcacaatgccaagaccaagccaagagaggagcagtacggctccacctatagggtggtgtctgtgctgacagtgctgcaccaggattggctgaacggcaaggagtataagtgcaaggtgtccaataaggccctgcccgcccctatcgagaagaccatctctaaggcaaagggacagcctagggagccacaggtgtacaccctgcctccatcccgggacgagctgacaaagaaccaggtgtctctgacgtgtctggtgaagggcttctatccctctgatatcgccgtggagtgggagagcaatggccagcctgagaacaattacaagaccacaccccctgtgctggacagcgatggctccttctttctgtatagcaagctgaccgtggataagtcccggtggcagcagggcaacgtgttttcttgtagcgtgatgcacgaggccctgcacaatcactacacacagaagtccctgtctctgagccctggcggtggaggtggctcaggaggaggcggttctgaagtgaaccctgccgctcatctgactggggctaactcaagtctgaccggaagtgggggacctctgctgtgggaaactcagctggggctggccttcctgaggggcctgagctatcacgacggcgccctggtggtgaccaaggcaggctactattacatctacagcaaggtgcagctgggaggagtgggatgcccactgggcctggcatccaccatcacacacggcctgtataagaggacccctcgctacccagaggagctggagctgctggtgagccagcagtccccttgtggaagggccacaagctcctctagagtgtggtgggatagctcctttctgggaggagtggtgcacctggaggcaggagagaaggtggtggtgcgggtgctggacgagagactggtgcggctgagagatggcaccagatcctatttcggcgcctttatggtg

SEQ ID NO: 49 - DNA, 2301 bp, synthetic construct
  misc_feature 1..2301: note = DNA sequence of anti-hu FAP HC hu IgG1 Fc knob-hu scLIGHT2
  source 1..2301: mol_type = other DNA
caggtgcagctggtgcagtccggagcagaggtgaagaagccaggagcctctgtgaaggtgagctgcaagacctccagatacaccttcacagagtatacaatccactgggtgcgccaggcacctggacagcggctggagtggatcggaggcatcaaccccaacaatggcatccctaactacaatcagaagtttaagggcagagtgaccatcacagtggacacctccgcctctacagcctatatggagctgagctccctgaggagcgaggataccgccgtgtactattgcgcccggagaaggatcgcctacggctatgacgagggccacgccatggattactggggccagggcaccctggtgacagtgtctagcgcctctaccaagggaccaagcgtgttcccactggcaccatcctctaagagcacctccggaggaacagccgccctgggctgtctggtgaaggactatttcccagagcccgtgacagtgtcctggaactctggcgccctgacctccggagtgcacacatttcctgccgtgctgcagagctccggcctgtacagcctgtctagcgtggtgaccgtgccatcctctagcctgggcacccagacatatatctgcaacgtgaatcacaagcctagcaatacaaaggtggacaagaaggtggagccaaagtcctgtgataagacccacacatgccccccttgtcctgcaccagagctgctgggaggaccaagcgtgttcctgtttccacccaagcccaaggacaccctgatgatctctcgcaccccagaggtgacatgcgtggtggtggacgtgagccacgaggaccccgaggtgaagtttaactggtacgtggatggcgtggaggtgcacaatgccaagaccaagccaagagaggagcagtacaactccacctatagggtggtgtctgtgctgacagtgctgcaccaggattggctgaacggcaaggagtataagtgcaaggtgtccaataaggccctgcccgcccctatcgagaagaccatctctaaggcaaagggacagcctagggagccacaggtgtacaccctgcctccatcccgggacgagctgacaaagaaccaggtgtctctgtggtgtctggtgaagggcttctatccctctgatatcgccgtggagtgggagagcaatggccagcctgagaacaattacaagaccacaccccctgtgctggacagcgatggctccttctttctgtatagcaagctgaccgtggataagtcccggtggcagcagggcaacgtgttttcttgtagcgtgatgcacgaggccctgcacaatcactacacacagaagtccctgtctctgagccctggcggtggaggtggctcaggaggaggcggttctgaagtgaaccctgccgctcatctgactggggctaactcaagtctgaccggaagtgggggacctctgctgtgggaaactcagctggggctggccttcctgaggggcctgagctatcacgacggcgccctggtggtgaccaaggcaggctactattacatctacagcaaggtgcagctgggaggagtgggatgcccactgggcctggcatccaccatcacacacggcctgtataagaggacccctcgctacccagaggagctggagctgctggtgagccagcagtccccttgtggaagggccacaagctcctctagagtgtggtgggatagctcctttctgggaggagtggtgcacctggaggcaggagagaaggtggtggtgcgggtgctggacgagagactggtgcggctgagagatggcaccagatcctatttcggcgcctttatggtgggtgggtctggcgaggtgaaccccgccgcccatctgaccggcgccaatagcagcctgacaggcagcggcggccctctgctgtgggagacacagctgggtcttgcttttctgcgcggcctgtcttatcacgacggcgctctggtcgtgaccaaggccggctactactacatctacagcaaggtgcaactgggcggcgtgggatgtcctctgggcctggcctctaccatcacacacggcctgtacaaaagaacccctcggtaccccgaggaactggaactcctggtcagccagcaatctccatgcggcagagccaccagctcttctagagtgtggtgggatagcagcttcctgggcggcgtggtgcacctggaggccggcgagaaggtggtggtcagagtgctggacgagagactggtgcggctgagagatgggaccagaagctacttcggcgcctttatggtg

SEQ ID NO: 50 - DNA, 1839 bp, synthetic construct
  misc_feature 1..1839: note = DNA sequence of anti-hu FAP HC hu IgG1 Fc hole-hu LIGHT
  source 1..1839: mol_type = other DNA
caggtgcagctggtgcagtccggagcagaggtgaagaagccaggagcctctgtgaaggtgagctgcaagacctccagatacaccttcacagagtatacaatccactgggtgcgccaggcacctggacagcggctggagtggatcggaggcatcaaccccaacaatggcatccctaactacaatcagaagtttaagggcagagtgaccatcacagtggacacctccgcctctacagcctatatggagctgagctccctgaggagcgaggataccgccgtgtactattgcgcccggagaaggatcgcctacggctatgacgagggccacgccatggattactggggccagggcaccctggtgacagtgtctagcgcctctaccaagggaccaagcgtgttcccactggcaccatcctctaagagcacctccggaggaacagccgccctgggctgtctggtgaaggactatttcccagagcccgtgacagtgtcctggaactctggcgccctgacctccggagtgcacacatttcctgccgtgctgcagagctccggcctgtacagcctgtctagcgtggtgaccgtgccatcctctagcctgggcacccagacatatatctgcaacgtgaatcacaagcctagcaatacaaaggtggacaagaaggtggagccaaagtcctgtgacaagacccacacatgcccaccatgtccagcacctgagctgctgggaggaccatccgtgttcctgtttcctccaaagcccaaggatacactgatgatcagccgcacacctgaggtgacctgcgtggtggtggacgtgtcccacgaggaccccgaggtgaagtttaactggtacgtggacggcgtggaggtgcacaatgccaagaccaagcccagggaggagcagtacaactctacatatcgcgtggtgagcgtgctgaccgtgctgcaccaggactggctgaacggcaaggagtacaagtgcaaggtgtctaataaggccctgccagcccccatcgagaagaccatcagcaaggcaaagggacagccaagggagcctcaggtgtatacactgccccctagccgcgatgagctgaccaagaaccaggtgtccctgtcttgtgccgtgaagggcttctacccatccgacatcgccgtggagtgggagtctaatggccagcccgagaacaattataagaccacaccacccgtgctggactccgatggctctttctttctggtgagcaagctgacagtggacaagtccagatggcagcagggcaacgtgtttagctgctccgtgatgcacgaggccctgcacaatcactacacccagaagtctctgagcctgtcccctggcggtggaggtggctcaggaggaggcggttctgaagtgaaccctgccgctcatctgactggggctaactcaagtctgaccggaagtgggggacctctgctgtgggaaactcagctggggctggccttcctgaggggcctgagctatcacgacggcgccctggtggtgaccaaggcaggctactattacatctacagcaaggtgcagctgggaggagtgggatgcccactgggcctggcatccaccatcacacacggcctgtataagaggacccctcgctacccagaggagctggagctgctggtgagccagcagtccccttgtggaagggccacaagctcctctagagtgtggtgggatagctcctttctgggaggagtggtgcacctggaggcaggagagaaggtggtggtgcgggtgctggacgagagactggtgcggctgagagatggcaccagatcctatttcggcgcctttatggtg

SEQ ID NO: 51 - DNA, 681 bp, synthetic construct
  misc_feature 1..681: note = DNA sequence of hu IgG1 Fc hole DANG
  source 1..681: mol_type = other DNA
gacaagacccacacatgcccaccttgtccagcaccagagctgctgggaggaccatccgtgttcctgtttccacccaagcccaaggataccctgatgatcagcaggaccccagaggtgacatgcgtggtggtggccgtgtcccacgaggaccctgaggtgaagttcaactggtacgtggatggcgtggaggtgcacaatgccaagacaaagccacgggaggagcagtacggcagcacctatagagtggtgtccgtgctgacagtgctgcaccaggactggctgaacggcaaggagtacaagtgcaaggtgtctaataaggccctgcctgccccaatcgagaagaccatcagcaaggcaaagggacagccaagggagcctcaggtgtataccctgcctccaagccgcgacgagctgacaaagaaccaggtgagcctgtcctgtgccgtgaagggcttctacccttccgatatcgccgtggagtgggagtctaatggccagccagagaacaattataagaccacaccccctgtgctggactccgatggctctttctttctggtgtctaagctgaccgtggataagagcaggtggcagcagggcaacgtgttttcttgtagcgtgatgcacgaggccctgcacaatcactatacacagaagtccctgtctctgagccctggcaag

SEQ ID NO: 52 - DNA, 681 bp, synthetic construct; identical to SEQ ID NO: 51
  misc_feature 1..681: note = DNA sequence of hu IgG1 Fc knob DANG
  source 1..681: mol_type = other DNA

SEQ ID NO: 53 - DNA, 1362 bp, synthetic construct
  misc_feature 1..1362: note = DNA sequence of anti-hu FAP HC hu IgG1 Fc DANG
  source 1..1362: mol_type = other DNA
caggtgcagctggtgcagtccggagcagaggtgaagaagccaggagcctctgtgaaggtgagctgcaagacctccagatacaccttcacagagtatacaatccactgggtgcgccaggcacctggacagcggctggagtggatcggaggcatcaaccccaacaatggcatccctaactacaatcagaagtttaagggcagagtgaccatcacagtggacacctccgcctctacagcctatatggagctgagctccctgaggagcgaggataccgccgtgtactattgcgcccggagaaggatcgcctacggctatgacgagggccacgccatggattactggggccagggcaccctggtgacagtgtctagcgcctctaccaagggaccaagcgtgttcccactggcaccatcctctaagagcacctccggaggaacagccgccctgggctgtctggtgaaggactatttcccagagcccgtgacagtgtcctggaactctggcgccctgacctccggagtgcacacatttcctgccgtgctgcagagctccggcctgtacagcctgtctagcgtggtgaccgtgccatcctctagcctgggcacccagacatatatctgcaacgtgaatcacaagcctagcaatacaaaggtggacaagaaggtggagccaaagtcctgtgataagacccacacatgccccccttgtcctgcaccagagctgctgggaggaccaagcgtgttcctgtttccacccaagcccaaggacaccctgatgatctctcgcaccccagaggtgacatgcgtggtggtggccgtgagccacgaggaccccgaggtgaagtttaactggtacgtggatggcgtggaggtgcacaatgccaagaccaagccaagagaggagcagtacggctccacctatagggtggtgtctgtgctgacagtgctgcaccaggattggctgaacggcaaggagtataagtgcaaggtgtccaataaggccctgcccgcccctatcgagaagaccatctctaaggcaaagggacagcctagggagccacaggtgtacaccctgcctccatcccgggacgagctgacaaagaaccaggtgtctctgacgtgtctggtgaagggcttctatccctctgatatcgccgtggagtgggagagcaatggccagcctgagaacaattacaagaccacaccccctgtgctggacagcgatggctccttctttctgtatagcaagctgaccgtggataagtcccggtggcagcagggcaacgtgttttcttgtagcgtgatgcacgaggccctgcacaatcactacacacagaagtccctgtctctgagccctggcaag

SEQ ID NO: 54 - DNA, 2154 bp, synthetic construct
  misc_feature 1..2154: note = DNA sequence of hu scLIGHT-LTb2-hu IgG1 Fc hole DANG
  source 1..2154: mol_type = other DNA
gaagtgaaccctgccgctcatctgactggggctaactcaagtctgaccggaagtgggggacctctgctgtgggaaactcagctggggctggccttcctgaggggcctgagctatcacgacggcgccctggtggtgaccaaggcaggctactattacatctacagcaaggtgcagctgggaggagtgggatgcccactgggcctggcatccaccatcacacacggcctgtataagaggacccctcgctacccagaggagctggagctgctggtgagccagcagtccccttgtggaagggccacaagctcctctagagtgtggtgggatagctcctttctgggaggagtggtgcacctggaggcaggagagaaggtggtggtgcgggtgctggacgagagactggtgcggctgagagatggcaccagatcctatttcggcgcctttatggtgggcggcggcggctctggaggaggaggaagcggaggaggaggctccctgccagccgcccacctgatcggcgcccccctgaagggccagggcctgggctgggagacaacaaaggagcaggccttcctgacctctggcacacagtttagcgacgcagagggcctggccctgccacaggatggcctgtattacctgtattgcctggtgggctacaggggaagggcaccacctggaggaggcgaccctcagggcaggagcgtgaccctgcgctctagcctgtatagggcaggaggagcatacggaccaggaacacctgagctgctgctggagggcgccgagacagtgacacctgtgctggatccagcccggagacagggctatggccctctgtggtacacctctgtgggattcggaggcctggtgcagctgaggaggggagagagggtgtacgtgaacatcagccacccagacatggtggattttgcccgcggcaagacattctttggcgccgtgatggtgggaggatccggcctgcctgcagcacacctgatcggagcaccactgaagggacagggcctgggatgggagacaaccaaagaacaggccttcctgacctccggcacacagttttctgatgccgaaggcctggccctgcctcaggacggcctgtactacctgtattgtctggtgggctaccggggcagagcaccacccggaggaggcgacccccagggcagatccgtgaccctgaggtcctctctgtacagagccggcggcgcctacggaccaggaacaccagagctgctgctggagggagcagagacagtgacacccgtgctggatcctgcacggagacagggatatggaccactgtggtatacttccgtcggctttggcggcctggtccagctgagaagaggagagcgggtgtacgtgaatatctctcatcctgatatggtggacttcgcacggggaaaaaccttctttggggctgtcatggtcggaggctctggaggaggcggcagcgacaagacccacacatgcccaccatgtccagcacctgagctgctgggaggaccatccgtgttcctgtttcctccaaagcccaaggatacactgatgatcagccgcacacctgaggtgacctgcgtggtggtggccgtgtcccacgaggaccccgaggtgaagtttaactggtacgtggacggcgtggaggtgcacaatgccaagaccaagcccagggaggagcagtacggctctacatatcgcgtggtgagcgtgctgaccgtgctgcaccaggactggctgaacggcaaggagtacaagtgcaaggtgtctaataaggccctgccagcccccatcgagaagaccatcagcaaggcaaagggacagccaagggagcctcaggtgtatacactgccccctagccgcgatgagctgaccaagaaccaggtgtccctgtcttgtgccgtgaagggcttctacccatccgacatcgccgtggagtgggagtctaatggccagcccgagaacaattataagaccacaccacccgtgctggactccgatggctctttctttctggtgagcaagctgacagtggacaagtccagatggcagcagggcaacgtgtttagctgctccgtgatgcacgaggccctgcacaatcactacacccagaagtctctgagcctgtcccctggcaag

SEQ ID NO: 55 - DNA, 2079 bp, synthetic construct
  misc_feature 1..2079: note = DNA sequence of hu scLIGHT-LIGHT(L118K, G119E)2-hu IgG1 Fc hole DANG
  source 1..2079: mol_type = other DNA
gaagtgaaccctgccgctcatctgactggggctaactcaagtctgaccggaagtgggggacctctgctgtgggaaactcagctggggctggccttcctgaggggcctgagctatcacgacggcgccctggtggtgaccaaggcaggctactattacatctacagcaaggtgcagctgggaggagtgggatgcccactgggcctggcatccaccatcacacacggcctgtataagaggacccctcgctacccagaggagctggagctgctggtgagccagcagtccccttgtggaagggccacaagctcctctagagtgtggtgggatagctcctttctgggaggagtggtgcacctggaggcaggagagaaggtggtggtgcgggtgctggacgagagactggtgcggctgagagatggcaccagatcctatttcggcgcctttatggtgggcggctctggtgaggtgaacccagcagcacacctgaccggagcaaatagctccctgacaggatccggaggaccactgctgtgggagacccagaaggagctggccttcctgaggggactgtcttatcacgacggcgccctggtggtgacaaaggcaggctactattacatctactctaaggtgcagctgggaggagtgggatgccctctgggactggccagcaccatcacacacggcctgtataagaggaccccaaggtaccctgaggagctggagctgctggtgtcccagcagtctccctgtggcagggccacatctagctcccgcgtgtggtgggattctagctttctgggaggagtggtgcacctggaggcaggagagaaggtggtggtgcgggtgctggacgagagactggtgcggctgagagatggcacccggagctatttcggcgcctttatggtgggcggctccggcgaggtgaaccccgccgcccacctgaccggcgccaacagcagcctgaccggcagcggcggccccctgctgtgggagacccagaaggagctggccttcctgcgcggcctgagctaccacgacggcgccctggtggtgaccaaggccggctactactacatctacagcaaggtgcagctgggcggcgtgggctgccccctgggcctggccagcaccatcacccacggcctgtacaagcgcaccccccgctaccccgaggagctggagctgctggtgagccagcagagcccctgcggccgcgccaccagcagcagccgcgtgtggtgggacagcagcttcctgggcggcgtggtgcacctggaggccggcgagaaggtggtggtgcgcgtgctggacgagcgcctggtgcgcctgcgcgacggcacccgcagctacttcggcgccttcatggtgggaggctctggaggaggcggcagcgacaagacccacacatgcccaccatgtccagcacctgagctgctgggaggaccatccgtgttcctgtttcctccaaagcccaaggatacactgatgatcagccgcacacctgaggtgacctgcgtggtggtggccgtgtcccacgaggaccccgaggtgaagtttaactggtacgtggacggcgtggaggtgcacaatgccaagaccaagcccagggaggagcagtacggctctacatatcgcgtggtgagcgtgctgaccgtgctgcaccaggactggctgaacggcaaggagtacaagtgcaaggtgtctaataaggccctgccagcccccatcgagaagaccatcagcaaggcaaagggacagccaagggagcctcaggtgtatacactgccccctagccgcgatgagctgaccaagaaccaggtgtccctgtcttgtgccgtgaagggcttctacccatccgacatcgccgtggagtgggagtctaatggccagcccgagaacaattataagaccacaccacccgtgctggactccgatggctctttctttctggtgagcaagctgacagtggacaagtccagatggcagcagggcaacgtgtttagctgctccgtgatgcacgaggccctgcacaatcactacacccagaagtctctgagcctgtcccctggcaag

SEQ ID NO: 56 - DNA, 2154 bp, synthetic construct
  misc_feature 1..2154: note = DNA sequence of hu scLIGHT(226-231)-LTb2-hu IgG1 Fc hole DANG
  source 1..2154: mol_type = other DNA
gaagtgaaccctgccgctcatctgactggggctaactcaagtctgaccggaagtgggggacctctgctgtgggaaactcagctggggctggccttcctgaggggcctgagctatcacgacggcgccctggtggtgaccaaggcaggctactattacatctacagcaaggtgcagctgggaggagtgggatgcccactgggcctggcatccaccatcacacacggcctgtataagaggacccctcgctacccagaggagctggagctgctggtgagccagcagtccccttgtggaagggccacaagctcctctagagtgtggtgggatagctcctttctgggaggagtggtgcacctggaggcaggagagaaggtggtggtgcgggtgctggacgagagactggtggactacaccaaggaggacagatcctatttcggcgcctttatggtgggcggcggcggctctggaggaggaggaagcggaggaggaggctccctgccagccgcccacctgatcggcgcccccctgaagggccagggcctgggctgggagacaacaaaggagcaggccttcctgacctctggcacacagtttagcgacgcagagggcctggccctgccacaggatggcctgtattacctgtattgcctggtgggctacaggggaagggcaccacctggaggaggcgaccctcagggcaggagcgtgaccctgcgctctagcctgtatagggcaggaggagcatacggaccaggaacacctgagctgctgctggagggcgccgagacagtgacacctgtgctggatccagcccggagacagggctatggccctctgtggtacacctctgtgggattcggaggcctggtgcagctgaggaggggagagagggtgtacgtgaacatcagccacccagacatggtggattttgcccgcggcaagacattctttggcgccgtgatggtgggaggatccggcctgcctgcagcacacctgatcggagcaccactgaagggacagggcctgggatgggagacaaccaaagaacaggccttcctgacctccggcacacagttttctgatgccgaaggcctggccctgcctcaggacggcctgtactacctgtattgtctggtgggctaccggggcagagcaccacccggaggaggcgacccccagggcagatccgtgaccctgaggtcctctctgtacagagccggcggcgcctacggaccaggaacaccagagctgctgctggagggagcagagacagtgacacccgtgctggatcctgcacggagacagggatatggaccactgtggtatacttccgtcggctttggcggcctggtccagctgagaagaggagagcgggtgtacgtgaatatctctcatcctgatatggtggacttcgcacggggaaaaaccttctttggggctgtcatggtcggaggctctggaggaggcggcagcgacaagacccacacatgcccaccatgtccagcacctgagctgctgggaggaccatccgtgttcctgtttcctccaaagcccaaggatacactgatgatcagccgcacacctgaggtgacctgcgtggtggtggccgtgtcccacgaggaccccgaggtgaagtttaactggtacgtggacggcgtggaggtgcacaatgccaagaccaagcccagggaggagcagtacggctctacatatcgcgtggtgagcgtgctgaccgtgctgcaccaggactggctgaacggcaaggagtacaagtgcaaggtgtctaataaggccctgccagcccccatcgagaagaccatcagcaaggcaaagggacagccaagggagcctcaggtgtatacactgccccctagccgcgatgagctgaccaagaaccaggtgtccctgtcttgtgccgtgaagggcttctacccatccgacatcgccgtggagtgggagtctaatggccagcccgagaacaattataagaccacaccacccgtgctggactccgatggctctttctttctggtgagcaagctgacagtggacaagtccagatggcagcagggcaacgtgtttagctgctccgtgatgcacgaggccctgcacaatcactacacccagaagtctctgagcctgtcccctggcaag

SEQ ID NO: 57 - DNA, 2154 bp, synthetic construct
  misc_feature 1..2154: note = DNA sequence of hu scLIGHT(195-198)-LTb2-hu IgG1 Fc hole DANG
  source 1..2154: mol_type = other DNA
gaagtgaaccctgccgctcatctgactggggctaactcaagtctgaccggaagtgggggacctctgctgtgggaaactcagctggggctggccttcctgaggggcctgagctatcacgacggcgccctggtggtgaccaaggcaggctactattacatctacagcaaggtgcagctgggaggagtgggatgcccactgggcctggcatccaccatcacacacggcctgtataagaggacccctcgctacccagaggagctggagctgctggtgagccagcagtccccttgtggaagggccacaagctcctctagcaactggttcgatagctcctttctgggaggagtggtgcacctggaggcaggagagaaggtggtggtgcgggtgctggacgagagactggtgcggctgagagatggcaccagatcctatttcggcgcctttatggtgggcggcggcggctctggaggaggaggaagcggaggaggaggctccctgccagccgcccacctgatcggcgcccccctgaagggccagggcctgggctgggagacaacaaaggagcaggccttcctgacctctggcacacagtttagcgacgcagagggcctggccctgccacaggatggcctgtattacctgtattgcctggtgggctacaggggaagggcaccacctggaggaggcgaccctcagggcaggagcgtgaccctgcgctctagcctgtatagggcaggaggagcatacggaccaggaacacctgagctgctgctggagggcgccgagacagtgacacctgtgctggatccagcccggagacagggctatggccctctgtggtacacctctgtgggattcggaggcctggtgcagctgaggaggggagagagggtgtacgtgaacatcagccacccagacatggtggattttgcccgcggcaagacattctttggcgccgtgatggtgggaggatccggcctgcctgcagcacacctgatcggagcaccactgaagggacagggcctgggatgggagacaaccaaagaacaggccttcctgacctccggcacacagttttctgatgccgaaggcctggccctgcctcaggacggcctgtactacctgtattgtctggtgggctaccggggcagagcaccacccggaggaggcgacccccagggcagatccgtgaccctgaggtcctctctgtacagagccggcggcgcctacggaccaggaacaccagagctgctgctggagggagcagagacagtgacacccgtgctggatcctgcacggagacagggatatggaccactgtggtatacttccgtcggctttggcggcctggtccagctgagaagaggagagcgggtgtacgtgaatatctctcatcctgatatggtggacttcgcacggggaaaaaccttctttggggctgtcatggtcggaggctctggaggaggcggcagcgacaagacccacacatgcccaccatgtccagcacctgagctgctgggaggaccatccgtgttcctgtttcctccaaagcccaaggatacactgatgatcagccgcacacctgaggtgacctgcgtggtggtggccgtgtcccacgaggaccccgaggtgaagtttaactggtacgtggacggcgtggaggtgcacaatgccaagaccaagcccagggaggagcagtacggctctacatatcgcgtggtgagcgtgctgaccgtgctgcaccaggactggctgaacggcaaggagtacaagtgcaaggtgtctaataaggccctgccagcccccatcgagaagaccatcagcaaggcaaagggacagccaagggagcctcaggtgtatacactgccccctagccgcgatgagctgaccaagaaccaggtgtccctgtcttgtgccgtgaagggcttctacccatccgacatcgccgtggagtgggagtctaatggccagcccgagaacaattataagaccacaccacccgtgctggactccgatggctctttctttctggtgagcaagctgacagtggacaagtccagatggcagcagggcaacgtgtttagctgctccgtgatgcacgaggccctgcacaatcactacacccagaagtctctgagcctgtcccctggcaag

SEQ ID NO: 58 - DNA, 2121 bp, synthetic construct
  misc_feature 1..2121: note = DNA sequence of hu scLIGHT-LTb2(GGSG)-hu IgG1 Fc hole DANG
  source 1..2121: mol_type = other DNA
gaagtgaaccctgccgctcatctgactggggctaactcaagtctgaccggaagtgggggacctctgctgtgggaaactcagctggggctggccttcctgaggggcctgagctatcacgacggcgccctggtggtgaccaaggcaggctactattacatctacagcaaggtgcagctgggaggagtgggatgcccactgggcctggcatccaccatcacacacggcctgtataagaggacccctcgctacccagaggagctggagctgctggtgagccagcagtccccttgtggaagggccacaagctcctctagagtgtggtgggatagctcctttctgggaggagtggtgcacctggaggcaggagagaaggtggtggtgcgggtgctggacgagagactggtgcggctgagagatggcaccagatcctatttcggcgcctttatggtgggaggaagcggactgccagccgcccacctgatcggcgcccccctgaagggccagggcctgggctgggagacaacaaaggagcaggccttcctgacctctggcacacagtttagcgacgcagagggcctggccctgccacaggatggcctgtattacctgtattgcctggtgggctacaggggaagggcaccacctggaggaggcgaccctcagggcaggagcgtgaccctgcgctctagcctgtatagggcaggaggagcatacggaccaggaacacctgagctgctgctggagggcgccgagacagtgacacctgtgctggatccagcccggagacagggctatggccctctgtggtacacctctgtgggattcggaggcctggtgcagctgaggaggggagagagggtgtacgtgaacatcagccacccagacatggtggattttgcccgcggcaagacattctttggcgccgtgatggtgggaggatccggcctgcctgcagcacacctgatcggagcaccactgaagggacagggcctgggatgggagacaaccaaagaacaggccttcctgacctccggcacacagttttctgatgccgaaggcctggccctgcctcaggacggcctgtactacctgtattgtctggtgggctaccggggcagagcaccacccggaggaggcgacccccagggcagatccgtgaccctgaggtcctctctgtacagagccggcggcgcctacggaccaggaacaccagagctgctgctggagggagcagagacagtgacacccgtgctggatcctgcacggagacagggatatggaccactgtggtatacttccgtcggctttggcggcctggtccagctgagaagaggagagcgggtgtacgtgaatatctctcatcctgatatggtggacttcgcacggggaaaaaccttctttggggctgtcatggtcggaggctctggaggaggcggcagcgacaagacccacacatgcccaccatgtccagcacctgagctgctgggaggaccatccgtgttcctgtttcctccaaagcccaaggatacactgatgatcagccgcacacctgaggtgacctgcgtggtggtggccgtgtcccacgaggaccccgaggtgaagtttaactggtacgtggacggcgtggaggtgcacaatgccaagaccaagcccagggaggagcagtacggctctacatatcgcgtggtgagcgtgctgaccgtgctgcaccaggactggctgaacggcaaggagtacaagtgcaaggtgtctaataaggccctgccagcccccatcgagaagaccatcagcaaggcaaagggacagccaagggagcctcaggtgtatacactgccccctagccgcgatgagctgaccaagaaccaggtgtccctgtcttgtgccgtgaagggcttctacccatccgacatcgccgtggagtgggagtctaatggccagcccgagaacaattataagaccacaccacccgtgctggactccgatggctctttctttctggtgagcaagctgacagtggacaagtccagatggcagcagggcaacgtgtttagctgctccgtgatgcacgaggccctgcacaatcactacacccagaagtctctgagcctgtcccctggcaag

SEQ ID NO: 59 - DNA, 1341 bp, synthetic construct
  misc_feature 1..1341: note = DNA sequence of anti-mu FAP HC mu IgG2a Fc knob DANG
  source 1..1341: mol_type = other DNA
caggtgcagctgcagcagtccggagcagagctggcaaggcctggagcctctgtgaacctgagctgcaaggcctccggctacaccttcacaaacaatggcatcaattggctgaagcagaggaccggacagggactggagtggatcggcgagatctacccaagatctaccaacacactgtataatgagaagttcaagggcaaggccaccctgacagcagaccggagctccaacaccgcctacatggagctgagaagcctgacatccgaggattctgccgtgtatttttgtgcacgcaccctgacagcacccttcgccttttggggacagggcaccctggtgacagtgagcgccgccaagaccacagcaccaagcgtgtatccactggcacccgtgtgcggcgataccacaggctctagcgtgaccctgggctgtctggtgaagggctacttccctgagccagtgaccctgacatggaacagcggctctctgtcctctggcgtgcacacctttcctgccgtgctgcagtccgatctgtatacactgagctcctctgtgaccgtgacaagctccacctggcccagccagtccatcacatgcaacgtggcccaccctgcctctagcaccaaggtggacaagaagatcgagccacggggccccacaatcaagccatgtccaccttgcaagtgtccagcacctaatctgctgggaggacctagcgtgttcatctttccacccaagatcaaggacgtgctgatgatctctctgagccctatcgtgacctgcgtggtggtggccgtgtctgaggacgatccagatgtgcagatcagctggttcgtgaacaatgtggaggtgcacaccgcccagacccagacacaccgggaggactacggctccacactgagagtggtgtctgccctgcccatccagcaccaggactggatgtccggcaaggagtttaagtgcaaggtgaacaataaggatctgccagcccccatcgagaggaccatctctaagcctaagggcagcgtgcgcgcaccacaggtgtatgtgctgcctccacccgaggaggagatgaccaagaagcaggtgacactgtggtgtatggtgaccgacttcatgccagaggatatctacgtggagtggaccaacaatggcaagacagagctgaactataagaatacagagcccgtgctggacagcgatggctcctactttatgtatagcaagctgagggtggagaagaagaactgggtggagcgcaattcctactcttgtagcgtggtgcacgagggcctgcacaaccaccacaccacaaagtccttttctagaacccccggcaag

SEQ ID NO: 60 - DNA, 639 bp, synthetic construct
  misc_feature 1..639: note = DNA sequence of anti-mu FAP LC
  source 1..639: mol_type = other DNA
cagatcgtgctgacacagtcccctgccatcatgtctgccagcccaggcgagaaggtgaccatgacatgctctgccagctccggcgtgaacttcatgcactggtaccagcagaagtctggcacaagccccaagcggtggatcttcgacacctccaagctggcctctggcgtgcctgccagattttccggctctggcagcggcacatcctattctctgaccatctctagcatggaggccgaggacgccgccacctactattgccagcagtggagcttcaatccccctacatttggcggcggcaccaagctggagatcaagagggcagatgcagcaccaacagtgtccatctttccaccctcctctgagcagctgaccagcggaggagcatccgtggtgtgcttcctgaacaacttctaccccaaggacatcaacgtgaagtggaagatcgatggctctgagaggcagaacggcgtgctgaatagctggacagaccaggattccaaggactctacctatagcatgagctccaccctgacactgaccaaggatgagtacgagaggcacaatagctatacatgcgaggccacccacaagacaagcacctcccctatcgtgaagtccttcaaccgcaatgagtgt

SEQ ID NO: 61 - DNA, 2088 bp, synthetic construct
  misc_feature 1..2088: note = DNA sequence of mu scLIGHT3-mu IgG2a Fc hole DANG
  source 1..2088: mol_type = other DNA
aaccctgcagcacacctgaccggagcaaatgcatccctgatcggaatcggaggaccactgctgtgggagacaaggctgggactggccttcctgaggggactgacctaccacgatggcgccctggtgacaatggagccaggctactattacgtgtatagcaaggtgcagctgtccggagtgggatgcccacagggactggccaacggcctgcctatcacccacggcctgtataagcggacaagcagataccccaaggagctggagctgctggtgtcccggagatctccttgtggaagggccaacagctcccgcgtgtggtgggattctagcttcctgggaggagtggtgcacctggaggcaggcgaggaggtggtggtgcgggtgcctggcaatagactggtgaggccaagggacggaacccggtcttacttcggagcctttatggtgggaggcagcggaaacccagcagcacacctgaccggcgccaacgccagcctgattggaatcggaggacctctgctgtgggaaaccaggctgggactggcctttctgagaggactgacctaccacgacggcgccctggtcaccatggagccaggctattactacgtgtactctaaggtgcagctgagtggcgtcggctgtcctcagggactggccaatggcctgcccattactcacggcctgtataagaggacaagccgctacccaaaagaactggagctgctggtgagcaggcgctccccatgtggaagggccaactcctctcgcgtgtggtgggatagctccttcctgggcggcgtcgtccacctggaagccggagaagaagtcgtggtgcgggtgccaggaaatagactggtgcggcctagagacggcaccagatcctatttcggcgcctttatggtgggcggctctggcaatcccgccgcccacctgactggcgccaacgcctctctgattggcattggcggccctctgctgtgggaaactagactgggcctggcctttctgcgcggcctgacttatcatgacggcgccctggtcactatggagcctggatattattacgtgtattccaaggtgcagctgtctggagtgggatgccctcagggcctggctaacggcctgccaattacacatggactgtacaaacggacaagcagataccctaaagaactggaactgctggtgtctcggagaagcccatgtggcagggccaactctagtcgcgtgtggtgggactcctctttcctgggcggcgtcgtgcacctggaagccggagaggaagtcgtggtgcgggtcccagggaacaggctggtgaggcctagggacggaaccaggagctactttggagcctttatggtcggcggcagcggaggaggaggctccgagccacgcggccccacaatcaagccatgccccccttgcaagtgtcctgcaccaaatctgctgggaggaccatccgtgttcatctttccacccaagatcaaggacgtgctgatgatcagcctgtccccaatcgtgacctgcgtggtcgtggccgtgagcgaggacgatcctgatgtgcagatctcctggttcgtgaacaatgtggaggtgcacaccgcccagacccagacacaccgggaggactacggctccacactgagagtggtgtctgccctgcccatccagcaccaggactggatgagcggcaaggagtttaagtgcaaggtgaacaataaggatctgcccgcccctatcgagcggacaatctctaagcctaagggcagcgtgagagccccacaggtgtatgtgctgcctccacccgaggaggagatgaccaagaagcaggtgacactgtcttgtgccgtgaccgacttcatgcctgaggatatctatgtggagtggaccaacaatggcaagacagagctgaactacaagaatacagagccagtgctggactccgatggctcttacttcatggtgagcaagctgagggtggagaagaagaactgggtggagcgcaattcttacagctgctccgtggtgcacgagggcctgcacaaccaccacaccacaaagtcttttagccggacccctggcaag

SEQ ID NO: 62 - DNA, 1341 bp, synthetic construct
  misc_feature 1..1341: note = DNA sequence of anti-mu FAP HC mu IgG2a Fc knob
  source 1..1341: mol_type = other DNA
caggtgcagctgcagcagtccggagcagagctggcaaggcctggagcctctgtgaacctgagctgcaaggcctccggctacaccttcacaaacaatggcatcaattggctgaagcagaggaccggacagggactggagtggatcggcgagatctacccaagatctaccaacacactgtataatgagaagttcaagggcaaggccaccctgacagcagaccggagctccaacaccgcctacatggagctgagaagcctgacatccgaggattctgccgtgtatttttgtgcacgcaccctgacagcacccttcgccttttggggacagggcaccctggtgacagtgagcgccgcaaagaccacagcaccaagcgtgtatccactggcacccgtgtgcggcgataccacaggctctagcgtgaccctgggctgtctggtgaagggctacttccctgagccagtgaccctgacatggaacagcggctctctgtcctctggcgtgcacacctttcctgccgtgctgcagtccgatctgtatacactgagctcctctgtgaccgtgacaagctccacctggcccagccagtccatcacatgcaacgtggcccaccctgcctctagcaccaaggtggacaagaagatcgagccacggggccccacaatcaagccatgtccaccttgcaagtgtccagcacctaatctgctgggaggacctagcgtgttcatctttccacccaagatcaaggacgtgctgatgatctctctgagccctatcgtgacctgcgtggtggtggacgtgtctgaggacgatccagatgtgcagatcagctggttcgtgaacaatgtggaggtgcacaccgcccagacccagacacaccgggaggactacaactccacactgagagtggtgtctgccctgcccatccagcaccaggactggatgtccggcaaggagtttaagtgcaaggtgaacaataaggatctgccagcccccatcgagaggaccatctctaagcctaagggcagcgtgcgcgcaccacaggtgtatgtgctgcctccacccgaggaggagatgaccaagaagcaggtgacactgtggtgtatggtgaccgacttcatgccagaggatatctacgtggagtggaccaacaatggcaagacagagctgaactataagaatacagagcccgtgctggacagcgatggctcctactttatgtatagcaagctgagggtggagaagaagaactgggtggagcgcaattcctactcttgtagcgtggtgcacgagggcctgcacaaccaccacaccacaaagtccttttctagaacccccggcaag

SEQ ID NO: 63 - DNA, 2088 bp, synthetic construct
  misc_feature 1..2088: note = DNA sequence of mu scLIGHT3-mu IgG2a Fc hole
  source 1..2088: mol_type = other DNA
aaccctgcagcacacctgaccggagcaaatgcatccctgatcggaatcggaggaccactgctgtgggagacaaggctgggactggccttcctgaggggactgacctaccacgatggcgccctggtgacaatggagccaggctactattacgtgtatagcaaggtgcagctgtccggagtgggatgcccacagggactggccaacggcctgcctatcacccacggcctgtataagcggacaagcagataccccaaggagctggagctgctggtgtcccggagatctccttgtggaagggccaacagctcccgcgtgtggtgggattctagcttcctgggaggagtggtgcacctggaggcaggcgaggaggtggtggtgcgggtgcctggcaatagactggtgaggccaagggacggaacccggtcttacttcggagcctttatggtgggaggcagcggaaacccagcagcacacctgaccggcgccaacgccagcctgattggaatcggaggacctctgctgtgggaaaccaggctgggactggcctttctgagaggactgacctaccacgacggcgccctggtcaccatggagccaggctattactacgtgtactctaaggtgcagctgagtggcgtcggctgtcctcagggactggccaatggcctgcccattactcacggcctgtataagaggacaagccgctacccaaaagaactggagctgctggtgagcaggcgctccccatgtggaagggccaactcctctcgcgtgtggtgggatagctccttcctgggcggcgtcgtccacctggaagccggagaagaagtcgtggtgcgggtgccaggaaatagactggtgcggcctagagacggcaccagatcctatttcggcgcctttatggtgggcggctctggcaatcccgccgcccacctgactggcgccaacgcctctctgattggcattggcggccctctgctgtgggaaactagactgggcctggcctttctgcgcggcctgacttatcatgacggcgccctggtcactatggagcctggatattattacgtgtattccaaggtgcagctgtctggagtgggatgccctcagggcctggctaacggcctgccaattacacatggactgtacaaacggacaagcagataccctaaagaactggaactgctggtgtctcggagaagcccatgtggcagggccaactctagtcgcgtgtggtgggactcctctttcctgggcggcgtcgtgcacctggaagccggagaggaagtcgtggtgcgggtcccagggaacaggctggtgaggcctagggacggaaccaggagctactttggagcctttatggtcggcggcagcggaggaggaggctccgagccacgcggccccacaatcaagccatgccccccttgcaagtgtcctgcaccaaatctgctgggaggaccatccgtgttcatctttccacccaagatcaaggacgtgctgatgatcagcctgtccccaatcgtgacctgcgtggtcgtggatgtgagcgaggacgatcctgatgtgcagatctcctggttcgtgaacaatgtggaggtgcacaccgcccagacccagacacaccgggaggactacaactccacactgagagtggtgtctgccctgcccatccagcaccaggactggatgagcggcaaggagtttaagtgcaaggtgaacaataaggatctgcccgcccctatcgagcggacaatctctaagcctaagggcagcgtgagagccccacaggtgtatgtgctgcctccacccgaggaggagatgaccaagaagcaggtgacactgtcttgtgccgtgaccgacttcatgcctgaggatatctatgtggagtggaccaacaatggcaagacagagctgaactacaagaatacagagccagtgctggactccgatggctcttacttcatggtgagcaagctgagggtggagaagaagaactgggtggagcgcaattcttacagctgctccgtggtgcacgagggcctgcacaaccaccacaccacaaagtcttttagccggacccctggcaag

SEQ ID NO: 64 - DNA, 2088 bp, synthetic construct
  misc_feature 1..2088: note = DNA sequence of mu scLIGHT(225-230)3-mu IgG2a Fc hole DANG
  source 1..2088: mol_type = other DNA
aaccctgcagcacacctgaccggagcaaatgcatccctgatcggaatcggaggaccactgctgtgggagacaaggctgggactggccttcctgaggggactgacctaccacgatggcgccctggtgacaatggagccaggctactattacgtgtatagcaaggtgcagctgtccggagtgggatgcccacagggactggccaacggcctgcctatcacccacggcctgtataagcggacaagcagataccccaaggagctggagctgctggtgtcccggagatctccttgtggaagggccaacagctcccgcgtgtggtgggattctagcttcctgggaggagtggtgcacctggaggcaggcgaggaggtggtggtgcgggtgcctggcaatagactggtggactacaccaaggaggatcggtcttacttcggagcctttatggtgggaggcagcggcaacccagcagcacacctgaccggcgccaacgccagcctgattggaatcggaggacctctgctgtgggaaaccaggctgggactggcctttctgagaggactgacctaccacgacggcgccctggtcaccatggagccaggctattactacgtgtactctaaggtgcagctgagtggcgtcggctgtcctcagggactggccaatggcctgcccattactcacggcctgtataagaggacaagccgctacccaaaagaactggagctgctggtgagcaggcgctccccatgtggaagggccaactcctctcgcgtgtggtgggatagctccttcctgggcggcgtcgtccacctggaagccggagaagaagtcgtggtgcgggtgccaggaaatagactggtggattacacaaaggaagacagatcctatttcggcgcctttatggtgggcggctccggaaatcccgccgcccacctgactggcgccaacgcctctctgattggcattggcggccctctgctgtgggaaactagactgggcctggcctttctgcgcggcctgacttatcatgacggcgccctggtcactatggagcctggatattattacgtgtattccaaggtgcagctgtctggagtgggatgccctcagggcctggctaacggcctgccaattacacatggactgtacaaacggacaagcagataccctaaagaactggaactgctggtgtctcggagaagcccatgtggcagggccaactctagtcgcgtgtggtgggactcctctttcctgggcggcgtcgtgcacctggaagccggagaggaagtcgtggtgcgggtcccagggaacaggctggtggactatactaaagaggacaggagctactttggagcctttatggtcggcggcagcgggggaggaggctccgagccacgcggccccacaatcaagccatgccccccttgcaagtgtcctgcaccaaatctgctgggaggaccatccgtgttcatctttccacccaagatcaaggacgtgctgatgatcagcctgtccccaatcgtgacctgcgtggtcgtggccgtgagcgaggacgatcctgatgtgcagatctcctggttcgtgaacaatgtggaggtgcacaccgcccagacccagacacaccgggaggactacggctccacactgagagtggtgtctgccctgcccatccagcaccaggactggatgagcggcaaggagtttaagtgcaaggtgaacaataaggatctgcccgcccctatcgagcggacaatctctaagcctaagggcagcgtgagagccccacaggtgtatgtgctgcctccacccgaggaggagatgaccaagaagcaggtgacactgtcttgtgccgtgaccgacttcatgcctgaggatatctatgtggagtggaccaacaatggcaagacagagctgaactacaagaatacagagccagtgctggactccgatggctcttacttcatggtgagcaagctgagggtggagaagaagaactgggtggagcgcaattcttacagctgctccgtggtgcacgagggcctgcacaaccaccacaccacaaagtcttttagccggacccctggcaag

SEQ ID NO: 65 - DNA, 2088 bp, synthetic construct
  misc_feature 1..2088: note = DNA sequence of mu scLIGHT(194-197)3-mu IgG2a Fc hole DANG
  source 1..2088: mol_type = other DNA
aaccctgcagcacacctgaccggagcaaatgcatccctgatcggaatcggaggaccactgctgtgggagacaaggctgggactggccttcctgaggggactgacctaccacgatggcgccctggtgacaatggagccaggctactattacgtgtatagcaaggtgcagctgtccggagtgggatgcccacagggactggccaacggcctgcctatcacccacggcctgtataagcggacaagcagataccccaaggagctggagctgctggtgtcccggagatctccttgtggaagggccaacagctccaacaattggttcgattctagcttcctgggaggagtggtgcacctggaggcaggcgaggaggtggtggtgcgggtgcctggcaatagactggtgaggccaagggacggaacccggtcttacttcggagcctttatggtgggaggcagcggcaacccagcagcacacctgaccggcgccaacgccagcctgattggaatcggaggacctctgctgtgggaaaccaggctgggactggcctttctgagaggactgacctaccacgacggcgccctggtcaccatggagccaggctattactacgtgtactctaaggtgcagctgagtggcgtcggctgtcctcagggactggccaatggcctgcccattactcacggcctgtataagaggacaagccgctacccaaaagaactggagctgctggtgagcaggcgctccccatgtggaagggccaactcctctaataattggttcgatagctccttcctgggcggcgtcgtccacctggaagccggagaagaagtcgtggtgcgggtgccaggaaatagactggtgcggcctagagacggcaccagatcctatttcggcgcctttatggtgggcggctccggaaatcccgccgcccacctgactggcgccaacgcctctctgattggcattggcggccctctgctgtgggaaactagactgggcctggcctttctgcgcggcctgacttatcatgacggcgccctggtcactatggagcctggatattattacgtgtattccaaggtgcagctgtctggagtgggatgccctcagggcctggctaacggcctgccaattacacatggactgtacaaacggacaagcagataccctaaagaactggaactgctggtgtctcggagaagcccatgtggcagggccaactctagtaacaattggtttgactcctctttcctgggcggcgtcgtgcacctggaagccggagaggaagtcgtggtgcgggtcccagggaacaggctggtgaggcctagggacggaaccaggagctactttggagcctttatggtcggcggcagcgggggaggaggctccgagccacgcggccccacaatcaagccatgccccccttgcaagtgtcctgcaccaaatctgctgggaggaccatccgtgttcatctttccacccaagatcaaggacgtgctgatgatcagcctgtccccaatcgtgacctgcgtggtcgtggccgtgagcgaggacgatcctgatgtgcagatctcctggttcgtgaacaatgtggaggtgcacaccgcccagacccagacacaccgggaggactacggctccacactgagagtggtgtctgccctgcccatccagcaccaggactggatgagcggcaaggagtttaagtgcaaggtgaacaataaggatctgcccgcccctatcgagcggacaatctctaagcctaagggcagcgtgagagccccacaggtgtatgtgctgcctccacccgaggaggagatgaccaagaagcaggtgacactgtcttgtgccgtgaccgacttcatgcctgaggatatctatgtggagtggaccaacaatggcaagacagagctgaactacaagaatacagagccagtgctggactccgatggctcttacttcatggtgagcaagctgagggtggagaagaagaactgggtggagcgcaattcttacagctgctccgtggtgcacgagggcctgcacaaccaccacaccacaaagtcttttagccggacccctggcaag

SEQ ID NO: 66 - DNA, 2277 bp, synthetic construct
  misc_feature 1..2277: note = DNA sequence of anti-mu FAP HC mu IgG2a Fc knob DANG-mu scLIGHT2
  source 1..2277: mol_type = other DNA
caggtgcagctgcagcagtccggagcagagctggcaaggcctggagcctctgtgaacctgagctgcaaggcctccggctacaccttcacaaacaatggcatcaattggctgaagcagaggaccggacagggactggagtggatcggcgagatctacccaagatctaccaacacactgtataatgagaagttcaagggcaaggccaccctgacagcagaccggagctccaacaccgcctacatggagctgagaagcctgacatccgaggattctgccgtgtatttttgtgcacgcaccctgacagcacccttcgccttttggggacagggcaccctggtgacagtgagcgccgccaagaccacagcaccaagcgtgtatccactggcacccgtgtgcggcgataccacaggctctagcgtgaccctgggctgtctggtgaagggctacttccctgagccagtgaccctgacatggaacagcggctctctgtcctctggcgtgcacacctttcctgccgtgctgcagtccgatctgtatacactgagctcctctgtgaccgtgacaagctccacctggcccagccagtccatcacatgcaacgtggcccaccctgcctctagcaccaaggtggacaagaagatcgagccacggggccccacaatcaagccatgtccaccttgcaagtgtccagcacctaatctgctgggaggacctagcgtgttcatctttccacccaagatcaaggacgtgctgatgatctctctgagccctatcgtgacctgcgtggtggtggccgtgtctgaggacgatccagatgtgcagatcagctggttcgtgaacaatgtggaggtgcacaccgcccagacccagacacaccgggaggactacggctccacactgagagtggtgtctgccctgcccatccagcaccaggactggatgtccggcaaggagtttaagtgcaaggtgaacaataaggatctgccagcccccatcgagaggaccatctctaagcctaagggcagcgtgcgcgcaccacaggtgtatgtgctgcctccacccgaggaggagatgaccaagaagcaggtgacactgtggtgtatggtgaccgacttcatgccagaggatatctacgtggagtggaccaacaatggcaagacagagctgaactataagaatacagagcccgtgctggacagcgatggctcctactttatgtatagcaagctgagggtggagaagaagaactgggtggagcgcaattcctactcttgtagcgtggtgcacgagggcctgcacaaccaccacaccacaaagtccttttctagaacccccggcaagggtggaggtggctcaggaggaggcggttctaaccctgcagcacacctgaccggagcaaatgcatccctgatcggaatcggaggaccactgctgtgggagacaaggctgggactggccttcctgaggggactgacctaccacgatggcgccctggtgacaatggagccaggctactattacgtgtatagcaaggtgcagctgtccggagtgggatgcccacagggactggccaacggcctgcctatcacccacggcctgtataagcggacaagcagataccccaaggagctggagctgctggtgtcccggagatctccttgtggaagggccaacagctcccgcgtgtggtgggattctagcttcctgggaggagtggtgcacctggaggcaggcgaggaggtggtggtgcgggtgcctggcaatagactggtgaggccaagggacggaacccggtcttacttcggcgcctttatggtgggtgggtctggcaatccagccgcccacctgacaggcgccaacgccagcctgatcggcatcggcggacctctgctgtgggagacaagactgggactggccttcctgagaggcctgacatatcacgatggcgccctggtgacaatggaacctggctactactacgtgtacagcaaggtgcagctgagcggagttggctgcccacagggcctcgccaatggcctgcctatcacccacggcctgtacaaacgcaccagcagataccccaaggaactggagctgctggtgtccaggcggtctccttgcggcagagccaactccagccgggtgtggtgggatagctctttcctgggcggcgtggtgcatctggaagccggcgaggaagtggtcgtgcgggtgccaggaaatagactggttagacctagagatgggaccagaagctacttcggcgcttttatggtg

SEQ ID NO: 67 - DNA, 1818 bp, synthetic construct
  misc_feature 1..1818: note = DNA sequence of anti-mu FAP HC mu IgG2a Fc hole DANG-mu LIGHT
  source 1..1818: mol_type = other DNA
caggtgcagctgcagcagtccggagcagagctggcaaggcctggagcctctgtgaacctgagctgcaaggcctccggctacaccttcacaaacaatggcatcaattggctgaagcagaggaccggacagggactggagtggatcggcgagatctacccaagatctaccaacacactgtataatgagaagttcaagggcaaggccaccctgacagcagaccggagctccaacaccgcctacatggagctgagaagcctgacatccgaggattctgccgtgtatttttgtgcacgcaccctgacagcacccttcgccttttggggacagggcaccctggtgacagtgagcgccgccaagaccacagcaccaagcgtgtatccactggcacccgtgtgcggcgataccacaggctctagcgtgaccctgggctgtctggtgaagggctacttccctgagccagtgaccctgacatggaacagcggctctctgtcctctggcgtgcacacctttcctgccgtgctgcagtccgatctgtatacactgagctcctctgtgaccgtgacaagctccacctggcccagccagtccatcacatgcaacgtggcccaccctgcctctagcaccaaggtggacaagaagatcgagccacgcggccccacaatcaagccatgccccccttgcaagtgtcctgcaccaaatctgctgggaggaccatccgtgttcatctttccacccaagatcaaggacgtgctgatgatcagcctgtccccaatcgtgacctgcgtggtcgtggccgtgagcgaggacgatcctgatgtgcagatctcctggttcgtgaacaatgtggaggtgcacaccgcccagacccagacacaccgggaggactacggctccacactgagagtggtgtctgccctgcccatccagcaccaggactggatgagcggcaaggagtttaagtgcaaggtgaacaataaggatctgcccgcccctatcgagcggacaatctctaagcctaagggcagcgtgagagccccacaggtgtatgtgctgcctccacccgaggaggagatgaccaagaagcaggtgacactgtcttgtgccgtgaccgacttcatgcctgaggatatctatgtggagtggaccaacaatggcaagacagagctgaactacaagaatacagagccagtgctggactccgatggctcttacttcatggtgagcaagctgagggtggagaagaagaactgggtggagcgcaattcttacagctgctccgtggtgcacgagggcctgcacaaccaccacaccacaaagtcttttagccggacccctggcaagggtggaggtggctcaggaggaggcggttctaaccctgcagcacacctgaccggagcaaatgcatccctgatcggaatcggaggaccactgctgtgggagacaaggctgggactggccttcctgaggggactgacctaccacgatggcgccctggtgacaatggagccaggctactattacgtgtatagcaaggtgcagctgtccggagtgggatgcccacagggactggccaacggcctgcctatcacccacggcctgtataagcggacaagcagataccccaaggagctggagctgctggtgtcccggagatctccttgtggaagggccaacagctcccgcgtgtggtgggattctagcttcctgggaggagtggtgcacctggaggcaggcgaggaggtggtggtgcgggtgcctggcaatagactggtgaggccaagggacggaacccggtcttacttcggcgcctttatggtg

SEQ ID NO: 68 - DNA, 1815 bp, synthetic construct
  misc_feature 1..1815: note = DNA sequence of anti-mu FAP HC mu IgG2a Fc DANG-mu LIGHT
  source 1..1815: mol_type = other DNA
caggtgcagctgcagcagtccggagcagagctggcaaggcctggagcctctgtgaacctgagctgcaaggcctccggctacaccttcacaaacaatggcatcaattggctgaagcagaggaccggacagggactggagtggatcggcgagatctacccaagatctaccaacacactgtataatgagaagttcaagggcaaggccaccctgacagcagaccggagctccaacaccgcctacatggagctgagaagcctgacatccgaggattctgccgtgtatttttgtgcacgcaccctgacagcacccttcgccttttggggacagggcaccctggtgacagtgagcgccgccaagaccacagcaccaagcgtgtatccactggcacccgtgtgcggcgataccacaggctctagcgtgaccctgggctgtctggtgaagggctacttccctgagccagtgaccctgacatggaacagcggctctctgtcctctggcgtgcacacctttcctgccgtgctgcagtccgatctgtatacactgagctcctctgtgaccgtgacaagctccacctggcccagccagtccatcacatgcaacgtggcccaccctgcctctagcaccaaggtggacaagaagatcgagccacggggccccacaatcaagccatgtccaccttgcaagtgtccagcacctaatctgctgggaggacctagcgtgttcatctttccacccaagatcaaggacgtgctgatgatctctctgagccctatcgtgacctgcgtggtggtggccgtgtctgaggacgatccagatgtgcagatcagctggttcgtgaacaatgtggaggtgcacaccgcccagacccagacacaccgggaggactacggctccacactgagagtggtgtctgccctgcccatccagcaccaggactggatgtccggcaaggagtttaagtgcaaggtgaacaataaggatctgccagcccccatcgagaggaccatctctaagcctaagggcagcgtgcgcgcaccacaggtgtatgtgctgcctccacccgaggaggagatgaccaagaagcaggtgacactgacgtgtatggtgaccgacttcatgccagaggatatctacgtggagtggaccaacaatggcaagacagagctgaactataagaatacagagcccgtgctggacagcgatggctcctactttatgtatagcaagctgagggtggagaagaagaactgggtggagcgcaattcctactcttgtagcgtggtgcacgagggcctgcacaaccaccacaccacaaagtccttttctagaacccccggcggtggaggtggctcaggaggaggcggttctaaccctgcagcacacctgaccggagcaaatgcatccctgatcggaatcggaggaccactgctgtgggagacaaggctgggactggccttcctgaggggactgacctaccacgatggcgccctggtgacaatggagccaggctactattacgtgtatagcaaggtgcagctgtccggagtgggatgcccacagggactggccaacggcctgcctatcacccacggcctgtataagcggacaagcagataccccaaggagctggagctgctggtgtcccggagatctccttgtggaagggccaacagctcccgcgtgtggtgggattctagcttcctgggaggagtggtgcacctggaggcaggcgaggaggtggtggtgcgggtgcctggcaatagactggtgaggccaagggacggaacccggtcttacttcggcgcctttatggtg

SEQ ID NO: 69 - DNA, 699 bp, synthetic construct
  misc_feature 1..699: note = DNA sequence of mu IgG2a Fc hole DANG
  source 1..699: mol_type = other DNA
gagccaaggggccccaccatcaagccatgccccccttgcaagtgtcctgcaccaaacctgctgggaggaccaagcgtgttcatctttccacccaagatcaaggacgtgctgatgatcagcctgtcccccatcgtgacatgcgtggtggtggccgtgtccgaggacgatcctgatgtgcagatctcttggttcgtgaacaatgtggaggtgcacaccgcccagacccagacacaccgggaggactatggctctacactgagagtggtgagcgccctgcccatccagcaccaggactggatgagcggcaaggagtttaagtgcaaggtgaacaataaggatctgcccgcccctatcgagcggaccatcagcaagcctaagggctccgtgagagccccacaggtgtacgtgctgcctccacccgaggaggagatgaccaagaagcaggtgacactgagctgtgccgtgaccgacttcatgcctgaggatatctacgtggagtggaccaacaatggcaagacagagctgaactataagaatacagagccagtgctggactccgatggctcttactttatggtgtccaagctgagggtggagaagaagaactgggtggagcgcaattcttatagctgctccgtggtgcacgagggcctgcacaatcaccacaccacaaagtctttcagcagaacccctggcaag

SEQ ID NO: 70 - DNA, 699 bp, synthetic construct
  misc_feature 1..699: note = DNA sequence of mu IgG2a Fc knob DANG
  source 1..699: mol_type = other DNA
gagccaaggggccccaccatcaagccatgccccccttgcaagtgtcctgcaccaaacctgctgggaggaccaagcgtgttcatctttccacccaagatcaaggacgtgctgatgatcagcctgtcccccatcgtgacatgcgtggtggtggccgtgtccgaggacgatcctgatgtgcagatctcttggttcgtgaacaatgtggaggtgcacaccgcccagacccagacacaccgggaggactacggctctacactgagagtggtgagcgccctgcccatccagcaccaggactggatgtccggcaaggagtttaagtgcaaggtgaacaataaggatctgcccgcccctatcgagcggaccatcagcaagcctaagggctccgtgagagccccacaggtgtatgtgctgcctccacccgaggaggagatgaccaagaagcaggtgacactgtggtgtatggtgaccgacttcatgcctgaggatatctacgtggagtggaccaacaatggcaagacagagctgaactataagaatacagagccagtgctggactccgatggctcttactttatgtattctaagctgagggtggagaagaagaactgggtggagcgcaattcttacagctgctccgtggtgcacgagggcctgcacaatcaccacaccacaaagtctttcagcagaacccctggcaag

SEQ ID NO: 71 - DNA, 699 bp, synthetic construct
  misc_feature 1..699: note = DNA sequence of mu IgG2a Fc knob
  source 1..699: mol_type = other DNA
gagccacgcggccccacaatcaagccatgccccccttgcaagtgtcctgcaccaaatctgctgggaggaccatccgtgttcatctttccacccaagatcaaggacgtgctgatgatcagcctgtccccaatcgtgacctgcgtggtcgtggacgtgagcgaggacgatcctgatgtgcagatctcctggttcgtgaacaatgtggaggtgcacaccgcccagacccagacacaccgggaggactacaactccacactgagagtggtgtctgccctgcccatccagcaccaggactggatgagcggcaaggagtttaagtgcaaggtgaacaataaggatctgcccgcccctatcgagcggacaatctctaagcctaagggcagcgtgagagccccacaggtgtatgtgctgcctccacccgaggaggagatgaccaagaagcaggtgacactgtggtgtatggtgaccgacttcatgcctgaggatatctatgtggagtggaccaacaatggcaagacagagctgaactacaagaatacagagccagtgctggactccgatggctcttacttcatgtacagcaagctgagggtggagaagaagaactgggtggagcgcaattcttacagctgctccgtggtgcacgagggcctgcacaaccaccacaccacaaagtcttttagccggacccctggcaag

SEQ ID NO: 72 - DNA, 1341 bp, synthetic construct
  misc_feature 1..1341: note = DNA sequence of anti-mu FAP HC mu IgG2a Fc DANG
  source 1..1341: mol_type = other DNA
caggtgcagctgcagcagtccggagcagagctggcaaggcctggagcctctgtgaacctgagctgcaaggcctccggctacaccttcacaaacaatggcatcaattggctgaagcagaggaccggacagggactggagtggatcggcgagatctacccaagatctaccaacacactgtataatgagaagttcaagggcaaggccaccctgacagcagaccggagctccaacaccgcctacatggagctgagaagcctgacatccgaggattctgccgtgtatttttgtgcacgcaccctgacagcacccttcgccttttggggacagggcaccctggtgacagtgagcgccgccaagaccacagcaccaagcgtgtatccactggcacccgtgtgcggcgataccacaggctctagcgtgaccctgggctgtctggtgaagggctacttccctgagccagtgaccctgacatggaacagcggctctctgtcctctggcgtgcacacctttcctgccgtgctgcagtccgatctgtatacactgagctcctctgtgaccgtgacaagctccacctggcccagccagtccatcacatgcaacgtggcccaccctgcctctagcaccaaggtggacaagaagatcgagccacggggccccacaatcaagccatgtccaccttgcaagtgtccagcacctaatctgctgggaggacctagcgtgttcatctttccacccaagatcaaggacgtgctgatgatctctctgagccctatcgtgacctgcgtggtggtggccgtgtctgaggacgatccagatgtgcagatcagctggttcgtgaacaatgtggaggtgcacaccgcccagacccagacacaccgggaggactacggctccacactgagagtggtgtctgccctgcccatccagcaccaggactggatgtccggcaaggagtttaagtgcaaggtgaacaataaggatctgccagcccccatcgagaggaccatctctaagcctaagggcagcgtgcgcgcaccacaggtgtatgtgctgcctccacccgaggaggagatgaccaagaagcaggtgacactgacgtgtatggtgaccgacttcatgccagaggatatctacgtggagtggaccaacaatggcaagacagagctgaactataagaatacagagcccgtgctggacagcgatggctcctactttatgtatagcaagctgagggtggagaagaagaactgggtggagcgcaattcctactcttgtagcgtggtgcacgagggcctgcacaaccaccacaccacaaagtccttttctagaacccccggcaag

SEQ ID NO: 73 - DNA, 2145 bp, synthetic construct
  misc_feature 1..2145: note = DNA sequence of mu scLIGHT-LTb2-mu IgG2a Fc hole DANG
  source 1..2145: mol_type = other DNA
aaccctgcagcacacctgaccggagcaaatgcatccctgatcggaatcggaggaccactgctgtgggagacaaggctgggactggccttcctgaggggactgacctaccacgatggcgccctggtgacaatggagccaggctactattacgtgtatagcaaggtgcagctgtccggagtgggatgcccacagggactggccaacggcctgcctatcacccacggcctgtataagcggacaagcagataccccaaggagctggagctgctggtgtcccggagatctccttgtggaagggccaacagctcccgcgtgtggtgggattctagcttcctgggaggagtggtgcacctggaggcaggcgaggaggtggtggtgcgggtgcctggcaatagactggtgaggccaagggacggaacccggtcttacttcggagcctttatggtgggaggcggtgggagtggtggcgggggatccggaggaggggggtcactgcctgccgctcacctgatcggcgcctggatgagcggccagggcctgagctgggaggcttctcaggaggaagccttcctgcggtccggcgcccagttcagccctacacacggcctggccctgccccaggatggcgtgtactacctgtactgccacgtgggctaccggggccggacccctcctgctggcagaagcagagccagatccctgaccctgcggagcgccctgtacagagccggcggagcttatggaagaggcagccctgagctgctgctggaaggcgctgaaaccgtgacccctgtcgtggaccccatcggatacggaagcctgtggtatacaagcgtgggattcggcggactggctcagctgagaagcggcgagcgggtgtacgtgaacatcagccaccccgacatggttgattaccggagaggaaagacattcttcggcgccgtgatggtcggaggctctggactgcccgccgcccacctgatcggcgcctggatgtctggccaaggcctcagctgggaagccagccaggaggaagcttttctgagaagcggcgcccaattttcccctacccatggcctggccctgcctcaggacggcgtgtattacctgtactgtcacgtgggctacagaggcagaaccccacctgccggcagaagccgggccagatctctgacactgcgctctgccctgtacagagccggcggcgcctacggcagaggctccccagagctgctgctcgagggcgccgagacagtgacccccgtggtggaccctatcggctacggcagcctgtggtacaccagcgtgggcttcggcggcctggcccagctgcgcagcggagagagagtgtacgtgaacatttctcaccctgatatggtggactacaggcggggcaagaccttcttcggagccgtgatggtggggggaagcggaggaggaggctccgagccacgcggccccacaatcaagccatgccccccttgcaagtgtcctgcaccaaatctgctgggaggaccatccgtgttcatctttccacccaagatcaaggacgtgctgatgatcagcctgtccccaatcgtgacctgcgtggtcgtggccgtgagcgaggacgatcctgatgtgcagatctcctggttcgtgaacaatgtggaggtgcacaccgcccagacccagacacaccgggaggactacggctccacactgagagtggtgtctgccctgcccatccagcaccaggactggatgagcggcaaggagtttaagtgcaaggtgaacaataaggatctgcccgcccctatcgagcggacaatctctaagcctaagggcagcgtgagagccccacaggtgtatgtgctgcctccacccgaggaggagatgaccaagaagcaggtgacactgtcttgtgccgtgaccgacttcatgcctgaggatatctatgtggagtggaccaacaatggcaagacagagctgaactacaagaatacagagccagtgctggactccgatggctcttacttcatggtgagcaagctgagggtggagaagaagaactgggtggagcgcaattcttacagctgctccgtggtgcacgagggcctgcacaaccaccacaccacaaagtcttttagccggacccctggcaag

SEQ ID NO: 74 - DNA, 2145 bp, synthetic construct
  misc_feature 1..2145: note = DNA sequence of mu scLIGHT-LTb2-mu IgG2a Fc hole
  source 1..2145: mol_type = other DNA
aaccctgcagcacacctgaccggagcaaatgcatccctgatcggaatcggaggaccactgctgtgggagacaaggctgggactggccttcctgaggggactgacctaccacgatggcgccctggtgacaatggagccaggctactattacgtgtatagcaaggtgcagctgtccggagtgggatgcccacagggactggccaacggcctgcctatcacccacggcctgtataagcggacaagcagataccccaaggagctggagctgctggtgtcccggagatctccttgtggaagggccaacagctcccgcgtgtggtgggattctagcttcctgggaggagtggtgcacctggaggcaggcgaggaggtggtggtgcgggtgcctggcaatagactggtgaggccaagggacggaacccggtcttacttcggagcctttatggtgggaggcggtgggagtggtggcgggggatccggaggaggggggtcactgcctgccgctcacctgatcggcgcctggatgagcggccagggcctgagctgggaggcttctcaggaggaagccttcctgcggtccggcgcccagttcagccctacacacggcctggccctgccccaggatggcgtgtactacctgtactgccacgtgggctaccggggccggacccctcctgctggcagaagcagagccagatccctgaccctgcggagcgccctgtacagagccggcggagcttatggaagaggcagccctgagctgctgctggaaggcgctgaaaccgtgacccctgtcgtggaccccatcggatacggaagcctgtggtatacaagcgtgggattcggcggactggctcagctgagaagcggcgagcgggtgtacgtgaacatcagccaccccgacatggttgattaccggagaggaaagacattcttcggcgccgtgatggtcggaggctctggactgcccgccgcccacctgatcggcgcctggatgtctggccaaggcctcagctgggaagccagccaggaggaagcttttctgagaagcggcgcccaattttcccctacccatggcctggccctgcctcaggacggcgtgtattacctgtactgtcacgtgggctacagaggcagaaccccacctgccggcagaagccgggccagatctctgacactgcgctctgccctgtacagagccggcggcgcctacggcagaggctccccagagctgctgctcgagggcgccgagacagtgacccccgtggtggaccctatcggctacggcagcctgtggtacaccagcgtgggcttcggcggcctggcccagctgcgcagcggagagagagtgtacgtgaacatttctcaccctgatatggtggactacaggcggggcaagaccttcttcggagccgtgatggtggggggaagcggaggaggaggctccgagccacgcggccccacaatcaagccatgccccccttgcaagtgtcctgcaccaaatctgctgggaggaccatccgtgttcatctttccacccaagatcaaggacgtgctgatgatcagcctgtccccaatcgtgacctgcgtggtcgtggacgtgagcgaggacgatcctgatgtgcagatctcctggttcgtgaacaatgtggaggtgcacaccgcccagacccagacacaccgggaggactacaactccacactgagagtggtgtctgccctgcccatccagcaccaggactggatgagcggcaaggagtttaagtgcaaggtgaacaataaggatctgcccgcccctatcgagcggacaatctctaagcctaagggcagcgtgagagccccacaggtgtatgtgctgcctccacccgaggaggagatgaccaagaagcaggtgacactgtcttgtgccgtgaccgacttcatgcctgaggatatctatgtggagtggaccaacaatggcaagacagagctgaactacaagaatacagagccagtgctggactccgatggctcttacttcatggtgagcaagctgagggtggagaagaagaactgggtggagcgcaattcttacagctgctccgtggtgcacgagggcctgcacaaccaccacaccacaaagtcttttagccggacccctggcaag

SEQ ID NO: 75 - protein, 222 aa, synthetic construct
  REGION 1..222: note = anti-hu FAP HC(heavy chain)
QVQLVQSGAEVKKPGASVKVSCKTSRYTFTEYTIHWVRQAPGQRLEWIGGINPNNGIPNYNQKFKGRVTITVDTSASTAYMELSSLRSEDTAVYYCARRRIAYGYDEGHAMDYWGQGTLVTVSSASTKGPSVFPLAPSSKSTSGGTAALGCLVKDYFPEPVTVSWNSGALTSGVHTFPAVLQSSGLYSLSSVVTVPSSSLGTQTYICNVNHKPSNTKVDKKV

SEQ ID NO: 76 - protein, 117 aa, synthetic construct
  REGION 1..117: note = anti-mu FAP HC(heavy chain)
QVQLQQSGAELARPGASVNLSCKASGYTFTNNGINWLKQRTGQGLEWIGEIYPRSTNTLYNEKFKGKATLTADRSSNTAYMELRSLTSEDSAVYFCARTLTAPFAFWGQGTLVTVSA

SEQ ID NO: 77 - protein, 240 aa, synthetic construct
  REGION 1..240: note = hu LIGHT protein origin
MEESVVRPSVFVVDGQTDIPFTRLGRSHRRQSCSVARVGLGLLLLLMGAGLAVQGWFLLQLHWRLGEMVTRLPDGPAGSWEQLIQERRSHEVNPAAHLTGANSSLTGSGGPLLWETQLGLAFLRGLSYHDGALVVTKAGYYYIYSKVQLGGVGCPLGLASTITHGLYKRTPRYPEELELLVSQQSPCGRATSSSRVWWDSSFLGGVVHLEAGEKVVVRVLDERLVRLRDGTRSYFGAFMV

SEQ ID NO: 78 - protein, 150 aa, synthetic construct
  REGION 1..150: note = hu LIGHT protein soluble form
EVNPAAHLTGANSSLTGSGGPLLWETQLGLAFLRGLSYHDGALVVTKAGYYYIYSKVQLGGVGCPLGLASTITHGLYKRTPRYPEELELLVSQQSPCGRATSSSRVWWDSSFLGGVVHLEAGEKVVVRVLDERLVRLRDGTRSYFGAFMV

SEQ ID NO: 79 - protein, 304 aa, synthetic construct
  REGION 1..304: note = hu scLIGHT2(dimer of LIGHT)
EVNPAAHLTGANSSLTGSGGPLLWETQLGLAFLRGLSYHDGALVVTKAGYYYIYSKVQLGGVGCPLGLASTITHGLYKRTPRYPEELELLVSQQSPCGRATSSSRVWWDSSFLGGVVHLEAGEKVVVRVLDERLVRLRDGTRSYFGAFMVGGSGEVNPAAHLTGANSSLTGSGGPLLWETQLGLAFLRGLSYHDGALVVTKAGYYYIYSKVQLGGVGCPLGLASTITHGLYKRTPRYPEELELLVSQQSPCGRATSSSRVWWDSSFLGGVVHLEAGEKVVVRVLDERLVRLRDGTRSYFGAFMV

SEQ ID NO: 80 - protein, 458 aa, synthetic construct
  REGION 1..458: note = hu scLIGHT3(trimer of LIGHT)
EVNPAAHLTGANSSLTGSGGPLLWETQLGLAFLRGLSYHDGALVVTKAGYYYIYSKVQLGGVGCPLGLASTITHGLYKRTPRYPEELELLVSQQSPCGRATSSSRVWWDSSFLGGVVHLEAGEKVVVRVLDERLVRLRDGTRSYFGAFMVGGSGEVNPAAHLTGANSSLTGSGGPLLWETQLGLAFLRGLSYHDGALVVTKAGYYYIYSKVQLGGVGCPLGLASTITHGLYKRTPRYPEELELLVSQQSPCGRATSSSRVWWDSSFLGGVVHLEAGEKVVVRVLDERLVRLRDGTRSYFGAFMVGGSGEVNPAAHLTGANSSLTGSGGPLLWETQLGLAFLRGLSYHDGALVVTKAGYYYIYSKVQLGGVGCPLGLASTITHGLYKRTPRYPEELELLVSQQSPCGRATSSSRVWWDSSFLGGVVHLEAGEKVVVRVLDERLVRLRDGTRSYFGAFMV

SEQ ID NO: 81 - protein, 150 aa, synthetic construct
  REGION 1..150: note = hu LIGHT(226-231 mutant)
EVNPAAHLTGANSSLTGSGGPLLWETQLGLAFLRGLSYHDGALVVTKAGYYYIYSKVQLGGVGCPLGLASTITHGLYKRTPRYPEELELLVSQQSPCGRATSSSRVWWDSSFLGGVVHLEAGEKVVVRVLDERLVDYTKEDRSYFGAFMV

SEQ ID NO: 82 - protein, 458 aa, synthetic construct
  REGION 1..458: note = hu scLIGHT(226-231)3
EVNPAAHLTGANSSLTGSGGPLLWETQLGLAFLRGLSYHDGALVVTKAGYYYIYSKVQLGGVGCPLGLASTITHGLYKRTPRYPEELELLVSQQSPCGRATSSSRVWWDSSFLGGVVHLEAGEKVVVRVLDERLVDYTKEDRSYFGAFMVGGSGEVNPAAHLTGANSSLTGSGGPLLWETQLGLAFLRGLSYHDGALVVTKAGYYYIYSKVQLGGVGCPLGLASTITHGLYKRTPRYPEELELLVSQQSPCGRATSSSRVWWDSSFLGGVVHLEAGEKVVVRVLDERLVDYTKEDRSYFGAFMVGGSGEVNPAAHLTGANSSLTGSGGPLLWETQLGLAFLRGLSYHDGALVVTKAGYYYIYSKVQLGGVGCPLGLASTITHGLYKRTPRYPEELELLVSQQSPCGRATSSSRVWWDSSFLGGVVHLEAGEKVVVRVLDERLVDYTKEDRSYFGAFMV

SEQ ID NO: 83 - protein, 150 aa, synthetic construct
  REGION 1..150: note = hu LIGHT(L118K, G119E)
EVNPAAHLTGANSSLTGSGGPLLWETQKELAFLRGLSYHDGALVVTKAGYYYIYSKVQLGGVGCPLGLASTITHGLYKRTPRYPEELELLVSQQSPCGRATSSSRVWWDSSFLGGVVHLEAGEKVVVRVLDERLVRLRDGTRSYFGAFMV

SEQ ID NO: 84 - protein, 458 aa, synthetic construct
  REGION 1..458: note = hu scLIGHT-LIGHT(L118K, G119E)2
EVNPAAHLTGANSSLTGSGGPLLWETQLGLAFLRGLSYHDGALVVTKAGYYYIYSKVQLGGVGCPLGLASTITHGLYKRTPRYPEELELLVSQQSPCGRATSSSRVWWDSSFLGGVVHLEAGEKVVVRVLDERLVRLRDGTRSYFGAFMVGGSGEVNPAAHLTGANSSLTGSGGPLLWETQKELAFLRGLSYHDGALVVTKAGYYYIYSKVQLGGVGCPLGLASTITHGLYKRTPRYPEELELLVSQQSPCGRATSSSRVWWDSSFLGGVVHLEAGEKVVVRVLDERLVRLRDGTRSYFGAFMVGGSGEVNPAAHLTGANSSLTGSGGPLLWETQKELAFLRGLSYHDGALVVTKAGYYYIYSKVQLGGVGCPLGLASTITHGLYKRTPRYPEELELLVSQQSPCGRATSSSRVWWDSSFLGGVVHLEAGEKVVVRVLDERLVRLRDGTRSYFGAFMV

SEQ ID NO: 85 - protein, 150 aa, synthetic construct
  REGION 1..150: note = hu LIGHT(195-198 mutant)
EVNPAAHLTGANSSLTGSGGPLLWETQLGLAFLRGLSYHDGALVVTKAGYYYIYSKVQLGGVGCPLGLASTITHGLYKRTPRYPEELELLVSQQSPCGRATSSSSNWFDSSFLGGVVHLEAGEKVVVRVLDERLVRLRDGTRSYFGAFMV

SEQ ID NO: 86 - protein, 458 aa, synthetic construct
  REGION 1..458: note = hu scLIGHT(195-198)3
EVNPAAHLTGANSSLTGSGGPLLWETQLGLAFLRGLSYHDGALVVTKAGYYYIYSKVQLGGVGCPLGLASTITHGLYKRTPRYPEELELLVSQQSPCGRATSSSSNWFDSSFLGGVVHLEAGEKVVVRVLDERLVRLRDGTRSYFGAFMVGGSGEVNPAAHLTGANSSLTGSGGPLLWETQLGLAFLRGLSYHDGALVVTKAGYYYIYSKVQLGGVGCPLGLASTITHGLYKRTPRYPEELELLVSQQSPCGRATSSSSNWFDSSFLGGVVHLEAGEKVVVRVLDERLVRLRDGTRSYFGAFMVGGSGEVNPAAHLTGANSSLTGSGGPLLWETQLGLAFLRGLSYHDGALVVTKAGYYYIYSKVQLGGVGCPLGLASTITHGLYKRTPRYPEELELLVSQQSPCGRATSSSSNWFDSSFLGGVVHLEAGEKVVVRVLDERLVRLRDGTRSYFGAFMV

SEQ ID NO: 87 - protein, 244 aa, synthetic construct
  REGION 1..244: note = Lymphotoxin beta(LTb) origin
MGALGLEGRGGRLQGRGSLLLAVAGATSLVTLLLAVPITVLAVLALVPQDQGGLVTETADPGAQAQQGLGFQKLPEEEPETDLSPGLPAAHLIGAPLKGQGLGWETTKEQAFLTSGTQFSDAEGLALPQDGLYYLYCLVGYRGRAPPGGGDPQGRSVTLRSSLYRAGGAYGPGTPELLLEGAETVTPVLDPARRQGYGPLWYTSVGFGGLVQLRRGERVYVNISHPDMVDFARGKTFFGAVMVG

SEQ ID NO: 88 - protein, 157 aa, synthetic construct
  REGION 1..157: note = LTb
LPAAHLIGAPLKGQGLGWETTKEQAFLTSGTQFSDAEGLALPQDGLYYLYCLVGYRGRAPPGGGDPQGRSVTLRSSLYRAGGAYGPGTPELLLEGAETVTPVLDPARRQGYGPLWYTSVGFGGLVQLRRGERVYVNISHPDMVDFARGKTFFGAVMV

SEQ ID NO: 89 - protein, 472 aa, synthetic construct
  REGION 1..472: note = hu scLIGHT-LTb2
EVNPAAHLTGANSSLTGSGGPLLWETQLGLAFLRGLSYHDGALVVTKAGYYYIYSKVQLGGVGCPLGLASTITHGLYKRTPRYPEELELLVSQQSPCGRATSSSRVWWDSSFLGGVVHLEAGEKVVVRVLDERLVRLRDGTRSYFGAFMVGGSGLPAAHLIGAPLKGQGLGWETTKEQAFLTSGTQFSDAEGLALPQDGLYYLYCLVGYRGRAPPGGGDPQGRSVTLRSSLYRAGGAYGPGTPELLLEGAETVTPVLDPARRQGYGPLWYTSVGFGGLVQLRRGERVYVNISHPDMVDFARGKTFFGAVMVGGSGLPAAHLIGAPLKGQGLGWETTKEQAFLTSGTQFSDAEGLALPQDGLYYLYCLVGYRGRAPPGGGDPQGRSVTLRSSLYRAGGAYGPGTPELLLEGAETVTPVLDPARRQGYGPLWYTSVGFGGLVQLRRGERVYVNISHPDMVDFARGKTFFGAVMV

SEQ ID NO: 90 - protein, 483 aa, synthetic construct
  REGION 1..483: note = hu scLIGHT(226-231)-LTb2
EVNPAAHLTGANSSLTGSGGPLLWETQLGLAFLRGLSYHDGALVVTKAGYYYIYSKVQLGGVGCPLGLASTITHGLYKRTPRYPEELELLVSQQSPCGRATSSSRVWWDSSFLGGVVHLEAGEKVVVRVLDERLVDYTKEDRSYFGAFMVGGGGSGGGGSGGGGSLPAAHLIGAPLKGQGLGWETTKEQAFLTSGTQFSDAEGLALPQDGLYYLYCLVGYRGRAPPGGGDPQGRSVTLRSSLYRAGGAYGPGTPELLLEGAETVTPVLDPARRQGYGPLWYTSVGFGGLVQLRRGERVYVNISHPDMVDFARGKTFFGAVMVGGSGLPAAHLIGAPLKGQGLGWETTKEQAFLTSGTQFSDAEGLALPQDGLYYLYCLVGYRGRAPPGGGDPQGRSVTLRSSLYRAGGAYGPGTPELLLEGAETVTPVLDPARRQGYGPLWYTSVGFGGLVQLRRGERVYVNISHPDMVDFARGKTFFGAVMV

SEQ ID NO: 91 - protein, 483 aa, synthetic construct
  REGION 1..483: note = hu scLIGHT(195-198)-LTb2
EVNPAAHLTGANSSLTGSGGPLLWETQLGLAFLRGLSYHDGALVVTKAGYYYIYSKVQLGGVGCPLGLASTITHGLYKRTPRYPEELELLVSQQSPCGRATSSSSNWFDSSFLGGVVHLEAGEKVVVRVLDERLVRLRDGTRSYFGAFMVGGGGSGGGGSGGGGSLPAAHLIGAPLKGQGLGWETTKEQAFLTSGTQFSDAEGLALPQDGLYYLYCLVGYRGRAPPGGGDPQGRSVTLRSSLYRAGGAYGPGTPELLLEGAETVTPVLDPARRQGYGPLWYTSVGFGGLVQLRRGERVYVNISHPDMVDFARGKTFFGAVMVGGSGLPAAHLIGAPLKGQGLGWETTKEQAFLTSGTQFSDAEGLALPQDGLYYLYCLVGYRGRAPPGGGDPQGRSVTLRSSLYRAGGAYGPGTPELLLEGAETVTPVLDPARRQGYGPLWYTSVGFGGLVQLRRGERVYVNISHPDMVDFARGKTFFGAVMV

SEQ ID NO: 92 - protein, 239 aa, synthetic construct
  REGION 1..239: note = mu LIGHT protein origin
MESVVQPSVFVVDGQTDIPFRRLEQNHRRRRCGTVQVSLALVLLLGAGLATQGWFLLRLHQRLGDIVAHLPDGGKGSWEKLIQDQRSHQANPAAHLTGANASLIGIGGPLLWETRLGLAFLRGLTYHDGALVTMEPGYYYVYSKVQLSGVGCPQGLANGLPITHGLYKRTSRYPKELELLVSRRSPCGRANSSRVWWDSSFLGGVVHLEAGEEVVVRVPGNRLVRPRDGTRSYFGAFMV

SEQ ID NO: 93 - protein, 149 aa, synthetic construct
  REGION 1..149: note = mu LIGHT protein soluble form
NPAAHLTGANASLIGIGGPLLWETRLGLAFLRGLTYHDGALVTMEPGYYYVYSKVQLSGVGCPQGLANGLPITHGLYKRTSRYPKELELLVSRRSPCGRANSSRVWWDSSFLGGVVHLEAGEEVVVRVPGNRLVRPRDGTRSYFGAFMV

SEQ ID NO: 94 - protein, 302 aa, synthetic construct
  REGION 1..302: note = mu scLIGHT2
NPAAHLTGANASLIGIGGPLLWETRLGLAFLRGLTYHDGALVTMEPGYYYVYSKVQLSGVGCPQGLANGLPITHGLYKRTSRYPKELELLVSRRSPCGRANSSRVWWDSSFLGGVVHLEAGEEVVVRVPGNRLVRPRDGTRSYFGAFMVGGSGNPAAHLTGANASLIGIGGPLLWETRLGLAFLRGLTYHDGALVTMEPGYYYVYSKVQLSGVGCPQGLANGLPITHGLYKRTSRYPKELELLVSRRSPCGRANSSRVWWDSSFLGGVVHLEAGEEVVVRVPGNRLVRPRDGTRSYFGAFMV

SEQ ID NO: 95 - protein, 455 aa, synthetic construct
  REGION 1..455: note = mu scLIGHT3
NPAAHLTGANASLIGIGGPLLWETRLGLAFLRGLTYHDGALVTMEPGYYYVYSKVQLSGVGCPQGLANGLPITHGLYKRTSRYPKELELLVSRRSPCGRANSSRVWWDSSFLGGVVHLEAGEEVVVRVPGNRLVRPRDGTRSYFGAFMVGGSGNPAAHLTGANASLIGIGGPLLWETRLGLAFLRGLTYHDGALVTMEPGYYYVYSKVQLSGVGCPQGLANGLPITHGLYKRTSRYPKELELLVSRRSPCGRANSSRVWWDSSFLGGVVHLEAGEEVVVRVPGNRLVRPRDGTRSYFGAFMVGGSGNPAAHLTGANASLIGIGGPLLWETRLGLAFLRGLTYHDGALVTMEPGYYYVYSKVQLSGVGCPQGLANGLPITHGLYKRTSRYPKELELLVSRRSPCGRANSSRVWWDSSFLGGVVHLEAGEEVVVRVPGNRLVRPRDGTRSYFGAFMV

SEQ ID NO: 96 - protein, 149 aa, synthetic construct
  REGION 1..149: note = mu LIGHT(225-230 mutant)
NPAAHLTGANASLIGIGGPLLWETRLGLAFLRGLTYHDGALVTMEPGYYYVYSKVQLSGVGCPQGLANGLPITHGLYKRTSRYPKELELLVSRRSPCGRANSSRVWWDSSFLGGVVHLEAGEEVVVRVPGNRLVDYTKEDRSYFGAFMV

SEQ ID NO: 97 - protein, 455 aa, synthetic construct
  REGION 1..455: note = mu scLIGHT(225-230)3
NPAAHLTGANASLIGIGGPLLWETRLGLAFLRGLTYHDGALVTMEPGYYYVYSKVQLSGVGCPQGLANGLPITHGLYKRTSRYPKELELLVSRRSPCGRANSSRVWWDSSFLGGVVHLEAGEEVVVRVPGNRLVDYTKEDRSYFGAFMVGGSGNPAAHLTGANASLIGIGGPLLWETRLGLAFLRGLTYHDGALVTMEPGYYYVYSKVQLSGVGCPQGLANGLPITHGLYKRTSRYPKELELLVSRRSPCGRANSSRVWWDSSFLGGVVHLEAGEEVVVRVPGNRLVDYTKEDRSYFGAFMVGGSGNPAAHLTGANASLIGIGGPLLWETRLGLAFLRGLTYHDGALVTMEPGYYYVYSKVQLSGVGCPQGLANGLPITHGLYKRTSRYPKELELLVSRRSPCGRANSSRVWWDSSFLGGVVHLEAGEEVVVRVPGNRLVDYTKEDRSYFGAFMV

SEQ ID NO: 98 - protein, 149 aa, synthetic construct
  REGION 1..149: note = mu LIGHT(194-197 mutant)
NPAAHLTGANASLIGIGGPLLWETRLGLAFLRGLTYHDGALVTMEPGYYYVYSKVQLSGVGCPQGLANGLPITHGLYKRTSRYPKELELLVSRRSPCGRANSSNNWFDSSFLGGVVHLEAGEEVVVRVPGNRLVRPRDGTRSYFGAFMV

SEQ ID NO: 99 - protein, 455 aa, synthetic construct
  REGION 1..455: note = mu scLIGHT(194-197)3
NPAAHLTGANASLIGIGGPLLWETRLGLAFLRGLTYHDGALVTMEPGYYYVYSKVQLSGVGCPQGLANGLPITHGLYKRTSRYPKELELLVSRRSPCGRANSSNNWFDSSFLGGVVHLEAGEEVVVRVPGNRLVRPRDGTRSYFGAFMVGGSGNPAAHLTGANASLIGIGGPLLWETRLGLAFLRGLTYHDGALVTMEPGYYYVYSKVQLSGVGCPQGLANGLPITHGLYKRTSRYPKELELLVSRRSPCGRANSSNNWFDSSFLGGVVHLEAGEEVVVRVPGNRLVRPRDGTRSYFGAFMVGGSGNPAAHLTGANASLIGIGGPLLWETRLGLAFLRGLTYHDGALVTMEPGYYYVYSKVQLSGVGCPQGLANGLPITHGLYKRTSRYPKELELLVSRRSPCGRANSSNNWFDSSFLGGVVHLEAGEEVVVRVPGNRLVRPRDGTRSYFGAFMV

SEQ ID NO: 100 - protein, 474 aa, synthetic construct
  REGION 1..474: note = mu scLIGHT-LTb2
NPAAHLTGANASLIGIGGPLLWETRLGLAFLRGLTYHDGALVTMEPGYYYVYSKVQLSGVGCPQGLANGLPITHGLYKRTSRYPKELELLVSRRSPCGRANSSRVWWDSSFLGGVVHLEAGEEVVVRVPGNRLVRPRDGTRSYFGAFMVGGGGSGGGGSGGGGSLPAAHLIGAWMSGQGLSWEASQEEAFLRSGAQFSPTHGLALPQDGVYYLYCHVGYRGRTPPAGRSRARSLTLRSALYRAGGAYGRGSPELLLEGAETVTPVVDPIGYGSLWYTSVGFGGLAQLRSGERVYVNISHPDMVDYRRGKTFFGAVMVGGSGLPAAHLIGAWMSGQGLSWEASQEEAFLRSGAQFSPTHGLALPQDGVYYLYCHVGYRGRTPPAGRSRARSLTLRSALYRAGGAYGRGSPELLLEGAETVTPVVDPIGYGSLWYTSVGFGGLAQLRSGERVYVNISHPDMVDYRRGKTFFGAVMV

SEQ ID NO: 101 - protein, 5 aa, synthetic construct
  REGION 1..5: note = anti-hu FAP HCDR1
EYTIH

SEQ ID NO: 102 - protein, 17 aa, synthetic construct
  REGION 1..17: note = anti-hu FAP HCDR2
GINPNNGIPNYNQKFKG

SEQ ID NO: 103 - protein, 15 aa, synthetic construct
  REGION 1..15: note = anti-hu FAP HCDR3
RRIAYGYDEGHAMDY

SEQ ID NO: 104 - protein, 17 aa, synthetic construct
  REGION 1..17: note = anti-hu FAP LCDR1
KSSQSLLYSRNQKNYLA

SEQ ID NO: 105 - protein, 7 aa, synthetic construct
  REGION 1..7: note = anti-hu FAP LCDR2
WASTRES

SEQ ID NO: 106 - protein, 9 aa, synthetic construct
  REGION 1..9: note = anti-hu FAP LCDR3
QQYFSYPLT

SEQ ID NO: 107 - protein, 124 aa, synthetic construct
  REGION 1..124: note = anti-hu FAP HCVR
QVQLVQSGAEVKKPGASVKVSCKTSRYTFTEYTIHWVRQAPGQRLEWIGGINPNNGIPNYNQKFKGRVTITVDTSASTAYMELSSLRSEDTAVYYCARRRIAYGYDEGHAMDYWGQGTLVTVSS

SEQ ID NO: 108 - protein, 113 aa, synthetic construct
  REGION 1..113: note = anti-hu FAP LCVR
DIVMTQSPDSLAVSLGERATINCKSSQSLLYSRNQKNYLAWYQQKPGQPPKLLIFWASTRESGVPDRFSGSGFGTDFTLTISSLQAEDVAVYYCQQYFSYPLTFGQGTKVEIK

SEQ ID NO: 109 - protein, 5 aa, synthetic construct
  REGION 1..5: note = anti-mu FAP HCDR1
NNGIN

SEQ ID NO: 110 - protein, 17 aa, synthetic construct
  REGION 1..17: note = anti-mu FAP HCDR2
EIYPRSTNTLYNEKFKG

SEQ ID NO: 111 - protein, 8 aa, synthetic construct
  REGION 1..8: note = anti-mu FAP HCDR3
TLTAPFAF

SEQ ID NO: 112 - protein, 10 aa, synthetic construct
  REGION 1..10: note = anti-mu FAP LCDR1
SASSGVNFMH

SEQ ID NO: 113 - protein, 7 aa, synthetic construct
  REGION 1..7: note = anti-mu FAP LCDR2
DTSKLAS

SEQ ID NO: 114 - protein, 9 aa, synthetic construct
  REGION 1..9: note = anti-mu FAP LCDR3
QQWSFNPPT

SEQ ID NO: 115 - protein, 117 aa, synthetic construct; identical to SEQ ID NO: 76
  REGION 1..117: note = anti-mu FAP HCVR

SEQ ID NO: 116 - protein, 107 aa, synthetic construct
  REGION 1..107: note = anti-mu FAP LCVR
QIVLTQSPAIMSASPGEKVTMTCSASSGVNFMHWYQQKSGTSPKRWIFDTSKLASGVPARFSGSGSGTSYSLTISSMEAEDAATYYCQQWSFNPPTFGGGTKLEIKR

SEQ ID NO: 117 - protein, 23 aa, synthetic construct
  REGION 1..23: note = hu IgG1 Hinge 1
EPKSCDKTHTCPPCPAPELLGGP

SEQ ID NO: 118 - protein, 18 aa, synthetic construct
  REGION 1..18: note = hu IgG1 Hinge 2
DKTHTCPPCPAPELLGGP

SEQ ID NO: 119 - protein, 16 aa, synthetic construct
  REGION 1..16: note = mu IgG2a Hinge
EPRGPTIKPCPPCKCP

SEQ ID NO: 120 - protein, 9 aa, synthetic construct
  REGION 1..9: note = Peptide Linker No. 1
GGGSGGGGS

SEQ ID NO: 121 - protein, 4 aa, synthetic construct
  REGION 1..4: note = Peptide Linker No. 2
GGGS

SEQ ID NO: 122 - protein, 4 aa, synthetic construct
  REGION 1..4: note = Peptide Linker No.3
GGSG

SEQ ID NO: 123 - protein, 8 aa, synthetic construct
  REGION 1..8: note = Peptide Linker No.4
GGSGGGGS

SEQ ID NO: 124 - protein, 15 aa, synthetic construct
  REGION 1..15: note = Peptide Linker No.5
GGGGSGGGGSGGGGS

SEQ ID NO: 125 - protein, 20 aa, synthetic construct
  REGION 1..20: note = Peptide Linker No.6
GGGGSGGGGSGGGGSGGGGS

SEQ ID NO: 126 - protein, 10 aa, synthetic construct
  REGION 1..10: note = Peptide Linker No.7
GGGGSGGGGS

SEQ ID NO: 127 - protein, 5 aa, synthetic construct
  REGION 1..5: note = NG-641 HCDR1
EYTIH

SEQ ID NO: 128 - protein, 17 aa, synthetic construct
  REGION 1..17: note = NG-641 HCDR2
GINPNNGIPNYNQKFKG

SEQ ID NO: 129 - protein, 15 aa, synthetic construct
  REGION 1..15: note = NG-641 HCDR3
RRIAYGYDEGHAMDY

SEQ ID NO: 130 - protein, 17 aa, synthetic construct
  REGION 1..17: note = NG-641 LCDR1
KSSQSLLYSRNQKNYLA

SEQ ID NO: 131 - protein, 7 aa, synthetic construct
  REGION 1..7: note = NG-641 LCDR2
WASTRES

SEQ ID NO: 132 - protein, 9 aa, synthetic construct
  REGION 1..9: note = NG-641 LCDR3
QQYFSYPLT

SEQ ID NO: 133 - protein, 5 aa, synthetic construct
  REGION 1..5: note = 28H1 HCDR1
SHAMS

SEQ ID NO: 134 - protein, 16 aa, synthetic construct
  REGION 1..16: note = 28H1 HCDR2
AIWASGEQYYADSVKG

SEQ ID NO: 135 - protein, 8 aa, synthetic construct
  REGION 1..8: note = 28H1 HCDR3
GWLGNFDY

SEQ ID NO: 136 - protein, 12 aa, synthetic construct
  REGION 1..12: note = 28H1 LCDR1
RASQSVSRSYLA

SEQ ID NO: 137 - protein, 7 aa, synthetic construct
  REGION 1..7: note = 28H1 LCDR2
GASTRAT

SEQ ID NO: 138 - protein, 9 aa, synthetic construct
  REGION 1..9: note = 28H1 LCDR3
QQGQVIPPT

SEQ ID NO: 139 - protein, 5 aa, synthetic construct
  REGION 1..5: note = 4B9 HCDR1
SYAMS

SEQ ID NO: 140 - protein, 17 aa, synthetic construct
  REGION 1..17: note = 4B9 HCDR2
AIIGSGASTYYADSVKG

SEQ ID NO: 141 - protein, 8 aa, synthetic construct
  REGION 1..8: note = 4B9 HCDR3
GWFGGFNY

SEQ ID NO: 142 - protein, 12 aa, synthetic construct
  REGION 1..12: note = 4B9 LCDR1
RASQSVTSSYLA

SEQ ID NO: 143 - protein, 7 aa, synthetic construct
  REGION 1..7: note = 4B9 LCDR2
VGSRRAT

SEQ ID NO: 144 - protein, 9 aa, synthetic construct
  REGION 1..9: note = 4B9 LCDR3
QQGIMLPPT

SEQ ID NO: 145 - protein, 5 aa, synthetic construct
  REGION 1..5: note = OMTX-705 HCDR1
ENIIH

SEQ ID NO: 146 - protein, 17 aa, synthetic construct
  REGION 1..17: note = OMTX-705 HCDR2
WFHPGSGSIKYNEKFKD

SEQ ID NO: 147 - protein, 11 aa, synthetic construct
  REGION 1..11: note = OMTX-705 HCDR3
HGGTGRGAMDY

SEQ ID NO: 148 - protein, 15 aa, synthetic construct
  REGION 1..15: note = OMTX-705 LCDR1
RASKSVSTSAYSYMH

SEQ ID NO: 149 - protein, 7 aa, synthetic construct
  REGION 1..7: note = OMTX-705 LCDR2
LASNLES

SEQ ID NO: 150 - protein, 9 aa, synthetic construct
  REGION 1..9: note = OMTX-705 LCDR3
QHSRELPYT

SEQ ID NO: 151 - protein, 5 aa, synthetic construct
  REGION 1..5: note = 3F2 HCDR1
SYAMS

SEQ ID NO: 152 - protein, 16 aa, synthetic construct
  REGION 1..16: note = 3F2 HCDR2
AISGSGGSTYYADSVK

SEQ ID NO: 153 - protein, 8 aa, synthetic construct
  REGION 1..8: note = 3F2 HCDR3
YCAKGWFG

SEQ ID NO: 154 - protein, 11 aa, synthetic construct
  REGION 1..11: note = 3F2 LCDR1
RASQSVTSSYL

SEQ ID NO: 155 - protein, 7 aa, synthetic construct
  REGION 1..7: note = 3F2 LCDR2
NVGSRRA

SEQ ID NO: 156 - protein, 9 aa, synthetic construct
  REGION 1..9: note = 3F2 LCDR3
CQQGIMLPP

SEQ ID NO: 157 - protein, 5 aa, synthetic construct
  REGION 1..5: note = 4G8 HCDR1
SYAMS

SEQ ID NO: 158 - protein, 16 aa, synthetic construct
  REGION 1..16: note = 4G8 HCDR2
AISGSGGSTYYADSVK

SEQ ID NO: 159 - protein, 8 aa, synthetic construct
  REGION 1..8: note = 4G8 HCDR3
YCAKGWLG

SEQ ID NO: 160 - protein, 11 aa, synthetic construct
  REGION 1..11: note = 4G8 LCDR1
RASQSVSRSYL

SEQ ID NO: 161 - protein, 7 aa, synthetic construct
  REGION 1..7: note = 4G8 LCDR2
IGASTRA

SEQ ID NO: 162 - protein, 9 aa, synthetic construct
  REGION 1..9: note = 4G8 LCDR3
CQQGQVIPP

SEQ ID NO: 163 - protein, 5 aa, synthetic construct
  REGION 1..5: note = 3D9 HCDR1
SYAMS

SEQ ID NO: 164 - protein, 16 aa, synthetic construct
  REGION 1..16: note = 3D9 HCDR2
AIGVSTGSTYYADSVK

SEQ ID NO: 165 - protein, 8 aa, synthetic construct
  REGION 1..8: note = 3D9 HCDR3
YCAKGWLG

SEQ ID NO: 166 - protein, 11 aa, synthetic construct
  REGION 1..11: note = 3D9 LCDR1
RASQSVSSSYL

SEQ ID NO: 167 - protein, 7 aa, synthetic construct
  REGION 1..7: note = 3D9 LCDR2
YGASSRA

SEQ ID NO: 168 - protein, 9 aa, synthetic construct
  REGION 1..9: note = 3D9 LCDR3
CQQGQLIPP

SEQ ID NO: 169 - protein, 5 aa, synthetic construct
  REGION 1..5: note = 4B3 HCDR1
SYAMS

SEQ ID NO: 170 - protein, 16 aa, synthetic construct
  REGION 1..16: note = 4B3 HCDR2
AISGSGGSTYYADSVK

SEQ ID NO: 171 - protein, 8 aa, synthetic construct
  REGION 1..8: note = 4B3 HCDR3
YCAKGWLG

SEQ ID NO: 172 - protein, 11 aa, synthetic construct
  REGION 1..11: note = 4B3 LCDR1
RASQSVSSNYL

SEQ ID NO: 173 - protein, 7 aa, synthetic construct
  REGION 1..7: note = 4B3 LCDR2
YGAYIRA

SEQ ID NO: 174 - protein, 9 aa, synthetic construct
  REGION 1..9: note = 4B3 LCDR3
CQQGQVIPP

SEQ ID NO: 175 - protein, 5 aa, synthetic construct
  REGION 1..5: note = 19G1 HCDR1
SYAMS

SEQ ID NO: 176 - protein, 16 aa, synthetic construct
  REGION 1..16: note = 19G1 HCDR2
AIISSGGLTYYADSVK

SEQ ID NO: 177 - protein, 8 aa, synthetic construct
  REGION 1..8: note = 19G1 HCDR3
YCAKGWFG

SEQ ID NO: 178 - protein, 11 aa, synthetic construct
  REGION 1..11: note = 19G1 LCDR1
RASQSVTSSYL

SEQ ID NO: 179 - protein, 7 aa, synthetic construct
  REGION 1..7: note = 19G1 LCDR2
NVGSRRA

SEQ ID NO: 180 - protein, 9 aa, synthetic construct
  REGION 1..9: note = 19G1 LCDR3
CQQGIMLPP

SEQ ID NO: 181 - protein, 5 aa, synthetic construct
  REGION 1..5: note = 20G8 HCDR1
SYAMS

SEQ ID NO: 182 - protein, 16 aa, synthetic construct
  REGION 1..16: note = 20G8 HCDR2
AIIGSGSRTYYADSVK

SEQ ID NO: 183 - protein, 8 aa, synthetic construct
  REGION 1..8: note = 20G8 HCDR3
YCAKGWFG

SEQ ID NO: 184 - protein, 11 aa, synthetic construct
  REGION 1..11: note = 20G8 LCDR1
RASQSVTSSYL

SEQ ID NO: 185 - protein, 7 aa, synthetic construct
  REGION 1..7: note = 20G8 LCDR2
NVGSRRA

SEQ ID NO: 186 - protein, 9 aa, synthetic construct
  REGION 1..9: note = 20G8 LCDR3
CQQGIMLPP

SEQ ID NO: 187 - protein, 5 aa, synthetic construct
  REGION 1..5: note = 5B8 HCDR1
SYAMS

SEQ ID NO: 188 - protein, 16 aa, synthetic construct
  REGION 1..16: note = 5B8 HCDR2
AIWGGGRSTYYADSVK

SEQ ID NO: 189 - protein, 8 aa, synthetic construct
  REGION 1..8: note = 5B8 HCDR3
YCAKGWFG

SEQ ID NO: 190 - protein, 11 aa, synthetic construct
  REGION 1..11: note = 5B8 LCDR1
RASQSVTSSYL

SEQ ID NO: 191 - protein, 7 aa, synthetic construct
  REGION 1..7: note = 5B8 LCDR2
NVGSRRA

SEQ ID NO: 192 - protein, 9 aa, synthetic construct
  REGION 1..9: note = 5B8 LCDR3
CQQGIMLPP

SEQ ID NO: 193 - protein, 5 aa, synthetic construct
  REGION 1..5: note = 5F1 HCDR1
SYAMS

SEQ ID NO: 194 - protein, 16 aa, synthetic construct
  REGION 1..16: note = 5F1 HCDR2
AIISSGASTYYADSVK

SEQ ID NO: 195 - protein, 8 aa, synthetic construct
  REGION 1..8: note = 5F1 HCDR3
YCAKGWFG

SEQ ID NO: 196 - protein, 11 aa, synthetic construct
  REGION 1..11: note = 5F1 LCDR1
RASQSVTSSYL

SEQ ID NO: 197 - protein, 7 aa, synthetic construct
  REGION 1..7: note = 5F1 LCDR2
NVGSRRA

SEQ ID NO: 198 - protein, 9 aa, synthetic construct
  REGION 1..9: note = 5F1 LCDR3
CQQGIMLPP

SEQ ID NO: 199 - protein, 5 aa, synthetic construct
  REGION 1..5: note = 14B3 HCDR1
SYAMS

SEQ ID NO: 200 - protein, 16 aa, synthetic construct
  REGION 1..16: note = 14B3 HCDR2
AILASGAITYYADSVK

SEQ ID NO: 201 - protein, 8 aa, synthetic construct
  REGION 1..8: note = 14B3 HCDR3
YCAKGWFG

SEQ ID NO: 202 - protein, 11 aa, synthetic construct
  REGION 1..11: note = 14B3 LCDR1
RASQSVTSSYL

SEQ ID NO: 203 - protein, 7 aa, synthetic construct
  REGION 1..7: note = 14B3 LCDR2
NVGSRRA

SEQ ID NO: 204 - protein, 9 aa, synthetic construct
  REGION 1..9: note = 14B3 LCDR3
CQQGIMLPP

SEQ ID NO: 205 - protein, 5 aa, synthetic construct
  REGION 1..5: note = 16F1 HCDR1
SYAMS

SEQ ID NO: 206 - protein, 16 aa, synthetic construct
  REGION 1..16: note = 16F1 HCDR2
GIIGSGGITYYADSVK

SEQ ID NO: 207 - protein, 8 aa, synthetic construct
  REGION 1..8: note = 16F1 HCDR3
YCAKGWFG

SEQ ID NO: 208 - protein, 11 aa, synthetic construct
  REGION 1..11: note = 16F1 LCDR1
RASQSVTSSYL

SEQ ID NO: 209 - protein, 7 aa, synthetic construct
  REGION 1..7: note = 16F1 LCDR2
NVGSRRA

SEQ ID NO: 210 - protein, 9 aa, synthetic construct
  REGION 1..9: note = 16F1 LCDR3
CQQGIMLPP

SEQ ID NO: 211 - protein, 5 aa, synthetic construct
  REGION 1..5: note = 16F8 HCDR1
SYAMS

SEQ ID NO: 212 - protein, 16 aa, synthetic construct
  REGION 1..16: note = 16F8 HCDR2
AILGSGGSTYYADSVK

SEQ ID NO: 213 - protein, 8 aa, synthetic construct
  REGION 1..8: note = 16F8 HCDR3
YCAKGWFG

SEQ ID NO: 214 - protein, 11 aa, synthetic construct
  REGION 1..11: note = 16F8 LCDR1
RASQSVTSSYL

SEQ ID NO: 215 - protein, 7 aa, synthetic construct
  REGION 1..7: note = 16F8 LCDR2
NVGSRRA

SEQ ID NO: 216 - protein, 9 aa, synthetic construct
  REGION 1..9: note = 16F8 LCDR3
CQQGIMLPP

SEQ ID NO: 217 - protein, 5 aa, synthetic construct
  REGION 1..5: note = O3C9 HCDR1
SFAMS

SEQ ID NO: 218 - protein, 16 aa, synthetic construct
  REGION 1..16: note = O3C9 HCDR2
AIIGSGSNTYYADSVK

SEQ ID NO: 219 - protein, 8 aa, synthetic construct
  REGION 1..8: note = O3C9 HCDR3
YCAKGWFG

SEQ ID NO: 220 - protein, 11 aa, synthetic construct
  REGION 1..11: note = O3C9 LCDR1
RASQSVTSSYL

SEQ ID NO: 221 - protein, 7 aa, synthetic construct
  REGION 1..7: note = O3C9 LCDR2
NVGSRRA

SEQ ID NO: 222 - protein, 9 aa, synthetic construct
  REGION 1..9: note = O3C9 LCDR3
CQQGIMLPP

SEQ ID NO: 223 - protein, 5 aa, synthetic construct
  REGION 1..5: note = 22A3 HCDR1
SYAMS

SEQ ID NO: 224 - protein, 16 aa, synthetic construct
  REGION 1..16: note = 22A3 HCDR2
AIIGSGSITYYADSVK

SEQ ID NO: 225 - protein, 8 aa, synthetic construct
  REGION 1..8: note = 22A3 HCDR3
YCAKGWFG

SEQ ID NO: 226 - protein, 11 aa, synthetic construct
  REGION 1..11: note = 22A3 LCDR1
RASQSVTSSYL

SEQ ID NO: 227 - protein, 7 aa, synthetic construct
  REGION 1..7: note = 22A3 LCDR2
NVGSRRA

SEQ ID NO: 228 - protein, 9 aa, synthetic construct
  REGION 1..9: note = 22A3 LCDR3
CQQGIMLPP

SEQ ID NO: 229 - protein, 5 aa, synthetic construct
  REGION 1..5: note = 29B11 HCDR1
SYAMS

SEQ ID NO: 230 - protein, 16 aa, synthetic construct
  REGION 1..16: note = 29B11 HCDR2
AIIGSGGITYYADSVK

SEQ ID NO: 231 - protein, 8 aa, synthetic construct
  REGION 1..8: note = 29B11 HCDR3
YCAKGWFG

SEQ ID NO: 232 - protein, 11 aa, synthetic construct
  REGION 1..11: note = 29B11 LCDR1
RASQSVTSSYL

SEQ ID NO: 233 - protein, 7 aa, synthetic construct
  REGION 1..7: note = 29B11 LCDR2
NVGSRRA

SEQ ID NO: 234 - protein, 9 aa, synthetic construct
  REGION 1..9: note = 29B11 LCDR3
CQQGIMLPP

SEQ ID NO: 235 - protein, 5 aa, synthetic construct
  REGION 1..5: note = O2D7 HCDR1
SYAMS

SEQ ID NO: 236 - protein, 16 aa, synthetic construct
  REGION 1..16: note = O2D7 HCDR2
AISGSGGSTYYADSVK

SEQ ID NO: 237 - protein, 8 aa, synthetic construct
  REGION 1..8: note = O2D7 HCDR3
YCAKGWFG

SEQ ID NO: 238 - protein, 11 aa, synthetic construct
  REGION 1..11: note = O2D7 LCDR1
RASQSVTSSYL

SEQ ID NO: 239 - protein, 7 aa, synthetic construct
  REGION 1..7: note = O2D7 LCDR2
NVGSRRA

SEQ ID NO: 240 - protein, 9 aa, synthetic construct
  REGION 1..9: note = O2D7 LCDR3
CQQAIMLPP

SEQ ID NO: 241 - protein, 5 aa, synthetic construct
  REGION 1..5: note = 23C10 HCDR1
SSAMS

SEQ ID NO: 242 - protein, 16 aa, synthetic construct
  REGION 1..16: note = 23C10 HCDR2
AISTNGNYTYYADSVK

SEQ ID NO: 243 - protein, 8 aa, synthetic construct
  REGION 1..8: note = 23C10 HCDR3
YCAKGWLG

SEQ ID NO: 244 - protein, 11 aa, synthetic construct
  REGION 1..11: note = 23C10 LCDR1
RASQSVSRSYL

SEQ ID NO: 245 - protein, 7 aa, synthetic construct
  REGION 1..7: note = 23C10 LCDR2
IGASTRA

SEQ ID NO: 246 - protein, 9 aa, synthetic construct
  REGION 1..9: note = 23C10 LCDR3
CQQGQVIPP

SEQ ID NO: 247 - protein, 157 aa, synthetic construct
  REGION 1..157: note = DARPin AMG-506/MP-0310
DLGKKLLEAARAGQDDEVRELLKAGADVNAKDVLGWTPLHLAAFEGHLEIVEVLLKAGADVNAKDKKGWTPLQLAARTGHLEIVEVLLKAGADVNAKDHIGATPLHLAAWQGHPEIVEVLLKAGADVNAQDKSGKTPADLAADAGHEDIAEVLQKAA

SEQ ID NO: 248 - protein, 124 aa, synthetic construct; identical to SEQ ID NO: 107
  REGION 1..124: note = VH of NG-641

SEQ ID NO: 249 - protein, 113 aa, synthetic construct; identical to SEQ ID NO: 108
  REGION 1..113: note = VL of NG-641

SEQ ID NO: 250 - protein, 116 aa, synthetic construct
  REGION 1..116: note = VH of 28H1
EVQLLESGGGLVQPGGSLRLSCAASGFTFSSHAMSWVRQAPGKGLEWVSAIWASGEQYYADSVKGRFTISRDNSKNTLYLQMNSLRAEDTAVYYCAKGWLGNFDYWGQGTLVTVSS

SEQ ID NO: 251 - protein, 108 aa, synthetic construct
  REGION 1..108: note = VL of 28H1
EIVLTQSPGTLSLSPGERATLSCRASQSVSRSYLAWYQQKPGQAPRLLIIGASTRATGIPDRFSGSGSGTDFTLTISRLEPEDFAVYYCQQGQVIPPTFGQGTKVEIK

SEQ ID NO: 252 - protein, 117 aa, synthetic construct
  REGION 1..117: note = VH of 4B9
EVQLLESGGGLVQPGGSLRLSCAASGFTFSSYAMSWVRQAPGKGLEWVSAIIGSGASTYYADSVKGRFTISRDNSKNTLYLQMNSLRAEDTAVYYCAKGWFGGFNYWGQGTLVTVSS

SEQ ID NO: 253 - protein, 108 aa, synthetic construct
  REGION 1..108: note = VL of 4B9
EIVLTQSPGTLSLSPGERATLSCRASQSVTSSYLAWYQQKPGQAPRLLINVGSRRATGIPDRFSGSGSGTDFTLTISRLEPEDFAVYYCQQGIMLPPTFGQGTKVEIK

SEQ ID NO: 254 - protein, 121 aa, synthetic construct
  REGION 1..121: note = VH of OMTX-705
QVQLVQSGAEVKKPGASVKVSCKASGYTFTENIIHWVRQAPGQGLEWMGWFHPGSGSIKYNEKFKDRVTMTTADTSTSTVYMELSSLRSEDTAVYYCARHGGTGRGAMDYWGQGTLVTVSS

SEQ ID NO: 255 - protein, 112 aa, synthetic construct
  REGION 1..112: note = VL of OMTX-705
DIQMIQSPSSLSASVGDRVTITCRASKSVSTSAYSYMHWYQQKPGKAPKLLIYLASNLESGVPSRFSGSGSGTDFILTISSLQPEDFATYYCQHSRELPYTFGQGTKLEIKR

SEQ ID NO: 256 - protein, 117 aa, synthetic construct
  REGION 1..117: note = VH of 3F2
EVQLLESGGGLVQPGGSLRLSCAASGFTFSSYAMSWVRQAPGKGLEWVSAISGSGGSTYYADSVKGRFTISRDNSKNTLYLQMNSLRAEDTAVYYCAKGWFGGFNYWGQGTLVTVSS

SEQ ID NO: 257 - protein, 108 aa, synthetic construct
  REGION 1..108: note = VL of 3F2
EIVLTQSPGTLSLYPGERATLSCRASQSVTSSYLAWYQQKPGQAPRLLINVGSRRATGIPDRFSGSGSGTDFTLTISRLEPEDFAVYYCQQGIMLPPTFGQGTKVEIK

SEQ ID NO: 258 - protein, 117 aa, synthetic construct
  REGION 1..117: note = VH of 4G8
EVQLLESGGGLVQPGGSLRLSCAASGFTFSSYAMSWVRQAPGKGLEWVSAISGSGGSTYYADSVKGRFTISRDNSKNTLYLQMNSLRAEDTAVYYCAKGWLGNFDYWGQGTLVTVSS

SEQ ID NO: 259 - protein, 108 aa, synthetic construct; identical to SEQ ID NO: 251
  REGION 1..108: note = VL of 4G8

SEQ ID NO: 260 - protein, 117 aa, synthetic construct
  REGION 1..117: note = VH of 3D9
EVQLLESGGGLVQPGGSLRLSCAASGFTFSSYAMSWVRQTPGKGLEWVSAIGVSTGSTYYADSVKGRFTISRDNSKNTLYLQMNSLRAEDTAVYYCAKGWLGPFDYWGQGTLVTVSS

SEQ ID NO: 261 - protein, 108 aa, synthetic construct
  REGION 1..108: note = VL of 3D9
EIVLTQSPGTLSLSPGERATLSKRASQSVSSSYLAWYQQKPGQAPRLLIYGASSRATGIPDRFSGSGSGTDFTLTISRLEPEDFAVYYCQQGQLIPPTFGQGTKVEIK

SEQ ID NO: 262 - protein, 117 aa, synthetic construct; identical to SEQ ID NO: 258
  REGION 1..117: note = VH of 4B3

SEQ ID NO: 263 - protein, 108 aa, synthetic construct
  REGION 1..108: note = VL of 4B3
EIVLTQSPGTLSLSPGERATLSCRASQSVSSNYLAWYQQKPGQAPRLLIYGAYIRATGIPDRFSGSGSGTDFTLTISRLEPEDFAVYYCQQGQVIPPTFGQGTKVEIK

SEQ ID NO: 264 - protein, 117 aa, synthetic construct
  REGION 1..117: note = VH of 19G1
EVQLLESGGGLVQPGGSLRLSCAASGFTFSSYAMSWVRQAPGKGLEWVSAIISSGGLTYYADSVKGRFTISRDNSKNTLYLQMNSLRAEDTAVYYCAKGWFGGFNYWGQGTLVTVSS

SEQ ID NO: 265 - protein, 108 aa, synthetic construct
  REGION 1..108: note = VL of 19G1
EIVLTQSPGTLSLSPGERATLSCRASQSVTSSYLAWYQQGPGQAPRLLINVGSRRATGIPDRFSGSGSGTDFTLTISRLEPEDFAVYYCQQGIMLPPTFGQGTKVEIK

SEQ ID NO: 266 - protein, 117 aa, synthetic construct
  REGION 1..117: note = VH of 20G8
EVQLLESGGGLVQPGGSLRLSCAASGFTFSSYAMSWVRQAPGKKLEWVSAIIGSGSRTYYADSVKGRFTISRDNSKNTLYLQMNSLRAEDTAVYYCAKGWFGGFNYWGQGTLVTVSS

SEQ ID NO: 267 - protein, 108 aa, synthetic construct; identical to SEQ ID NO: 253
  REGION 1..108: note = VL of 20G8

SEQ ID NO: 268 - protein, 117 aa, synthetic construct
  REGION 1..117: note = VH of 5B8
EVQLLESGGGLVQPGGSLRLSCAASGFTFSSYAMSWVRQAPGKGLEWVSAIWGGGRSTYYADSVKGRFTISRDNSKNTLYLQMNSLRAEDTAVYYCAKGWFGGFNYWGQGTLVTVSS

SEQ ID NO: 269 - protein, 108 aa, synthetic construct; identical to SEQ ID NO: 253
  REGION 1..108: note = VL of 5B8

SEQ ID NO: 270 - protein, 117 aa, synthetic construct
  REGION 1..117: note = VH of 5F1
EVQLLESGGGLVQPGGSLRLSCAASGFTFSSYAMSWVRQAPGKGLEWVSAIISSGASTYYADSVKGRFTISRDNSKNTLYLQMNSLRAEDTAVYYCAKGWFGGFNYWGQGTLVTVSS

SEQ ID NO: 271 - protein, 108 aa, synthetic construct; identical to SEQ ID NO: 253
  REGION 1..108: note = VL of 5F1

SEQ ID NO: 272 - protein, 117 aa, synthetic construct
  REGION 1..117: note = VH of 14B3
EVQLLESGGGLVQPGGSLRLSCAASGFTFSSYAMSWVRQAPGKGLEWVSAILASGAITYYADSVKGRFTISRDNSKNTLYLQMNSLRAEDTAVYYCAKGWFGGFNYWGQGTLVTVSS

SEQ ID NO: 273 - protein, 108 aa, synthetic construct
  REGION 1..108: note = VL of 14B3
EIVLTQSPGTLSLSPGERATLSCRASQSVTSSYLAWYQQGPGGAPRLLINVGSRRATGIPDRFSGSGSGTDFTLTISRLEPEDFAVYYCQQGIMLPPTFGQGTKVEIK

SEQ ID NO: 274 - protein, 117 aa, synthetic construct
  REGION 1..117: note = VH of 16F1
EVQLLESGGGLVQPGGSLRLSCAASGFTFSSYAMSWVRQAPGKGLEWVSGIIGSGGITYYADSVKGDFTISRDNSGNTLYLQMNSLRAEDTAVYYCAKGWFGGFNYWGQGTLVTVSS

SEQ ID NO: 275 - protein, 108 aa, synthetic construct; identical to SEQ ID NO: 253
  REGION 1..108: note = VL of 16F1

SEQ ID NO: 276 - protein, 117 aa, synthetic construct
  REGION 1..117: note = VH of 16F8
EVQLLESGGGLVQPGGSLRLSCAASGFTFSSYAMSWVRQAPGKGLEWVSAILGSGGSTYYADSVKGRFTISRDNSKNTLYLQMNSLRAEDTAVYYCAKGWFGGFNYWGQGTLVTVSS

SEQ ID NO: 277 - protein, 108 aa, synthetic construct; identical to SEQ ID NO: 253
  REGION 1..108: note = VL of 16F8

SEQ ID NO: 278 - protein, 117 aa, synthetic construct
  REGION 1..117: note = VH of O3C9
EVQLLESGGGLVQPGGSLRLSCAASGFTFSSFAMSWVRQSPGKGLEWVSAIIGSGSNTYYADSVKGRFTISRDNSKNTLYLQMNSLRAEDTAVYYCAKGWFGGFNYWGQGTLVTVSS

SEQ ID NO: 279 - protein, 108 aa, synthetic construct; identical to SEQ ID NO: 253
  REGION 1..108: note = VL of O3C9

SEQ ID NO: 280 - protein, 117 aa, synthetic construct
  REGION 1..117: note = VH of 22A3
EVQLLESGGGLVQPGGSLRLSCAASGFTFSSYAMSWVRQAPGKGLEWVSAIIGSGSITYYADSVKGRFTISRDNSKNTLYLQMNSLRAEDTAVYYCAKGWFGGFNYWGQGTLVTVSS

SEQ ID NO: 281 - protein, 108 aa, synthetic construct; identical to SEQ ID NO: 253
  REGION 1..108: note = VL of 22A3

SEQ ID NO: 282 - protein, 117 aa, synthetic construct
  REGION 1..117: note = VH of 29B11
EVQLLESGGGLVQPGGSLRLSCAASGFTFSSYAMSWVRQAPGKGLEWVSAIIGSGGITYYADSVKGRFTISRDNSKNTLYLQMNSLRAEDTAVYYCAKGWFGGFNYWGQGTLVTVSS

SEQ ID NO: 283 - protein, 108 aa, synthetic construct; identical to SEQ ID NO: 253
  REGION 1..108: note = VL of 29B11

SEQ ID NO: 284 - protein, 117 aa, synthetic construct; identical to SEQ ID NO: 256
  REGION 1..117: note = VH of O2D7

SEQ ID NO: 285 - protein, 108 aa, synthetic construct
  REGION 1..108: note = VL of O2D7
EIVLTQSPGTLSLSPGERATLSCRASQSVTSSYLAWYQQKPGQAPRLLINVGSRRATGTPDRFSGSGSGTDFTLTISRLEPEDFAVYYCQQAIMLPPTFGQGTKVEIK

SEQ ID NO: 286 - protein, 117 aa, synthetic construct
  REGION 1..117: note = VH of 23C10
EVQLLESGGGLVQPGGSLRLSCAASGFTFSSSAMSWVRQAPGKGLEWVSAISTNGNYTYYADSVKGRFTISRDNSKNTLYLQMNSLRAEDTAVYYCAKGWLGNFDYWGQGTLVTVSS

SEQ ID NO: 287 - protein, 108 aa, synthetic construct; identical to SEQ ID NO: 251
  REGION 1..108: note = VL of 23C10

SEQ ID NO: 288 - protein, 318 aa, synthetic construct
  REGION 1..318: note = human scLTb2
LPAAHLIGAPLKGQGLGWETTKEQAFLTSGTQFSDAEGLALPQDGLYYLYCLVGYRGRAPPGGGDPQGRSVTLRSSLYRAGGAYGPGTPELLLEGAETVTPVLDPARRQGYGPLWYTSVGFGGLVQLRRGERVYVNISHPDMVDFARGKTFFGAVMVGGSGLPAAHLIGAPLKGQGLGWETTKEQAFLTSGTQFSDAEGLALPQDGLYYLYCLVGYRGRAPPGGGDPQGRSVTLRSSLYRAGGAYGPGTPELLLEGAETVTPVLDPARRQGYGPLWYTSVGFGGLVQLRRGERVYVNISHPDMVDFARGKTFFGAVMV

SEQ ID NO: 289 - protein, 306 aa, synthetic construct
  REGION 1..306: note = Mouse LTb origin
MGTRGLQGLGGRPQGRGCLLLAVAGATSLVTLLLAVPITVLAVLALVPQDQGRRVEKIIGSGAQAQKRLDDSKPSCILPSPSSLSETPDPRLHPQRSNASRNLASTSQGPVAQSSREASAWMTILSPAADSTPDPGVQQLPKGEPETDLNPELPAAHLIGAWMSGQGLSWEASQEEAFLRSGAQFSPTHGLALPQDGVYYLYCHVGYRGRTPPAGRSRARSLTLRSALYRAGGAYGRGSPELLLEGAETVTPVVDPIGYGSLWYTSVGFGGLAQLRSGERVYVNISHPDMVDYRRGKTFFGAVMVG

SEQ ID NO: 290 - protein, 153 aa, synthetic construct
  REGION 1..153: note = Mouse LTb
LPAAHLIGAWMSGQGLSWEASQEEAFLRSGAQFSPTHGLALPQDGVYYLYCHVGYRGRTPPAGRSRARSLTLRSALYRAGGAYGRGSPELLLEGAETVTPVVDPIGYGSLWYTSVGFGGLAQLRSGERVYVNISHPDMVDYRRGKTFFGAVMV

SEQ ID NO: 291 - protein, 310 aa, synthetic construct
  REGION 1..310: note = Mouse scLTb2
LPAAHLIGAWMSGQGLSWEASQEEAFLRSGAQFSPTHGLALPQDGVYYLYCHVGYRGRTPPAGRSRARSLTLRSALYRAGGAYGRGSPELLLEGAETVTPVVDPIGYGSLWYTSVGFGGLAQLRSGERVYVNISHPDMVDYRRGKTFFGAVMVGGSGLPAAHLIGAWMSGQGLSWEASQEEAFLRSGAQFSPTHGLALPQDGVYYLYCHVGYRGRTPPAGRSRARSLTLRSALYRAGGAYGRGSPELLLEGAETVTPVVDPIGYGSLWYTSVGFGGLAQLRSGERVYVNISHPDMVDYRRGKTFFGAVMV

SEQ ID NO: 292 - protein, 227 aa, synthetic construct
  REGION 1..227: note = hu IgG1 Fc Origin
DKTHTCPPCPAPELLGGPSVFLFPPKPKDTLMISRTPEVTCVVVDVSHEDPEVKFNWYVDGVEVHNAKTKPREEQYNSTYRVVSVLTVLHQDWLNGKEYKCKVSNKALPAPIEKTISKAKGQPREPQVYTLPPSRDELTKNQVSLTCLVKGFYPSDIAVEWESNGQPENNYKTTPPVLDSDGSFFLYSKLTVDKSRWQQGNVFSCSVMHEALHNHYTQKSLSLSPGK

SEQ ID NO: 293 - protein, 233 aa, synthetic construct
  REGION 1..233: note = mu IgG2a Fc Origin
EPRGPTIKPCPPCKCPAPNLLGGPSVFIFPPKIKDVLMISLSPIVTCVVVDVSEDDPDVQISWFVNNVEVHTAQTQTHREDYNSTLRVVSALPIQHQDWMSGKEFKCKVNNKDLPAPIERTISKPKGSVRAPQVYVLPPPEEEMTKKQVTLTCMVTDFMPEDIYVEWTNNGKTELNYKNTEPVLDSDGSYFMYSKLRVEKKNWVERNSYSCSVVHEGLHNHHTTKSFSRTPGK

SEQ ID NO: 294 - protein, 227 aa, synthetic construct [sequence omitted]

SEQ ID NO: 295 - protein, 227 aa, synthetic construct
  REGION 1..227: note = hu IgG1 Fc hole
DKTHTCPPCPAPELLGGPSVFLFPPKPKDTLMISRTPEVTCVVVDVSHEDPEVKFNWYVDGVEVHNAKTKPREEQYNSTYRVVSVLTVLHQDWLNGKEYKCKVSNKALPAPIEKTISKAKGQPREPQVYTLPPSRDELTKNQVSLSCAVKGFYPSDIAVEWESNGQPENNYKTTPPVLDSDGSFFLVSKLTVDKSRWQQGNVFSCSVMHEALHNHYTQKSLSLSPGK

SEQ ID NO: 296 - protein, 233 aa, synthetic construct
  REGION 1..233: note = mu IgG2a Fc hole
EPRGPTIKPCPPCKCPAPNLLGGPSVFIFPPKIKDVLMISLSPIVTCVVVDVSEDDPDVQISWFVNNVEVHTAQTQTHREDYNSTLRVVSALPIQHQDWMSGKEFKCKVNNKDLPAPIERTISKPKGSVRAPQVYVLPPPEEEMTKKQVTLSCAVTDFMPEDIYVEWTNNGKTELNYKNTEPVLDSDGSYFMVSKLRVEKKNWVERNSYSCSVVHEGLHNHHTTKSFSRTPGK

SEQ ID NO: 297 - protein, 227 aa, synthetic construct
  REGION 1..227: note = hu IgG1 Fc DANG
DKTHTCPPCPAPELLGGPSVFLFPPKPKDTLMISRTPEVTCVVVAVSHEDPEVKFNWYVDGVEVHNAKTKPREEQYGSTYRVVSVLTVLHQDWLNGKEYKCKVSNKALPAPIEKTISKAKGQPREPQVYTLPPSRDELTKNQVSLTCLVKGFYPSDIAVEWESNGQPENNYKTTPPVLDSDGSFFLYSKLTVDKSRWQQGNVFSCSVMHEALHNHYTQKSLSLSPGK

SEQ ID NO: 298 - protein, 233 aa, synthetic construct
  REGION 1..233: note = mu IgG2a Fc DANG
EPRGPTIKPCPPCKCPAPNLLGGPSVFIFPPKIKDVLMISLSPIVTCVVVAVSEDDPDVQISWFVNNVEVHTAQTQTHREDYGSTLRVVSALPIQHQDWMSGKEFKCKVNNKDLPAPIERTISKPKGSVRAPQVYVLPPPEEEMTKKQVTLTCMVTDFMPEDIYVEWTNNGKTELNYKNTEPVLDSDGSYFMYSKLRVEKKNWVERNSYSCSVVHEGLHNHHTTKSFSRTPGK